European Patent Application EP 4 215 039 A1, published July 26, 2023. Title: Lox3 gene modulation and armyworm tolerance. Applicant: KWS SAAT SE & Co. KGaA. The sequence listing filed with the application follows.

SEQUENCE LISTING (89 sequences)

SEQ ID NO: 1 - DNA, 201 bp, Artificial Sequence
  RNAi target region sense strand before RGA2intronII
ctgccgcacgggccgcaagcccaccaaaaccgaccccaactcggagagccgactgtcgctggtggagcagatctacgtgccgcgggacgagcgcttcggccacctcaagatgtccgacttcctgggctactccatcaaggccatcacgcagggcatcatcccggcggtgcgcacgtacgtggacaccaccccgggcgagtt

SEQ ID NO: 2 - DNA, 201 bp, Artificial Sequence
  RNAi target region antisense strand after the RGA2intronII
aactcgcccggggtggtgtccacgtacgtgcgcaccgccgggatgatgccctgcgtgatggccttgatggagtagcccaggaagtcggacatcttgaggtggccgaagcgctcgtcccgcggcacgtagatctgctccaccagcgacagtcggctctccgagttggggtcggttttggtgggcttgcggcccgtgcggcag

SEQ ID NO: 3 - DNA, 312 bp, Artificial Sequence
  RGA2intronII sequence from Triticum aestivum
gtatggatagtgtatcttcatactgcatttgtttaatttgaaaatggttatctagttgcctaacaaaatatagctgggatatcatataacacatgtgcaggtgacatggaaaaaaatgcctatttttctatgcactaactattcatcatgtgacatacttccccaaaaaactaaataagccaaattttccagcttccgagtcctgaaaaagagtagtgtacctgatacaatttatagagtttttttttcgaaaagaagggatggccctcatagatagagtactaactaaaagtctacttttaccaatttcag

SEQ ID NO: 4 - DNA, 726 bp, Artificial Sequence
  Sequence of RNAi cassette
ctgccgcacgggccgcaagcccaccaaaaccgaccccaactcggagagccgactgtcgctggtggagcagatctacgtgccgcgggacgagcgcttcggccacctcaagatgtccgacttcctgggctactccatcaaggccatcacgcagggcatcatcccggcggtgcgcacgtacgtggacaccaccccgggcgagttcgagaggtatggatagtgtatcttcatactgcatttgtttaatttgaaaatggttatctagttgcctaacaaaatatagctgggatatcatataacacatgtgcaggtgacatggaaaaaaatgcctatttttctatgcactaactattcatcatgtgacatacttccccaaaaaactaaataagccaaattttccagcttccgagtcctgaaaaagagtagtgtacctgatacaatttatagagtttttttttcgaaaagaagggatggccctcatagatagagtactaactaaaagtctacttttaccaatttcaggcctcgaactcgcccggggtggtgtccacgtacgtgcgcaccgccgggatgatgccctgcgtgatggccttgatggagtagcccaggaagtcggacatcttgaggtggccgaagcgctcgtcccgcggcacgtagatctgctccaccagcgacagtcggctctccgagttggggtcggttttggtgggcttgcggcccgtgcggcag

SEQ ID NO: 5 - DNA, 12924 bp, Artificial Sequence
  Sequence of a complete artificial vector
aaaaggatctaggtgaagatcctttttgataatctcatgaccaaaatcccttaacgtgagttttcgttccactgagcgtcagaccccgtagaaaagatcaaaggatcttcttgagatcctttttttctgcgcgtaatctgctgcttgcaaacaaaaaaaccaccgctaccagcggtggtttgtttgccggatcaagagctaccaactctttttccgaaggtaactggcttcagcagagcgcagataccaaatactgttcttctagtgtagccgtagttaggccaccacttcaagaactctgtagcaccgcctacatacctcgctctgctaatcctgttaccagtggctgctgccagtggcgataagtcgtgtcttaccgggttggactcaagacgatagttaccggataaggcgcagcggtcgggctgaacggggggttcgtgcacacagcccagcttggagcgaacgacctacaccgaactgagatacctacagcgtgagctatgagaaagcgccacgcttcccgaagggagaaaggcggacaggtatccggtaagcggcagggtcggaacaggagagcgcacgagggagcttccagggggaaacgcctggtatctttatagtcctgtcgggtttcgccacctctgacttgagcgtcgatttttgtgatgctcgtcaggggggcggagcctatggaaaaacgccagcaacgcggcctttttacggttcctggccttttgctggccttttgctcacatgttctttcctgcgttatcccctgattctgtggataaccgattaccgcctttgagtgagctgataccgctcgccgcagccgaacgaccgagcgcagcgagtcagtgagcgaggaagcggaagagcgcctgatgcggtattttctccttacgcatctgtgcggtatttcacaccgcatatggtgcactctcagtacaatctgctctgatgccgcatagttaagccagtatacactccgctatcgctacgtgactgggtcatggctgcgccccgacacccgccaacacccgctgacgcgccctgacgggcttgtctgctcccggcatccgcttacagacaagctgtgaccgtctccgggagctgcatgtgtcagaggttttcaccgtcatcaccgaaacgcgcgaggcaggggtacgtcgaggtcgatccaacccctccgctgctatagtgcagtcggcttctgacgttcagtgcagccgtcttctgaaaacgacatgtcgcacaagtcctaagttacgcgacaggctgccgccctgcccttttcctggcgttttcttgtcgcgtgttttagtcgcataaagtagaatacttgcgactagaaccggagacattacgccatgaacaagagcgccgccgctggcctgctgggctatgcccgcgtcagcaccgacgaccaggacttgaccaaccaacgggccgaactgcacgcggccggctgcaccaagctgttttccgagaagatcaccggcaccaggcgcgaccgcccggagctggccaggatgcttgaccacctacgccctggcgacgttgtgacagtgaccaggctagaccgcctggcccgcagcacccgcgacctactggacattgccgagcgcatccaggaggccggcgcgggcctgcgtagcctggcagagccgtgggccgacaccaccacgccggccggccgcatggtgttgaccgtgttcgccggcattgccgagttcgagcgttccctaatcatcgaccgcacccggagcgggcgcgaggccgccaaggcgcgaggcgtgaagtttggcccccgccctaccctcaccccggcacagatcgcgcacgcccgcgagctgatcgaccaggaaggccgcaccgtgaaagaggcggctgcactgcttggcgtgcatcgctcgaccctgtaccgcgcacttgagcgcagcgaggaagtgacgcccaccgaggccaggcggcgcggtgccttccgtgaggacgcattgaccgaggccgacgccctggcggccgccgagaatgaacgccaagaggaacaagcatgaaaccgcaccaggacggccaggacgaaccgtttttcattaccgaagagatcgaggcggagatgatcgcggccgggtacgtgttcgagccgcccgcgcacgtctcaaccgtgcggctgcatgaaatcctggccggtttgtctgatgccaagctcgcggcctggccggcgagcttggccgctgaagaaaccgagcgccgccgtctaaaaaggtgatgtgtatttgagtaaaacagcttgcgtcatgcggtcgctgcgtatatgatgcgatgagtaaataaacaaatacgcaaggggaacgcatgaaggttatcgctgtacttaaccagaaaggcgggtcaggcaagacgaccatcgcaacccatctagcccgcgccctgcaactcgccggggccgatgttctgttagtcgattccgatccccagggcagtgcccgcgattgggcggccgtgcgggaagatcaaccgctaaccgttgtcggcatcgaccgcccgacgattgaccgcgacgtgaaggccatcggccggcgcgacttcgtagtgatcgacggagcgccccaggcggcggacttggctgtgtccgcgatcaaggcagccgacttcgtgctgattccggtgcagccaagcccttacgacatatgggccaccgccgacctggtggagctggttaagcagcgcattgaggtcacggatggaaggctacaagcggcctttgtcgtgtcgcgggcgatcaaaggcacgcgcatcggcggtgaggttgccgaggcgctggccgggtacgagctgcccattcttgagtcccgtatcacgcagcgcgtgagctacccaggcactgccgccgccggcacaaccgttcttgaatcagaacccgagggcgacgctgcccgcgaggtccaggcgctggccgctgaaattaaatcaaaactcatttgagttaatgaggtaaagagaaaatgagcaaaagcacaaacacgctaagtgccggccgtccgagcgcacgcagcagcaaggctgcaacgttggccagcctggcagacacgccagccatgaagcgggtcaactttcagttgccggcggaggatcacaccaagctgaagatgtacgcggtacgccaaggcaagaccattaccgagctgctatctgaatacatcgcgcagctaccagagtaaatgagcaaatgaataaatgagtagatgaattttagcggctaaaggaggcggcatggaaaatcaagaacaaccaggcaccgacgccgtggaatgccccatgtgtggaggaacgggcggttggccaggcgtaagcggctgggttgtctgccggccctgcaatggcactggaacccccaagcccgaggaatcggcgtgagcggtcgcaaaccatccggcccggtacaaatcggcgcggcgctgggtgatgacctggtggagaagttgaaggcggcgcaggccgcccagcggcaacgcatcgaggcagaagcacgccccggtgaatcgtggcaagcggccgctgatcgaatccgcaaagaatcccggcaaccgccggcagccggtgcgccgtcgattaggaagccgcccaagggcgacgagcaaccagattttttcgttccgatgctctatgacgtgggcacccgcgatagtcgcagcatcatggacgtggccgttttccgtctgtcgaagcgtgaccgacgagctggcgaggtgatccgctacgagcttccagacgggcacgtagaggtttccgcagggccggccggcatggcgagtgtgtgggattacgacctggtactgatggcggtttcccatctaaccgaatccatgaaccgataccgggaagggaagggagacaagcccggccgcgtgttccgtccacacgttgcggacgtactcaagttctgccggcgagccgatggcggaaagcagaaagacgacctggtagaaacctgcattcggttaaacaccacgcacgttgccatgcagcgtacgaagaaggccaagaacggccgcctggtgacggtatccgagggtgaagccttgattagccgctacaagatcgtaaagagcgaaaccgggcggccggagtacatcgagatcgagctagctgattggatgtaccgcgagatcacagaaggcaagaacccggacgtgctgacggttcaccccgattactttttgatcgatcccggcatcggccgttttctctaccgcctggcacgccgcgccgcaggcaaggcagaagccagatggttgttcaagacgatctacgaacgcagtggcagcgccggagagttcaagaagttctgtttcaccgtgcgcaagctgatcgggtcaaatgacctgccggagtacgatttgaaggaggaggcggggcaggctggcccgatcctagtcatgcgctaccgcaacctgatcgagggcgaagcatccgccggttcctaatgtacggagcagatgctagggcaaattgccctagcaggggaaaaaggtcgaaaaggtctctttcctgtggatagcacgtacattgggaacccaaagccgtacattgggaaccggaacccgtacattgggaacccaaagccgtacattgggaaccggtcacacatgtaagtgactgatataaaagagaaaaaaggcgatttttccgcctaaaactctttaaaacttattaaaactcttaaaacccgcctggcctgtgcataactgtctggccagcgcacagccgaagagctgcaaaaagcgcctacccttcggtcgctgcgctccctacgccccgccgcttcgcgtcggcctatcgcggccgctggccgctcaaaaatggctggcctacggccaggcaatctaccagggcgcggacaagccgcgccgtcgccactcgaccgccggcgcccacatcaaggcaccggtgggtatgcctgacgatgcgtggagaccgaaaccttgcgctcgttcgccagccaggacagaaatgcctcgacttcgctgctgcccaaggttgccgggtgacgcacaccgtggaaacggatgaaggcacgaacccagtggacataagcctgttcggttcgtaagctgtaatgcaagtagcgtatgcgctcacgcaactggtccagaaccttgaccgaacgcagcggtggtaacggcgcagtggcggttttcatggcttgttatgactgtttttttggggtacagtctatgcctcgggcatccaagcagcaagcgcgttacgccgtgggtcgatgtttgatgttatggagcagcaacgatgttacgcagcagggcagtcgccctaaaacaaagttaaacatcatgagggaagcggtgatcgccgaagtatcgactcaactatcagaggtagttggcgtcatcgagcgccatctcgaaccgacgttgctggccgtacatttgtacggctccgcagtggatggcggcctgaagccacacagtgatattgatttgctggttacggtgaccgtaaggcttgatgaaacaacgcggcgagctttgatcaacgaccttttggaaacttcggcttcccctggagagagcgagattctccgcgctgtagaagtcaccattgttgtgcacgacgacatcattccgtggcgttatccagctaagcgcgaactgcaatttggagaatggcagcgcaatgacattcttgcaggtatcttcgagccagccacgatcgacattgatctggctatcttgctgacaaaagcaagagaacatagcgttgccttggtaggtccagcggcggaggaactctttgatccggttcctgaacaggatctatttgaggcgctaaatgaaaccttaacgctatggaactcgccgcccgactgggctggcgatgagcgaaatgtagtgcttacgttgtcccgcatttggtacagcgcagtaaccggcaaaatcgcgccgaaggatgtcgctgccgactgggcaatggagcgcctgccggcccagtatcagcccgtcatacttgaagctagacaggcttatcttggacaagaagaagatcgcttggcctcgcgcgcagatcagttggaagaatttgtccactacgtgaaaggcgagatcaccaaggtagtcggcaaataatgtctaacaattcgttcaagccgacgccgcttcgcggcgcggcttaactcaagcgttagatgcactaagcacataattgctcacagccaaactatcaggtcaagtctgcttttattatttttaagcgtgcataataagccctacacaaattgggagatatatcatgaaaggctggctttttcttgttatcgcaatagttggcgaagtaatcgcaacatagcttgcttggtcgttccgcgtgaacgtcggctcgattgtacctgcgttcaaatactttgcgatcgtgttgcgcgcctgcccggtgcgtcggctgatctcacggatcgactgcttctctcgcaacgccatccgacggatgatgtttaaaagtcccatgtggatcactccgttgccccgtcgctcaccgtgttggggggaaggtgcacatggctcagttctcaatggaaattatctgcctaaccggctcagttctgcgtagaaaccaacatgcaagctccaccgggtgcaaagcggcagcggcggcaggatatattcaattgtaaatggcttcatgtccgggaaatctacatggatcagcaatgagtatgatggtcaatatggagaaaaagaaagagtaattaccaattttttttcaattcaaaaatgtagatgtccgcagcgttattataaaatgaaagtacattttgataaaacgacaaattacgatccgtcgtatttataggcgaaagcaataaacaaattattctaattcggaaatctttatttcgacgtgtctacattcacgtccaaatgggggcttagatgagaaacttcacgatcggctctagctagggataacagggtaatgcgtgctgcagggctgaagcggtgcgggaagagctgcaggctgaggtacaccaactacctgaggcccaacctcaagcacgagaacttcacgtacgcactggattttggttttaggaattagaaattttattgatagaagtattttacaaatacaaatacatactaagggtttcttatatgctcaacacatgagcgaaaccctataagaaccctaattcccttatctgggaactactcacacattattatagagagagatagatttgtagagagagactggtgatttcagcttcagatctttactccggcagcgttgtgtcgcccgcgttgagcggccgttgcatgagcaccgtgtcgatccagcggccgaacttgaagccgacggacttgagcacgcctgcctgcacgaagccgcaggcggcatgcagaccgagggacgccgtattgccgctgtcgccgacgttcgcaatcagttgccgccacgggccgccttcgcaacgcgcgatgagcgtgagcaacagcgtgcgccctacgccctgcccgatcgcatcgggggcgatatacaccgagtcttccagcgtgaaacggtaggcggagcgcggccggtaatgcgtggcgtatgcgtagccgagcagcttgccgtcgcgttcggcgacgagatacggcagtccggcgtcgagtaccttggcgcaacgcgcgcgcatctcggtgtcgtcgggtggcacctcttcgaacgatgccgtgccggtacgcacgtgatgggcgtagatggccgtgatggcgggcaggtcgtcgtcacgcacgacgcgcaccgtgcatgcgcaacgcgccagttcgacgccgacgcgttgcggcgcgtcgggagtggaggggtgagacgaagatgacggcatggtctgcagctcgagccgcagctgcacgggtccaggaaagcaatcgcatagtcaagctaaatcatcaagatgcaaacttttcgcccttgctaaacacggtaaaattcgaatggacatgtgtggagcagcaaaggccttacgtccgagaaacagggccactcaacgagttagttaaattcaaagaaagaaacgcctccttgcaagttgcaacattcctagatcatactaatgaaaatgacgtccttcattaaagaacagggaagatagatttttgctccatagatcgtatgatgtgttcagccagactgtcggatggaccacacggtaatagcagtgctggacgatgttacatcgagaaagattactagccttttcatgggagtaaaggatataaaagaaataagttcaccacgattgcaggatagcatacaagatcagcgccactgcggcactgttcatcgaaaaaaaactgtggacgaagctttccccaaaattactcaacgaatcataaaccaagattagtcagatcaagagacagaggagaaacaaggcggacctttgcagtcgaggtcctctccaaatgaaatgaacttccttatatagaggaagggtcttgcgaaggatagtgggattgtgcgtcatcccttacgtcagtggagatatcacatcaatccacttgctttgaagacgtggttggaacgtcttctttttccacgatgttcctcgtgggtgggggtccatctttgggaccactgtcggtagaggcatcttgaacgatagcctttcctttatcgcaatgatggcatttgtagaagccatcttccttttctactgtcctttcgatgaagtgacagatagctgggcaatggaatccgaggaggtttcccgatattaccctttgttgaaaagtctcaatagccctctggtcttctgagactgtatctttgatattcttggagtagacgagagtgtcgtgctccaccatgtatcacatcaatccacttgctttgaagacgtggttggaacgtcttctttttccacgatgttcctcgtgggtgggggtccatctttgggaccactgtcggtagaggcatcttgaacgatagcctttcctttatcgcaatgatggcatttgtagaagccatcttccttttctactgtcctttcgatgaagtgacagatagctgggcaatggaatccgaggaggtttcccgatattaccctttgttgaaaagtctcaatagccctctggtcttctgaacgcgtgctgcagggctgaagcggtgcgggaagagctgcaggctgaggtacaccaactacctgaggcccaacctcaagcacgagaacttcacgtacgctagggataacagggtaatccaatggtctagaggccatggcggccgcgtcgagcgatctagtaacatagatgacaccgcgcgcgataatttatcctagtttgcgcgctatattttgttttctatcgcgtattaaatgtataattgcgggactctaatcataaaaacccatctcataaataacgtcatgcattacatgttaattattacatgcttaacgtaattcaacagaaattatatgataatcatcgcaagaccggcaacaggattcaatcttaagaaactttattgccaaatgtttgaacgatcggggaaattcgagtcgacacgcgtaagcttgaattcctgcagcccgggggattgctgccgcacgggccgcaagcccaccaaaaccgaccccaactcggagagccgactgtcgctggtggagcagatctacgtgccgcgggacgagcgcttcggccacctcaagatgtccgacttcctgggctactccatcaaggccatcacgcagggcatcatcccggcggtgcgcacgtacgtggacaccaccccgggcgagttcgaggcctgaaattggtaaaagtagacttttagttagtactctatctatgagggccatcccttcttttcgaaaaaaaaactctataaattgtatcaggtacactactctttttcaggactcggaagctggaaaatttggcttatttagttttttggggaagtatgtcacatgatgaatagttagtgcatagaaaaataggcatttttttccatgtcacctgcacatgtgttatatgatatcccagctatattttgttaggcaactagataaccattttcaaattaaacaaatgcagtatgaagatacactatccatacctctcgaactcgcccggggtggtgtccacgtacgtgcgcaccgccgggatgatgccctgcgtgatggccttgatggagtagcccaggaagtcggacatcttgaggtggccgaagcgctcgtcccgcggcacgtagatctgctccaccagcgacagtcggctctccgagttggggtcggttttggtgggcttgcggcccgtgcggcagcaatccccgggtacctctagacttgtacagctcgtccatgccgtacaggaacaggtggtggcggccctcggagcgacctgcagaagtaacaccaaacaacagggtgagcatcgacaaaagaaacagtaccaagcaaataaatagcgtatgaaggcagggctaaaaaaatccacatatagctgctgcatatgccatcatccaagtatatcaagatcaaaataattataaaacatacttgtttattataatagataggtactcaaggttagagcatatgaatagatgctgcatatgccatcatgtatatgcatcagtaaaacccacatcaacatgtatacctatcctagatcgatatttccatccatcttaaactcgtaactatgaagatgtatgacacacacatacagttccaaaattaataaatacaccaggtagtttgaaacagtattctactccgatctagaacgaatgaacgaccgcccaaccacaccacatcatcacaaccaagcgaacaaaaagcatctctgtatatgcatcagtaaaacccgcatcaacatgtatacctatcctagatcgatatttccatccatcatcttcaattcgtaactatgaatatgtatggcacacacatacagatccaaaattaataaatccaccaggtagtttgaaacagaattctactccgatctagaacgaccgcccaaccagaccacatcatcacaaccaagacaaaaaaaagcatgaaaagatgacccgacaaacaagtgcacggcatatattgaaataaaggaaaagggcaaaccaaaccctatgcaacgaaacaaaaaaaatcatgaaatcgatcccgtctgcggaacggctagagccatcccaggattccccaaagagaaacactggcaagttagcaatcagaacgtgtctgacgtacaggtcgcatccgtgtacgaacgctagcagcacggatctaacacaaacacggatctaacacaaacatgaacagaagtagaactaccgggccctaaccatggaccggaacgccgatctagagaaggtagagagggggggggggggaggacgagcggcgtaccttgaagcggaggtgccgacgggtggatttgggggagatccactagttctagagcggccgccaccgcggtggaattctcgaggtcctctccaaatgaaatgaacttccttatatagaggaagggtcttgcgaaggatagtgggattgtgcgtcatcccttacgtcagtggagatatcacatcaatccacttgctttgaagacgtggttggaacgtcttctttttccacgatgttcctcgtgggtgggggtccatctttgggaccactgtcggtagaggcatcttgaacgatagcctttcctttatcgcaatgatggcatttgtagaagccatcttccttttctactgtcctttcgatgaagtgacagatagctgggcaatggaatccgaggaggtttcccgatattaccctttgttgaaaagtctcaatagccctctggtcttctgagactgtatctttgatattcttggagtagacgagagtgtcgtgctccaccatgtatcacatcaatccacttgctttgaagacgtggttggaacgtcttctttttccacgatgttcctcgtgggtgggggtccatctttgggaccactgtcggtagaggcatcttgaacgatagcctttcctttatcgcaatgatggcatttgtagaagccatcttccttttctactgtcctttcgatgaagtgacagatagctgggcaatggaatccgaggaggtttcccgatattaccctttgttgaaaagtctcaatagccctctggtcttctgaacctgcatagtaaggccttaagggccagatcttgggcccttagtgtatgcgaagtgtaaaggacgcttgcgtgtatgcgtagttagtgttgggtcgatggcctacctttggcgattattgggcccggtacccgatcagattgtcgtttcccgccttcggtttaaactatcagtgtttgacaggatatattggcgggtaaacctaagagaaaagagcgtttattagaataatcggatatttaaaagggcgtgaaaaggtttatccgttcgtccatttgtatgtgcatgccaaccacagggttcccctcgggagtgcttggcattccgtgcgataatgacttctgttcaaccacccaaacgtcggaaagcctgacgacggagcagcattccaaaaagatcccttggctcgtctgggtcggctagaaggtcgagtgggctgctgtggcttgatccctcaacgcggtcgcggacgtagcgcagcgccgaaaaatcctcgatcgcaaatccgacgctgtcgaaaagcgtgatctgcttgtcgctctttcggccgacgtcctggccagtcatcacgcgccaaagttccgtcacaggatgatctggcgcgagttgctggatctcgccttcaatccgggtctgtggcgggaactccacgaaaatatccgaacgcagcaagatatcgcggtgcatctcggtcttgcctgggcagtcgccgccgacgccgttgatgtggacgccg

SEQ ID NO: 6 - DNA, 4801 bp, Zea mays
cacagcctcacacagacaccaacgccactgcactgcaaaagcaagagcagctagctagtaaagatgctgagcgggatcatcgacgggctgacgggggcgaacaagcatgcgcggctcaagggcacggtggtgctcatgcgcaagaacgtgctggacctcaacgacttcggcgccaccgtcgttgacagcatcagcgagttcctcggcaagggggtcacctgccagctcatcagctccaccctcgtcgacgccagtgagtaccgcgccgcgccgccggcacctctccgatctgcgcttccccatgtcgatcgatctcgatctctctaggctctagagctatagctctctcggcccccactttttacctttgcaagcattttccctgcatgcgaaacaagcgatagtttactatttgggcggccatgctgctgctgcttcggctaccttgcctccgtcatctttgacgggacatggaaagaaagaaagaatagagagagagacagagagagagagagagcaaacaccgagaaaaagacagcaaagctagttgtagcctgggcgcagaacacagcaccagatgctggctagctcgtgacaaagtaaaaaaagagaggaacgaacacagtagtaccaagagatcagggacgagacctttctactttgaactggattatatattggattctttatcagtaacttactgctgctagtatacccctaccctagtctcggggcgacgtgcctgcgtgcatgcccgacgcgtacgaaacacatcgacggactcacatgggccaccgcgcgcgcgcgtgcctgctttaactttcgctgtgcagacaacggcaaccgcgggcgggtcggggcggaggcgaacctggagcagtggctgacgagcctgccgtcgctgacgaccggcgagtccaagttcggcgtcacgttcgactgggaggtggagaagctgggagtgccgggggccgtcgtcgtcaagaacaaccacgccgccgagttcttcctcaagacaatcaccctcgacgacgtgcccggccgcggcgccgtcaccttcgtcgccaactcctgggtctaccccgcgggcaagtaccgctacaaccgcgtcttcttctccaacgatgtgagtcctttctcgatagatcattatgtttgtttgttattttgtttcttggtatcatgtaggcatgtagctagccgccatgtcgtcagttggagtgcagtaggtaggaaaaaggacgacatgggatgggagtggttaagaaaatccatgcaagtgggactagtgtgtaactggtagtatagctgaagaatctagtggtagaatgatcttgtacgtgaataatgtttctgacgctgagcgctgaggctatccgcaaccgttaaccctaaatttttccctctatatcattttttcctctattttcctccctattttttcatctcccgcagcggttccccctaaatactccccctatatctcactaccactataaaatattattttctataccaattatcaattttttatctactaacaattactcgtggacccacagcacagtgtttagggtgatgaacagtgacacgctagatctgaagggagagagaaggggaccgacacgtagggagcctgtagagggcaccgctgcggccgtagggtgctccctacgcgccgcatacaaggggaggggggagaggcagcggtaaccgctgcgcacagcctgagggcgaggcatgtgagttcaccacgtgagtagcagcaaaaggaaacaacccttcttcacccggctatcatctaacgtatcgccccgggagaatcaataactctaacgagatgacgaaaagtcaaaaataaagtcgtgtgatggccatgaaagtcagtcaagcaaatcagctgctaacacgtgtcccttatctacaggtgtaagagagtagagtcttgtcaatcaacctgggttgttttctatctgcgttttaccgtccgtcagtcagtcggccaacatgccacgctgatctttctgtcttttggtgccgccccgattccgaacggcggcgcagacgtacctgccaagccagatgccggcggcgctgaagccgtaccgcgacgacgagctccgcaacctccgcggcgacgaccagcagggcccctaccaggagcacgaccgcgtgtaccgctacgacgtctacaacgacctcggcgagcccgacggcggcaacccgcgccccatcctcggcggctccgccgaccacccgtacccgcgccgctgccgcacgggccgcaagcccaccaaaaccggtgcgtgcgccgtgcgcggctcttctatcttctcggacgcaacatttgctgcagggcagagaggttgttgacgctgacctgtgaccgcatcgcagaccccaactcggagagccgactgtcgctggtggagcagatctacgtgccgcgggacgagcgcttcggccacctcaagatgtccgacttcctgggctactccatcaaggccatcacgcagggcatcatcccggcggtgcgcacgtacgtggacaccaccccgggcgagttcgactccttccaggacatcatcaacctgtacgagggcgggatcaagctgcccaagatccaggcgctcgaggacatgcgcaagctcttcccgctccagctcgtcaaggacctcctccccgccggcggggactacctgctcaagctccccatcccacagatcatccaaggcacgtcacgtataccgatcgatgtcaggggccggctgttgtctggtctgcatatatatatgtgctcctatggttaactgtgactgcgtacgtttcgcggaacagaggacaagaacgcgtggaggaccgacgaggagttcgcgcgggaggtgctcgccggcgtcaacccgatggtgatcacgcgcctcacggtgagtcactcactttgtgcaaaatgcgagacccgacccgagacggaatgtgcctgacgcgctcgatttacaggagttcccgcccaagagcacgctggaccccagcaagtacggcgaccacaccagcacgatcacggcggagcacatcgagaagaacctcgagggcctcacggtgcagcaggcgctggacggcaacaggctctacatcctggaccaccacgaccgcttcatgccgttcctcatcgacgtcaacaacctggagggcaacttcatctacgccaccaggacgctcttcttcctgcgcggcgacggcaggctcgcgcccctcgccatcgagctcagcgagccgtacatcgacggggacctcaccgtggccaagagcaaggtctacacgccggcgtccagcggcgtcgaggcctgggtgtggcagctcgccaaggcctatgtcgccgtcaacgactctggctggcaccaactcgtcagccactggtacgtacgaagaactacaactactcctatatatgtcctatatgacaatggcatcgcatcgtgtcatgtctatgacatcgccaaatgcatgcgttgatggtcatgatctattctctgcgtgcgtgcaggctgaacacccacgcggtgatggagccgttcgtgatcgcgacgaaccggcagctgagcgtgacgcacccggtgcacaagctcctgagctcgcacttccgcgacaccatgaccatcaacgcgctggcgcggcagacgctcatcaacggcggcggcatcttcgagatgaccgtcttcccgggcaagtacgcgctgggcatgtcctccgtggtgtacaagagctggaacttcaccgagcagggcctccccgccgacctcgtcaagaggggcgtggcggtggcggacccgtccagcccgtacaaggtgcggctgctgatcgaggactacccgtacgcgagcgacgggctggccatctggcacgccatcgagcagtgggtgggcgagtacctggccatctactaccccgacgacggcgcgctgcggggcgacgaggagctgcaggcgtggtggaaggaggtgcgcgaggtcgggcacggcgaccacaaggacgcgccctggtggcccaagatgcaggccgtgtcggagctcgccagcgcctgcaccaccatcatctggatcgcgtcggcgctccacgccgccgtcaacttcggccagtacccgtacgcggggtacctcccgaacaggcccacggtgagccggcgccggatgccggagcccggcagcaaggagtacgaggagctggagcgcgacccggagcgcggcttcatccacaccatcacgagccagatccagaccatcatcggcatctcgctcatcgagatcctctccaagcactcctccgacgaggtgtacctcggccagcgcgacacccccgagtggacctccgacgcccgggcgctggcggcgttcaagaggttcagcgacgcgctggtcaagatcgagggcaaggtggtgggcgagaaccgcgacccgcagctgaggaacaggaacggccccgccgagttcccctacatgctgctctatcccaacacctctgaccacagtggcgccgccgcagggctcactgccaagggcatccccaacagcatctccatctgagcgactggtaccactaccaccccaggagtgctacgtacgagctggtacatgaataagctaatataagcaatcgtgtaaacgggaagagagcggccggcacgagacggaccatgtattttgcgtaaacgtgtgggctggtgaatcgaattactaccacgtaataagtgaagtgcttgttgcaatcattggcctgccagcttcaagattcttgcagttactattct

SEQ ID NO: 7 - DNA, 2595 bp, Zea mays
atgctgagcgggatcatcgacgggctgacgggggcgaacaagcatgcgcggctcaagggcacggtggtgctcatgcgcaagaacgtgctggacctcaacgacttcggcgccaccgtcgttgacagcatcagcgagttcctcggcaagggggtcacctgccagctcatcagctccaccctcgtcgacgccaacaacggcaaccgcgggcgggtcggggcggaggcgaacctggagcagtggctgacgagcctgccgtcgctgacgaccggcgagtccaagttcggcgtcacgttcgactgggaggtggagaagctgggagtgccgggggccgtcgtcgtcaagaacaaccacgccgccgagttcttcctcaagacaatcaccctcgacgacgtgcccggccgcggcgccgtcaccttcgtcgccaactcctgggtctaccccgcgggcaagtaccgctacaaccgcgtcttcttctccaacgatacgtacctgccaagccagatgccggcggcgctgaagccgtaccgcgacgacgagctccgcaacctccgcggcgacgaccagcagggcccctaccaggagcacgaccgcgtgtaccgctacgacgtctacaacgacctcggcgagcccgacggcggcaacccgcgccccatcctcggcggctccgccgaccacccgtacccgcgccgctgccgcacgggccgcaagcccaccaaaaccgaccccaactcggagagccgactgtcgctggtggagcagatctacgtgccgcgggacgagcgcttcggccacctcaagatgtccgacttcctgggctactccatcaaggccatcacgcagggcatcatcccggcggtgcgcacgtacgtggacaccaccccgggcgagttcgactccttccaggacatcatcaacctgtacgagggcgggatcaagctgcccaagatccaggcgctcgaggacatgcgcaagctcttcccgctccagctcgtcaaggacctcctccccgccggcggggactacctgctcaagctccccatcccacagatcatccaagaggacaagaacgcgtggaggaccgacgaggagttcgcgcgggaggtgctcgccggcgtcaacccgatggtgatcacgcgcctcacggagttcccgcccaagagcacgctggaccccagcaagtacggcgaccacaccagcacgatcacggcggagcacatcgagaagaacctcgagggcctcacggtgcagcaggcgctggacggcaacaggctctacatcctggaccaccacgaccgcttcatgccgttcctcatcgacgtcaacaacctggagggcaacttcatctacgccaccaggacgctcttcttcctgcgcggcgacggcaggctcgcgcccctcgccatcgagctcagcgagccgtacatcgacggggacctcaccgtggccaagagcaaggtctacacgccggcgtccagcggcgtcgaggcctgggtgtggcagctcgccaaggcctatgtcgccgtcaacgactctggctggcaccaactcgtcagccactggctgaacacccacgcggtgatggagccgttcgtgatcgcgacgaaccggcagctgagcgtgacgcacccggtgcacaagctcctgagctcgcacttccgcgacaccatgaccatcaacgcgctggcgcggcagacgctcatcaacggcggcggcatcttcgagatgaccgtcttcccgggcaagtacgcgctgggcatgtcctccgtggtgtacaagagctggaacttcaccgagcagggcctccccgccgacctcgtcaagaggggcgtggcggtggcggacccgtccagcccgtacaaggtgcggctgctgatcgaggactacccgtacgcgagcgacgggctggccatctggcacgccatcgagcagtgggtgggcgagtacctggccatctactaccccgacgacggcgcgctgcggggcgacgaggagctgcaggcgtggtggaaggaggtgcgcgaggtcgggcacggcgaccacaaggacgcgccctggtggcccaagatgcaggccgtgtcggagctcgccagcgcctgcaccaccatcatctggatcgcgtcggcgctccacgccgccgtcaacttcggccagtacccgtacgcggggtacctcccgaacaggcccacggtgagccggcgccggatgccggagcccggcagcaaggagtacgaggagctggagcgcgacccggagcgcggcttcatccacaccatcacgagccagatccagaccatcatcggcatctcgctcatcgagatcctctccaagcactcctccgacgaggtgtacctcggccagcgcgacacccccgagtggacctccgacgcccgggcgctggcggcgttcaagaggttcagcgacgcgctggtcaagatcgagggcaaggtggtgggcgagaaccgcgacccgcagctgaggaacaggaacggccccgccgagttcccctacatgctgctctatcccaacacctctgaccacagtggcgccgccgcagggctcactgccaagggcatccccaacagcatctccatctga

SEQ ID NO: 8 - protein, 864 aa, Zea mays
MLSGIIDGLTGANKHARLKGTVVLMRKNVLDLNDFGATVVDSISEFLGKGVTCQLISSTLVDANNGNRGRVGAEANLEQWLTSLPSLTTGESKFGVTFDWEVEKLGVPGAVVVKNNHAAEFFLKTITLDDVPGRGAVTFVANSWVYPAGKYRYNRVFFSNDTYLPSQMPAALKPYRDDELRNLRGDDQQGPYQEHDRVYRYDVYNDLGEPDGGNPRPILGGSADHPYPRRCRTGRKPTKTDPNSESRLSLVEQIYVPRDERFGHLKMSDFLGYSIKAITQGIIPAVRTYVDTTPGEFDSFQDIINLYEGGIKLPKIQALEDMRKLFPLQLVKDLLPAGGDYLLKLPIPQIIQEDKNAWRTDEEFAREVLAGVNPMVITRLTEFPPKSTLDPSKYGDHTSTITAEHIEKNLEGLTVQQALDGNRLYILDHHDRFMPFLIDVNNLEGNFIYATRTLFFLRGDGRLAPLAIELSEPYIDGDLTVAKSKVYTPASSGVEAWVWQLAKAYVAVNDSGWHQLVSHWLNTHAVMEPFVIATNRQLSVTHPVHKLLSSHFRDTMTINALARQTLINGGGIFEMTVFPGKYALGMSSVVYKSWNFTEQGLPADLVKRGVAVADPSSPYKVRLLIEDYPYASDGLAIWHAIEQWVGEYLAIYYPDDGALRGDEELQAWWKEVREVGHGDHKDAPWWPKMQAVSELASACTTIIWIASALHAAVNFGQYPYAGYLPNRPTVSRRRMPEPGSKEYEELERDPERGFIHTITSQIQTIIGISLIEILSKHSSDEVYLGQRDTPEWTSDARALAAFKRFSDALVKIEGKVVGENRDPQLRNRNGPAEFPYMLLYPNTSDHSGAAAGLTAKGIPNSISI

SEQ ID NO: 9 - DNA, 4150 bp, Zea mays
atgctgagcgggatcatcgacgggctgacgggggcgaacaagcatgcgcggctcaagggcacggtggtgctcatgcgcaagaacgtgctggacctcaacgacttcggcgccaccgtcgttgacagcatcagcgagttcctcggcaagggggtcacctgccagctcatcagctccaccctcgtcgacgccagtgagtaccgcgccgcgccgccggcacctctccgatctgcgcttccccatgtcgatcgatctcgatctctctaggctctagagctatagctctctcggcccccactttttacctttgcaagcattttccctgcatgcgaaacaagcgatagtttactatttgggcggccatgctgctgctgcttcggctaccttgcctccgtcatctttgacgggacatggaaagaaagaaagaatagagagagagacagagagagagagagagcaaacaccgagaaaaagacagcaaagctagttgtagcctgggcgcagaacacagcaccagatgctggctagctcgtgacaaagtaaaaaaagagaggaacgaacacagtagtaccaagagatcagggacgagacctttctactttgaactggattatatattggattctttatcagtaacttactgctgctagtatacccctaccctagtctcggggcgacgtgcctgcgtgcatgcccgacgcgtacgaaacacatcgacggactcacatgggccaccgcgcgcgcgcgtgcctgctttaactttcgctgtgcagacaacggcaaccgcgggcgggtcggggcggaggcgaacctggagcagtggctgacgagcctgccgtcgctgacgaccggcgagtccaagttcggcgtcacgttcgactgggaggtggagaagctgggagtgccgggggccgtcgtcgtcaagaacaaccacgccgccgagttcttcctcaagacaatcaccctcgacgacgtgcccggccgcggcgccgtcaccttcgtcgccaactcctgggtctaccccgcgggcaagtaccgctacaaccgcgtcttcttctccaacgatgtgagtcctttctcgatagatcattatgtttgtttgtttattggtatcatgtagctagccgccatgtcgtcagttggagtgcagtaggtaggaaaaaggacgacatgggatgggagtggttaagaaaatccatgcaagtgggactagtgtgtaactggtagtatagctgaagaatctagtggtagaatgatcttgtacgtgaataatgtttctgacgctgatcgctgagggcgaggcatgtgagttcaccacgtgagtagcagcaaaaggaaacaaccttcttcacccggctatcatctaacgtatcgccccgggagaatcaataactttattaacgagatgacgaaaagtcaaaaaaaaaaagtcgtgtgatggccatgatagtcagtcaagcaaatcagcgtccaacacgtgtcccttatctacaggtgtaagagagtagagtcttgtcaatcaacctgggttgttttctatctgcgttttaccgtccgtcagtcagtcggccaacatgccacgctgatctttctgtcttttggtgccgccccgattccgaacggcggcgcagacgtacctgccaagccagatgccggcggcgctgaagccgtaccgcgacgacgagctccgcaacctccgcggcgacgaccagcagggcccctaccaggagcacgaccgcgtgtaccgctacgacgtctacaacgacctcggcgagcccgacggcggcaacccgcgccccatcctcggcggctccgccgagcacccgtacccgcgccgctgccgcacgggccgcaagcccaccaagaccggtgcgtgcgccgtgcgcggctcttctatcttctcggacgcaacatttgctgcagggcagagaggttgttgacgctgacctgtgaccgcatcgcagaccccaactcggagagccggctgtcgctggtggagcagatctacgtgccgcgggacgagcgcttcggccacctcaagatgtccgacttcctgggctactccatcaaggccatcacgcagggcatcatcccggcggtgcgcacgtacgtggacaccaccccgggcgagttcgactccttccaggacatcatcaacctgtacgagggcgggatcaagctgcccaagatccaggcgctcgaggacatgcgcaagctcttcccgctccagctcgtcaaggacctcctccccgcaggcggggactacctgctcaagctccccatcccacagatcatccaaggcacgtcaggggccgggccggctgtctggtctgcatatatatatgtgctcctatggttaactgactgcgtacgtttcgcggaacagaggacaagaatgcgtggaggaccgacgaggagttcgcgcgggaggtgctcgccggcgtcaacccgatggtgatcacgcgcctcacagtaagtcactcactttgtgcaaaatgcgagaccagactcccgagacggaacgtgcctgacgagctcgatttacaggagttcccgcccaagagcacgctggaccccagcaagtacggcgaccacaccagcaccatcacggcggagcacatcgagaagaacctcgagggcctcacggtgcagcaggcgctggacggcaacaggctctacatcctggaccaccacgaccgcttcatgccgttcctcatcgacgtcaacaacctggagggcaacttcatctacgccaccaggacgctcttcttcctgcgcggcgacggcaggctcgcgcccctcgccatcgagctcagcgagccgtacatcgacggggacctcaccgtggccaagagcaaggtctacacgccggcgtccagcggcgtcgaggcctgggtgtggcagctcgccaaggcctatgtcgccgtcaacgactctggctggcaccaactcgtcagccactggtacgtacgaaagaactacaaccactcctatgtcctatatgacaatggcatcgcatcgtgtcatgtgtcgtgtctatgtcatcgccaaatgcatgcgtttcctggtcaaccgccgtccggtgatatgatctattctctgcgtgcgtgcatgcaggctgaacacgcacgcggtgatggagccgttcgtgatcgcgacgaaccggcagctgagcgtgacgcacccggtgcacaagctcctgagctcgcacttccgcgacaccatgaccatcaacgcgctggcgcggcagacgctcatcaacggcggcggcatcttcgagatgaccgtcttcccgggcaagtacgcgctgggcatgtcctccgtggtgtacaagagctggaacttcaccgagcagggcctccccgccgacctcgtcaagaggggcgtggcggtggcggacccgtccagcccgtacaaggtgcggctgctgatcgaggactacccgtacgcgagcgacgggctggccatctggcacgccatcgagcagtgggtgggcgagtacctggccatctactaccccgacgacggcgcgctgcggggcgacgaggagctgcaggcgtggtggaaggaggtgcgcgaggtcgggcacggcgaccacaaggacgcgccctggtggcccaagatgcaggccgtgtcggagctcgccagcgcctgcaccaccatcatctggatcgcgtcggcgctccacgccgccgtcaacttcggccagtacccgtacgcggggtacctcccgaacaggcccacggtgagccggcgccggatgccggagcccggcagcaaggagtacgaggagctggagcgcgacccggagcgcgccttcatccacaccatcacgagccagatccagaccatcatcggcatctcgctcatcgagatcctctccaagcactcctccgacgaggtgtacctcggccagcgcgacacccccgagtggacctccgacgcccgggcgctggcggcgttcaagaggttcagcgacgcgctggtcaagatcgagggcaaggtggtgggcgagaaccgcgacccgcagctgaggaacaggaacggccccgccgagttcccctacatgctgctctaccccaacacctctgaccacagtggcgccgccgcagggctcactgccaagggcatccccaacagcatctccatctga

SEQ ID NO: 10 - DNA, 2595 bp, Zea mays
atgctgagcgggatcatcgacgggctgacgggggcgaacaagcatgcgcggctcaagggcacggtggtgctcatgcgcaagaacgtgctggacctcaacgacttcggcgccaccgtcgttgacagcatcagcgagttcctcggcaagggggtcacctgccagctcatcagctccaccctcgtcgacgccaacaacggcaaccgcgggcgggtcggggcggaggcgaacctggagcagtggctgacgagcctgccgtcgctgacgaccggcgagtccaagttcggcgtcacgttcgactgggaggtggagaagctgggagtgccgggggccgtcgtcgtcaagaacaaccacgccgccgagttcttcctcaagacaatcaccctcgacgacgtgcccggccgcggcgccgtcaccttcgtcgccaactcctgggtctaccccgcgggcaagtaccgctacaaccgcgtcttcttctccaacgatacgtacctgccaagccagatgccggcggcgctgaagccgtaccgcgacgacgagctccgcaacctccgcggcgacgaccagcagggcccctaccaggagcacgaccgcgtgtaccgctacgacgtctacaacgacctcggcgagcccgacggcggcaacccgcgccccatcctcggcggctccgccgagcacccgtacccgcgccgctgccgcacgggccgcaagcccaccaagaccgaccccaactcggagagccggctgtcgctggtggagcagatctacgtgccgcgggacgagcgcttcggccacctcaagatgtccgacttcctgggctactccatcaaggccatcacgcagggcatcatcccggcggtgcgcacgtacgtggacaccaccccgggcgagttcgactccttccaggacatcatcaacctgtacgagggcgggatcaagctgcccaagatccaggcgctcgaggacatgcgcaagctcttcccgctccagctcgtcaaggacctcctccccgcaggcggggactacctgctcaagctccccatcccacagatcatccaagaggacaagaatgcgtggaggaccgacgaggagttcgcgcgggaggtgctcgccggcgtcaacccgatggtgatcacgcgcctcacagagttcccgcccaagagcacgctggaccccagcaagtacggcgaccacaccagcaccatcacggcggagcacatcgagaagaacctcgagggcctcacggtgcagcaggcgctggacggcaacaggctctacatcctggaccaccacgaccgcttcatgccgttcctcatcgacgtcaacaacctggagggcaacttcatctacgccaccaggacgctcttcttcctgcgcggcgacggcaggctcgcgcccctcgccatcgagctcagcgagccgtacatcgacggggacctcaccgtggccaagagcaaggtctacacgccggcgtccagcggcgtcgaggcctgggtgtggcagctcgccaaggcctatgtcgccgtcaacgactctggctggcaccaactcgtcagccactggctgaacacgcacgcggtgatggagccgttcgtgatcgcgacgaaccggcagctgagcgtgacgcacccggtgcacaagctcctgagctcgcacttccgcgacaccatgaccatcaacgcgctggcgcggcagacgctcatcaacggcggcggcatcttcgagatgaccgtcttcccgggcaagtacgcgctgggcatgtcctccgtggtgtacaagagctggaacttcaccgagcagggcctccccgccgacctcgtcaagaggggcgtggcggtggcggacccgtccagcccgtacaaggtgcggctgctgatcgaggactacccgtacgcgagcgacgggctggccatctggcacgccatcgagcagtgggtgggcgagtacctggccatctactaccccgacgacggcgcgctgcggggcgacgaggagctgcaggcgtggtggaaggaggtgcgcgaggtcgggcacggcgaccacaaggacgcgccctggtggcccaagatgcaggccgtgtcggagctcgccagcgcctgcaccaccatcatctggatcgcgtcggcgctccacgccgccgtcaacttcggccagtacccgtacgcggggtacctcccgaacaggcccacggtgagccggcgccggatgccggagcccggcagcaaggagtacgaggagctggagcgcgacccggagcgcgccttcatccacaccatcacgagccagatccagaccatcatcggcatctcgctcatcgagatcctctccaagcactcctccgacgaggtgtacctcggccagcgcgacacccccgagtggacctccgacgcccgggcgctggcggcgttcaagaggttcagcgacgcgctggtcaagatcgagggcaaggtggtgggcgagaaccgcgacccgcagctgaggaacaggaacggccccgccgagttcccctacatgctgctctaccccaacacctctgaccacagtggcgccgccgcagggctcactgccaagggcatccccaacagcatctccatctga

SEQ ID NO: 11 - protein, 864 aa, Zea mays
MLSGIIDGLTGANKHARLKGTVVLMRKNVLDLNDFGATVVDSISEFLGKGVTCQLISSTLVDANNGNRGRVGAEANLEQWLTSLPSLTTGESKFGVTFDWEVEKLGVPGAVVVKNNHAAEFFLKTITLDDVPGRGAVTFVANSWVYPAGKYRYNRVFFSNDTYLPSQMPAALKPYRDDELRNLRGDDQQGPYQEHDRVYRYDVYNDLGEPDGGNPRPILGGSAEHPYPRRCRTGRKPTKTDPNSESRLSLVEQIYVPRDERFGHLKMSDFLGYSIKAITQGIIPAVRTYVDTTPGEFDSFQDIINLYEGGIKLPKIQALEDMRKLFPLQLVKDLLPAGGDYLLKLPIPQIIQEDKNAWRTDEEFAREVLAGVNPMVITRLTEFPPKSTLDPSKYGDHTSTITAEHIEKNLEGLTVQQALDGNRLYILDHHDRFMPFLIDVNNLEGNFIYATRTLFFLRGDGRLAPLAIELSEPYIDGDLTVAKSKVYTPASSGVEAWVWQLAKAYVAVNDSGWHQLVSHWLNTHAVMEPFVIATNRQLSVTHPVHKLLSSHFRDTMTINALARQTLINGGGIFEMTVFPGKYALGMSSVVYKSWNFTEQGLPADLVKRGVAVADPSSPYKVRLLIEDYPYASDGLAIWHAIEQWVGEYLAIYYPDDGALRGDEELQAWWKEVREVGHGDHKDAPWWPKMQAVSELASACTTIIWIASALHAAVNFGQYPYAGYLPNRPTVSRRRMPEPGSKEYEELERDPERAFIHTITSQIQTIIGISLIEILSKHSSDEVYLGQRDTPEWTSDARALAAFKRFSDALVKIEGKVVGENRDPQLRNRNGPAEFPYMLLYPNTSDHSGAAAGLTAKGIPNSISI

SEQ ID NO: 12 - DNA, 4108 bp, Zea mays
  misc_feature (378)..(388): n is a, c, g, or t
atgctgagcgggatcatcgacgggctgacgggggcgaacaagcatgcgcggctcaagggcacggtggtgctcatgcgcaagaacgtgctggacctcaacgacttcggcgccaccgtcgttgacagcatcagcgagttcctcggcaagggggtcacctgccagctcatcagctccaccctcgtcgacgccagtgagtaccgcgccgcgccgccggcacctctccgatctgcgcttccccatgtcgatcgatctcgatctctctaggctctagagctatagctctctcggcccccactttttacctttgcaagcattttccctgcatgcgaaacaagcgatagtttactatttgggcggccatgctgctgctgcttcggnnnnnnnnnnnaatagagagagagacagagagagagagagagagagagagcaaacaccgagaaaaagacagcaaagctagttgtagcctgggcgcagaacacagcaccagatgctggctagctcgtgacaaagtaaaaaaagagaggaacgaacacagtagtaccaagagatcagggacgagacctttctactttgaactggattatatattggattctttatcagtaacttactgctgctagtatacccctaccctagtctcggggcgacgtgcctgcgtgcatgcccgacgcgtacgaaacacatcgacggactcacatgggccaccgcgcgcgcgcgtgcctgctttaactttcgctgtgcagacaacggcaaccgcgggcgggtcggggcggaggcgaacctggagcagtggctgacgagcctgccgtcgctgacgaccggcgagtccaagttcggcgtcacgttcgactgggaggtggagaagctgggagtgccgggggccgtcgtcgtcaagaacaaccacgccgccgagttcttcctcaagacaatcaccctcgacgacgtgcccggccgcggcgccgtcaccttcgtcgccaactcctgggtctaccccgcgggcaagtaccgctacaaccgcgtcttcttctccaacgatgtgagtcctttctcgatagatcattatgtttgtttgtttattggtatcatgtagctagccgccatgtcgtcagttggagtgcagtaggtaggaaaaaggacgacatgggatgggagtggttaagaaaatccatgcaagtgggactagtgtgtaactggtagtatagctgaagaatctagtggtagaatgatcttgtacgtgaataatgtttctgacgctgagcgctgagggcgaggcatgtgagttcaccacgtgagtagcagcaaaaggaaacgacccttcttcacccggctatcatctaacgtatcgccccgggagaatcaataactttaacgagatgacgaaaagtcaaaaataaagtcgtgtgatggccatgaaagtcagtcaagcaaatcagctgctaacacgtgtcccttatctacaggtgtaagagtagagtcttgtcaatcaacctgggttgttttctatctgcgttttaccgtccgtcagtcagtcggccaacatgccacgctgatctttctgtcttttggtgccgccccgattccgaacggcggcgcagacgtacctgccaagccagatgccggcggcgctgaagccgtaccgcgacgacgagctccgcaacctccgcggcgacgaccagcagggcccctaccaggagcacgaccgcgtgtaccgctacgacgtctacaacgacctcggcgagcccgacggcggcaacccgcgccccatcctcggcggctccgccgaccacccgtacccgcgccgctgccgcacgggccgcaagcccaccaaaaccggtgcgtgcgccgtgcgcggctcttctatcttctcggacgcaacatttgctgcagggcagagaggttgttgacgctgacctgtgaccgcatcgcagaccccaactcggagagccgactgtcgctggtggagcagatctacgtgccgcgggacgagcgcttcggccacctcaagatgtccgacttcctgggctactccatcaaggccatcacgcagggcatcatcccggcggtgcgcacgtacgtggacaccaccccgggcgagttcgactccttccaggacatcatcaacctgtacgagggcgggatcaagctgcccaagatccaggcgctcgaggacatgcgcaagctcttcccgctccagctcgtcaaggacctcctccccgccggcggggactacctgctcaagctccccatcccacagatcatccaaggcacgtcacgtataccgatcgatgtcaggggccggctgttgtctggtctgcatatatatatgtgctcctatggttaactgtgactgcgtacgtttcgcggaacagaggacaagaacgcgtggaggaccgacgaggagttcgcgcgggaggtgctcgccggcgtcaacccgatggtgatcacgcgcctcacggtgagtcactcactttgtgcaaaatgcgagacccgacccgagacggaatgtgcctgacgcgctcgatttacaggagttcccgcccaagagcacgctggaccccagcaagtacggcgaccacaccagcacgatcacggcggagcacatcgagaagaacctcgagggcctcacggtgcagcaggcgctggacgccaacaggctctacatcctggaccaccacgaccgcttcatgccgttcctcatcgacgtcaacaacctggagggcaacttcatctacgccaccaggacgctcttcttcctgcgcggcgacggcaggctcgcgcccctcgccatcgagctcagcgagccgtacatcgacggggacctcaccgtggccaagagcaaggtctacacgccggcgtccagcggcgtcgaggcctgggtgtggcagctcgccaaggcctatgtcgccgtcaacgactctggctggcaccaactcgtcagccactggtacgtacgaagaactacaactactcctatatatgtcctatatgacaatggcatcgcatcgtgtcatgtctatgacatcgccaaatgcatgcgttgatggtcatgatctattctctgcgtgcgtgcaggctgaacacccacgcggtgatggagccgttcgtgatcgcgacgaaccggcagctgagcgtgacgcacccggtgcacaagctcctgagctcgcacttccgcgacaccatgaccatcaacgcgctggcgcggcagacgctcatcaacggcggcggcatcttcgagatgaccgtcttcccgggcaagtacgcgctgggcatgtcctccgtggtgtacaagagctggaacttcaccgagcagggcctccccgccgacctcgtcaagaggggcgtggcggtggcggacccgtccagcccgtacaaggtgcggctgctgatcgaggactacccgtacgcgagcgacgggctggccatctggcacgccatcgagcagtgggtgggcgagtacctggccatctactaccccgacgacggcgcgctgcggggcgacgaggagctgcaggcgtggtggaaggaggtgcgcgaggtcgggcacggcgaccacaaggacgcgccctggtggcccaagatgcaggccgtgtcggagctcgccagcgcctgcaccaccatcatctggatcgcgtcggcgctccacgccgccgtcaacttcggccagtacccgtacgcggggtacctcccgaacaggcccacggtgagccggcgccggatgccggagcccggcagcaaggagtacgaggagctggagcgcgacccggagcgcgccttcatccacaccatcacgagccagatccagaccatcatcggcatctcgctcatcgagatcctctccaagcactcctccgacgaggtgtacctcggccagcgcgacacccccgagtggacctccgacgcccgggcgctggcggcgttcaagaggttcagcgacgcgctggtcaagatcgagggcaaggtggtgggcgagaaccgcgacccgcagctgaggaacaggaacggccccgccgagttcccctacatgctgctctaccccaacacctctgaccacagtggcgccgccgcagggctcactgccaagggcatccccaacagcatctccatctga

SEQ ID NO: 13 - DNA, 2595 bp, Zea mays
atgctgagcgggatcatcgacgggctgacgggggcgaacaagcatgcgcggctcaagggcacggtggtgctcatgcgcaagaacgtgctggacctcaacgacttcggcgccaccgtcgttgacagcatcagcgagttcctcggcaagggggtcacctgccagctcatcagctccaccctcgtcgacgccaacaacggcaaccgcgggcgggtcggggcggaggcgaacctggagcagtggctgacgagcctgccgtcgctgacgaccggcgagtccaagttcggcgtcacgttcgactgggaggtggagaagctgggagtgccgggggccgtcgtcgtcaagaacaaccacgccgccgagttcttcctcaagacaatcaccctcgacgacgtgcccggccgcggcgccgtcaccttcgtcgccaactcctgggtctaccccgcgggcaagtaccgctacaaccgcgtcttcttctccaacgatacgtacctgccaagccagatgccggcggcgctgaagccgtaccgcgacgacgagctccgcaacctccgcggcgacgaccagcagggcccctaccaggagcacgaccgcgtgtaccgctacgacgtctacaacgacctcggcgagcccgacggcggcaacccgcgccccatcctcggcggctccgccgaccacccgtacccgcgccgctgccgcacgggccgcaagcccaccaaaaccgaccccaactcggagagccgactgtcgctggtggagcagatctacgtgccgcgggacgagcgcttcggccacctcaagatgtccgacttcctgggctactccatcaaggccatcacgcagggcatcatcccggcggtgcgcacgtacgtggacaccaccccgggcgagttcgactccttccaggacatcatcaacctgtacgagggcgggatcaagctgcccaagatccaggcgctcgaggacatgcgcaagctcttcccgctccagctcgtcaaggacctcctccccgccggcggggactacctgctcaagctccccatcccacagatcatccaagaggacaagaacgcgtggaggaccgacgaggagttcgcgcgggaggtgctcgccggcgtcaacccgatggtgatcacgcgcctcacggagttcccgcccaagagcacgctggaccccagcaagtacggcgaccacaccagcacgatcacggcggagcacatcgagaagaacctcgagggcctcacggtgcagcaggcgctggacgccaacaggctctacatcctggaccaccacgaccgcttcatgccgttcctcatcgacgtcaacaacctggagggcaacttcatctacgccaccaggacgctcttcttcctgcgcggcgacggcaggctcgcgcccctcgccatcgagctcagcgagccgtacatcgacggggacctcaccgtggccaagagcaaggtctacacgccggcgtccagcggcgtcgaggcctgggtgtggcagctcgccaaggcctatgtcgccgtcaacgactctggctggcaccaactcgtcagccactggctgaacacccacgcggtgatggagccgttcgtgatcgcgacgaaccggcagctgagcgtgacgcacccggtgcacaagctcctgagctcgcacttccgcgacaccatgaccatcaacgcgctggcgcggcagacgctcatcaacggcggcggcatcttcgagatgaccgtcttcccgggcaagtacgcgctgggcatgtcctccgtggtgtacaagagctggaacttcaccgagcagggcctccccgccgacctcgtcaagaggggcgtggcggtggcggacccgtccagcccgtacaaggtgcggctgctgatcgaggactacccgtacgcgagcgacgggctggccatctggcacgccatcgagcagtgggtgggcgagtacctggccatctactaccccgacgacggcgcgctgcggggcgacgaggagctgcaggcgtggtggaaggaggtgcgcgaggtcgggcacggcgaccacaaggacgcgccctggtggcccaagatgcaggccgtgtcggagctcgccagcgcctgcaccaccatcatctggatcgcgtcggcgctccacgccgccgtcaacttcggccagtacccgtacgcggggtacctcccgaacaggcccacggtgagccggcgccggatgccggagcccggcagcaaggagtacgaggagctggagcgcgacccggagcgcgccttcatccacaccatcacgagccagatccagaccatcatcggcatctcgctcatcgagatcctctccaagcactcctccgacgaggtgtacctcggccagcgcgacacccccgagtggacctccgacgcccgggcgctggcggcgttcaagaggttcagcgacgcgctggtcaagatcgagggcaaggtggtgggcgagaaccgcgacccgcagctgaggaacaggaacggccccgccgagttcccctacatgctgctctaccccaacacctctgaccacagtggcgccgccgcagggctcactgccaagggcatccccaacagcatctccatctga

SEQ ID NO: 14 - protein, 864 aa, Zea mays
MLSGIIDGLTGANKHARLKGTVVLMRKNVLDLNDFGATVVDSISEFLGKGVTCQLISSTLVDANNGNRGRVGAEANLEQWLTSLPSLTTGESKFGVTFDWEVEKLGVPGAVVVKNNHAAEFFLKTITLDDVPGRGAVTFVANSWVYPAGKYRYNRVFFSNDTYLPSQMPAALKPYRDDELRNLRGDDQQGPYQEHDRVYRYDVYNDLGEPDGGNPRPILGGSADHPYPRRCRTGRKPTKTDPNSESRLSLVEQIYVPRDERFGHLKMSDFLGYSIKAITQGIIPAVRTYVDTTPGEFDSFQDIINLYEGGIKLPKIQALEDMRKLFPLQLVKDLLPAGGDYLLKLPIPQIIQEDKNAWRTDEEFAREVLAGVNPMVITRLTEFPPKSTLDPSKYGDHTSTITAEHIEKNLEGLTVQQALDANRLYILDHHDRFMPFLIDVNNLEGNFIYATRTLFFLRGDGRLAPLAIELSEPYIDGDLTVAKSKVYTPASSGVEAWVWQLAKAYVAVNDSGWHQLVSHWLNTHAVMEPFVIATNRQLSVTHPVHKLLSSHFRDTMTINALARQTLINGGGIFEMTVFPGKYALGMSSVVYKSWNFTEQGLPADLVKRGVAVADPSSPYKVRLLIEDYPYASDGLAIWHAIEQWVGEYLAIYYPDDGALRGDEELQAWWKEVREVGHGDHKDAPWWPKMQAVSELASACTTIIWIASALHAAVNFGQYPYAGYLPNRPTVSRRRMPEPGSKEYEELERDPERAFIHTITSQIQTIIGISLIEILSKHSSDEVYLGQRDTPEWTSDARALAAFKRFSDALVKIEGKVVGENRDPQLRNRNGPAEFPYMLLYPNTSDHSGAAAGLTAKGIPNSISI

SEQ ID NO: 15 - DNA, 20683 bp, Zea mays
  misc_feature (11321)..(11676): n is a, c, g, or t
  misc_feature (13711)..(13986): n is a, c, g, or t
  misc_feature (14689)..(14733): n is a, c, g, or t
  misc_feature (15101)..(15387): n is a, c, g, or t
  misc_feature (15987)..(16486): n is a, c, g, or t
  misc_feature (17031)..(17530): n is a, c, g, or t
atgctgagcgggatcatcgacgggctgacgggggcgaacaagcatgcgcggctcaagggcacggtggtgctcatgcgcaagaacgtgctggacctcaacgacttcggcgccaccgtcgtcgacagcatcagcgagttcctcggcaagggggtcacctgccagctcatcagctccactctcgtcgacgccagtgagtaccgcgccgccggcacctctccgatctgcgtgcgcttccccatgtcgatcgatctcgatctctctaggctctagagctatagctctctcggccgccactttttacctttgcaagcattttccccccgcatgcgaaacaagcgaataagcgatagtatactatttgggcggccatgctgctgcttcggctaccttgcctccgtcgtctttgacgggacatggaaagaaagaaagaatagcgagagagagacagagacagcgagagagagagatagagcaaacaccgagaaaaagacagcaaagctagttgtagcctgggcgcagagcacagcaccagatgctggctagctcgtgacaaagtaaaaaaaggaacgaacacagtagtgccaagagatcagggacgagacctttctactttgaactggattatatattggattctttatcagtaacttactgctgctagtatacccctaccctagtctcggggcgacgtgcctgcgtgcatgcccgacgcgtacgaaacacatcgacggactcacatgggccaccgcgcgcgcgcgtgcctgctttaactttcgctgtgcagacaacggcaaccgcgggcgggtcggggcggaggcgaacctggagcagtggctgacgagcctgccgtcgctgacgaccggcgagtccaagttcggcgtcacgttcgactgggaggtggagaagctgggagtgccgggggccgtcgtcgtcaagaacaaccacgccgccgagttcttcctcaagacaatcaccctcgacgacgtgcccggccgcggcgccgtcaccttcgtcgccaactcctgggtctaccccgcgggcaagtaccgctacaaccgcgtcttcttctccaacgatgtgagtcctttctcgatagatcattatgtttgtttgttattttgtttcttggtatcatgtaggcatgtagctagccgccatgtcgtcagttggagtgcagtaggtaggaaaaaggacgacatgggatgggagtggttaagaaaatccatgcaagtgggactagtgtgtaactggtagtatagctgaagaatctagtggtagaatgatcttgtacgtgaataatgtttctgacgctgagcgctgaggctatccgcaaccgttaaccctaaatttttccctctatatcattttttcctctattttcctccctattttttcatctcccgcagcggttccccctaaatactccccctatatcccactaccactataaaatattattttctataccaattatcaattttttatctactaacaattactcgtggacccacagcacagtgtttagggtgatgaacagtgacacgctagatctgaagggagagagaaggggaccgacacgtagggagcctgtagagggcaccgctgcggccgtagggtgctccctacgcgccgcatacaaggggaggggggagaggcagcggtaaccgctgcgcacagcctgagggcgaggcatgtgagttcaccacgtgagtagcagcaaaaggaaacaacccttcttcacccggctatcatctaacgtatcgccccgggagaatcaataactctaacgagatgacgaaaagtcaaaaataaagtcgtgtgatggccatgaaagtcagtcaagcaaatcagctgctaacacgtgtcccttatctacaggtgtaagagagtagagtcttgtcaatcaacctgggttgttttctatctgcgttttaccgtccgtcagtcagtcggccaacatgccacgctgatctttctgtcttttggtgccgccccgattccgaacggcggcgcagacgtacctgccaagccagatgccggcggcgctgaagccgtaccgcgacgacgagctccgcaacctccgcggcgacgaccagcagggcccctaccaggagcacgaccgcgtgtaccgctacgacgtctacaacgacctcggcgagcccgacggcggcaacccgcgccccatcctcggcggctccgccgaccacccgtacccgcgccgctgccgcacgggccgcaagcccaccaaaaccggtgcgtgcgccgtgcgcggctcttctatcttctcggacgcaacatttgctgcagggcagagaggttgttgacgctgacctgtgaccgcatcgcagaccccaactcggagagccgactgtcgctggtggagcagatctacgtgccgcgggacgagcgcttcggccacctcaagatgtccgacttcctgggctactccatcaaggccatcacgcagggcatcatcccggcggtgcgcacgtacgtggacaccaccccgggcgagttcgactccttccaggacatcatcaacctgtacgagggcgggatcaagctgcccaagatccaggcgctcgaggacatgcgcaagctcttcccgctccagctcgtcaaggacctcctccccgccggcggggactacctgctcaagctccccatcccacagatcatccaaggcacgtcacgtataccgatcgatgtcaggggccggctgttgtctggtctgcatatatatatgtgctcctatggttaactgtgactgcgtacgtttcgcggaacagaggacaagaacgcgtggaggaccgacgaggagttcgcgcgggaggtgctcgccggcgtcaacccgatggtgatcacgcgcctcacggtgagtcactcactttgtgcaaaatgcgagacccgacccgagacggaatgtgcctgacgcgctcgatttacaggagttcccgcccaagagcacgctggaccccagcaagtacggcgaccacaccagcacgatcacggcggagcacatcgagaagaacctcgagggcctcacggtgcagcaggcgctggacggcaacaggctctacatcctggaccaccacgaccgcttcatgccgttcctcatcgacgtcaacaacctggagggcaacttcatctacgccaccaggacgctcttcttcctgcgcggcgacggcaggctcgcgcccctcgccatcgagctcagcgagccgtacatcgacggggacctcaccgtggccaagagcaaggtctacacgccggcgtccagcggcgtcgaggcctgggtgtggcagctcgccaaggcctatgtcgccgtcaacgactctggctggcaccaactcgtcagccactggtacgtacgaagaactacaactactcctatatatgtcctatatgacaatggcatcgcatcgtgtcatgtctatgacatcgccaaatgcatgcgttgatggtcatgatctattctctgcgtgcgtgcaggctgaacacccacgcggtgatggagccgttcgtgatcgcgacgaaccggcagctgagcgtgacgcacccggtgcacaagctcctgagctcgcacttccgcgacaccatgaccatcaacgcgctggcgcggcagacgctcatcaacggcggcggcatcttcgagatgaccgtcttcccgggcaagtacgcgctgggcatgtcctccgtggtgtacaagagctggaacttcaccgagcagggcctccccgccgacctcgtcaagaggggcgtggcggtggcggacccgtccagcccgtacaaggtgcggctgctgatcgaggactacccgtacgcgagcgacgggctggccatctggcacgccatcgagcagtgggtgggcgagtacctggccatctactaccccgacgacggcgcgctgcggggcgacgaggagctgcaggcgtggtggaaggaggtgcgcgaggtcgggcacggcgaccacaaggacgcgccctggtggcccaagatgcaggccgtgtcggagctcgccagcgcctgcaccaccatcatctggatcgcgtcggcgctccacgccgccgtcaacttcggccagtacccgtacgcggggtacctcccgaacaggcccacggtgagccggcgccggatgccggagcccggcagcaaggagtacgaggagctggagcgcgacccggagcgcggcttcatccacaccatcacgagccagatccagaccatcatcggcatctcgctcatcgagatcctctccaagcactcctccgacgaggtgtacctcggccagcgcgacacccccgagtggacctccgacgcccgggcgctggcggcgttcaagaggttcagcgacgcgctggtcaagatcgagggcaaggtggtgggcgagaaccgcgacccgcagctgaggaacaggaacggccccgccgagttcccctacatgctgctctatcccaacacctctgaccacagtggcgccgccgcagggctcactgccaagggcatccccaacagcatctccatctgagcgactggtaccactaccaccccaggagtgctacgtacgagctggtacatgaataagctaatataagcaatcgtgtaaacgggaagagagcggccggcacgagacggaccatgtattttgcgtaaacgtgtgggctggtgaatcgaattactaccacgtaataagtgaagtgcttgttgcaatcattggcctgccagcttcaagattcttgcagttactattctagtcgtttcgcagtgctcctcgatcacaacatttcacgaggtgttttattacaataatttggagctattcaatttcaaagcctatgtagaatactatatgttgtagggacattagtcccacatagctaaccaaaaataaaatttaatcgatttaaatatcaacggtccagtggtcatctattaagattatgctcaacagaccatgcatgcatatgttgtgtaagattatgacaacattatttagaggtgtcttgataagtgtccttgccgaaaacatagtggattcttatatgcttttgttcactgccaaagagttgtggaatacgacaatcattgcgaaaaagggtggcatcaaagtttgccactggacacagcggaaaccaccaaggaacgataactggttttccaaagcagtggactcgcccccaaaataatcagagaactcagggcagtggaaactgctgacctcaaggtggtactagcagacgccttataaaagaaccggtagatgcaatcttctggagagagagagagagaaaaaaaaaagaagaagttgctagatggaatcgtgcaaatcttcacctaatggcgactgctaccaccgaataaaaaagaagtgcaaatcttcacctagacgttctcagaaacggcaccatgctgcagctgcgatacgaaccaggctggggcggcaggtgaagctgacacggtgccgctgctgcaccgggcgaataaataatagtactgacaataatgctaaattagaatggaacagacgacatgattagaatgatatgctctcctttgctcattttgttccacacgtgtttggtgaagccgtgcctagtatataactatatatactacgttggtacagcactaaattcccttttccccattttcagtggttggcctttcccattctgatcggcccaaagcagcgctttagcaattgactaatccgtcgacctttggcgcctagcctttcctatgggcatgtttcctatggttgcaaattccatctaaggcgcatccaaatcgtacaaagacagtagatgagctgtccgtccttcctcctctctagctgctggcgggcggggtgcacttggtgatgtcgattagttttagttttatggcctatttggttcagtctgccaggcaaagaatcctaaccctaggcactcaaaataagataatcatagtatcttaagcttgattaaatctataaaatgaaaaaaaaaacaataacttttgtaccattagatccttttattagttatgtctttatagtatacctatttgatgtcataaatctctataaatattttttataactctaatcaaaattgagatatttgggctctaaaaaaactaggataatttataattcagtttgaaaagtacaagaagataactaaactagaagagaaggacaatttccaaaaacgtaccgtggacgtacgtttcgatgctcgttacgatgtggacgctttatttgcaaatgtttcacgtgcggtgacgcgttcacgtaccataagctctatggatataatagtataatcaggcccgtttaccatgtctcctgccgccttcgactcctttttattttagcgtactgtactttgaacggattaggagctaagcgaagctacaatttagcttgtataaacctgcagccgtgtcaaactgtactagtcaaaagtcaaaagaacagttccagcgcgagcaatatggccgctgcccttctctcaacgttctgcttttggacttgtgtgatgtttggttcgtatatttaggggataagtaactgataatgttaaactatatttgtttaaattaactgtaattagatacacactataaagtgatgctgatctattcaagcttattactgttgatacttaagcgtgaatcattatcattactatttatgttataatatatgaaccaaacggcagtaccgtacagcagcaaagaagctagaacaaaattcttttctaattttttcatatagtcgagcctacgaggtatgttttctgagagaatatagattatgatagatctaagagtgtttctataataatctagccaactgccaaatacattcgtagttaatctttctagtccgcctgacattcctagtatacgtactacagtgcagggcatcttaaattcggatcaggttgccaatcatcgaaaattgtgatccacttgcgcatatgatatggtcaagacgtcaagttggatagggggggagtagtagtagttgaatgggcaagagcgcgtattttatatagacgtatagcgtcacaagccgccaggaagggaaaaaaaaatatagtgtgtgagtagcgaagaaaactctccccctctgaaaattcttgcattttgacgacatccgattcaatcattcagtagtacgtagtgtatttattttattgggatttagaaaaccagaccctgatatgatcctacgacggctggatggcagtttagtgttattcgactgtttcacgcgattactccctccgtttctttttatttgtcgctagatagtgttacactatccaacgacaaataaaaagaaacggaggaagtatttaggaagtgacgagtctagctaacccgattggttcaaatcctttcttcatcaatcaaccgttaaacggccgtgtcaatcggtgttggcgaaccgttaaaaccgtagcagccccagtggagtggggccttcttgtcgagttacacggtgttttatcctatcccgtggtcgctaacacgcacatgcctgggatgacagatgacactaacacgcacatgctcaattactactaacgcagaagtcaggtgcaattaaagagcagtaaatgcccaagtccctgttctgcttccaggacaggacaggaacactgtgatgaaacaacattcatcaggacggcacgcgaccgccgatgttcggcgacgacagctccgtaacatttcaccgctgaagcctgaagggagagggacctggcgtgcgctagcagctgctgatgacgccagccagacatggcaccacacgagacacggccgcccggttgaccggcgaagcagcccgggggtttccaagtcatcgccggtttccgcgggttcgccgtcgccagtcgccaactttggacagacagagacagtcagctcgggctctcgtctcgtccgtgctcgctctcgtctcgcatcgcacctgcgcgttgctggctcggcgtggacctggcgcggcgccggagccccgttagaaaccgcgcgtgtgcccgtgctatccatggtctcctgtaaatggtgtaatcttatcttatttaccgcatcaccattaacaatttaacacgagacgcacgacacccaagcctgtgatgccgacgtataccacaccatctaatccaaatccctgcattttttagtctctcagtcatcatcgactcatcgtttttttaatccattcacttttttttccaccttttcgtatacacgtcgctgtcgcctccatcgctgggctggcaagagaacgcgaggcgaagcagccgcggccgcccgcctatttatcgcgggctcgcggcacagggcagcggcagttccatacatacatacaccaaccgtgcgtgaaggaaggcctttgctcgccgccacatcacattggcaggcgaggcgagggagcgagcagcagggcaaggcatccacacccacacccaccggacactccctgagaagcgagaagcgagaagcgaagagcggccggccaccatgttctggcacggggtcgcggaccggctgacggggaagaacaaggaggcgtggaacgagggaaagatccgcggcacggtgaggctggtcaagaaggaggtgctggacgtcggcgacttcaacgcctcgctcctcgacggcgtacacaggatcctcggctgggacgacggcgtcgccttccagctcgtcagcgccaccgcggccgaccccagtaagcgcgaccctgcatcacgcccccctccccctacccccctatggaagattggaagtcgaccgaacgcccccgctcccggtggccgtgggccgtgaacgccggcggccgcgctcgctggagcgtgggcggaacctacgccatgcgtcggacgtgcgtttcgccgtccatttcggtttttcccctttccttacttttctctatacgaaggatacgaagaaacattttatcaaacaattccaatggatgctgatgaaaaacctgtagaatccgtgcccgtctgataaaaaaaaaaaactgcgactttgtttttctggccacccgtccatcttgacgcaagcagacaggcatgggacaggatcctcgggcgcgtaataaccgcctgcagtgtgttggtctctggtacgtgggacccgtagcgcctgggtccgtgtctcagcgacccaggcgctttttggcgttttgtgtggtagggcttgcgttttcaagtctgaactgggaactgggaaccttgtagccccggacatggaatggaacagttgtttgggggcattcaatgcgattgagatggcgtccgtgaaaactttactgtaattttcactgcaaacgattgattgactgattgattgaacgagtcttcaggcaacgggagccgcggcaaggtcgggaaggcggcgcacctggaggaggcggtggtgtcgctcaagtcgacgacggacggggagaccgtgtaccgggtgagcttcgagtgggacgggtcgcagggcgtcccgggcgccgtcctggtcaggaacctgcagcacgccgagttcttcctcaagtcgctcaccctcgagggcgtccccggcaggggcaccgtcgtcttcgtcgccaactcgtggatctacccgcacaatctctactcccaggaacgcgtcttcttcgccaacgacgtgagtattcttccccttcggtttcttttttgggttcgctggcgacgtgagtattcttactcaggatacgaaatcttgagcaatgtgacacacttgcgtgtgataaacacatccagagcttatttgctacgaaatgtggctacagagcacggatcgggtgctagtcaactattcatcattttttttaaaaactctcctaaccgttttaggttcgttctagatcaaactatttaaactttaaccaacaatacatatataaaattaaattattttgaactaaaagaattatatattattgtagttcaacttacgataaatctagtaacttttttatgttgtaaaatcttataaaatatctgatataatcagttaaagttgacactgattgacttagcataaatctaaaacgactaatttcatgtggacgaaaagagtatgtgtgtatcatgttagatatatctagatccttacgtgataagaatacgtgctctactgttagctcctttttattaatgtaaaaacctagattgggtatagatccagtttagtggacatttggttacctatgaattctgggaatgagataaactttatctgctattcaaccatacgtttgatttttctatattgggtaatgtactgtaagagagaatctcaaatactaactccattgttaaatatatgacgtcattgatttttttttaaaaaaaactttaaccactcagcttattcaataaaaaatatatattattatttactttgttataattttttttattatttaaggtaatttaagcatgaatttagatttttaaataaatattttgaataaaataagtgttcaaagttttttaaaattcaactgtatcatatattaaaaaacggatgtactatcaactttgtgctgcattttttaggtagcgtgcagacttcatgttataaaaattcaactttgtgctgcattttttgggtagtgtgcagacttcatgttataaaaattcaccgtttgagccttagctcccaaactggccagcctggtcttcgggtcaagtccacaggcggccgtacagcatcgacaaccattattgctatatactattattgtccgtactgcactatcgatcgaacacacgcacccacagacgcatcactcatgttacggatagccggcagcaatcaaagtgttcgtctggctacagtaaattcttgcgtgatttgtgtatagggccttcaccatcatttgctgatcgatccagaactggttgataggagtcagaagaaatgtaacaagtcttgtatagttctctcttggtagtccaaagaaaaggagaaatcaatacaaaggttaagtctggtacatcacagtatcatactatcacagaccgagcatcctgaagtccaaattatctcatgttgcatcatattttctttatcggacacgtaggagagctacatatcattattatcgagaaaagaatgtttttttaacatgcagaagagccatgtggctcatgttgcaccgcaatccataacaaggacgcatagatagattaacccagtgttggaagtcaaattgagcagcgcggacagtccagcgctgaggccggacggtccgcggtccggacagtccgcggtggtggcgcggacggtccgcgcgnnnnnnnnnnnnnnnnnnnnnnnnnnnnnnnnnnnnnnnnnnnnnnnnnnnnnnnnnnnnnnnnnnnnnnnnnnnnnnnnnnnnnnnnnnnnnnnnnnnnnnnnnnnnnnnnnnnnnnnnnnnnnnnnnnnnnnnnnnnnnnnnnnnnnnnnnnnnnnnnnnnnnnnnnnnnnnnnnnnnnnnnnnnnnnnnnnnnnnnnnnnnnnnnnnnnnnnnnnnnnnnnnnnnnnnnnnnnnnnnnnnnnnnnnnnnnnnnnnnnnnnnnnnnnnnnnnnnnnnnnnnnnnnnnnnnnnnnnnnnnnnnnnnnnnnnnnnnnnnnnnnnnnnnnnnnnnnnnnnnnnnnnnnnnnnnnnnngccggcgactttcgccggcccctgcgcacgcgcggaccgtccggcctgtaggtgcggaccgtccggccgtcaggcagggaacctttgcccctgctccaggtcgcggaccgtccggtccctggtcgcggaccgtccgcgcctgtgcagagagcaccaccgccggttcttgttgagtgtttggcgcccgaaaaaggtgtcaacatacttttggcgactccgctggggaaggtgtttagatctactaaaaatcaggccctcaaatggccggttctaaagatcacaccgatatctccccggacaatatcctgaagccggctgttgaaagtctgacgaccgatgagcaacagcaatacgaggactacatgcgtcaagcgagggagaaattcttatcacaatacacggtggatcgccaccaaaaagttgtcaaacatggagagactgacgtcgcatctcttctatcttcgcttcaagtccccaacgtaagtaaacccgacgacatccaatttattaaacagtatgtagatcagcagcaggatcaaatgaaacaacagattgtagggttagaaaagtcaattagaaaattaacgcgtacgttggagaagtctcttgctcctagttttccatcatatgagactagtaacaggatatctatgtctaatacatcggcaacaaatggggatttgcagccccagccattatatggtatgccgatgaactcatatacaggacaagtaccaccaccgccatccctgcttggtagatcggcacccatgaacacggtcggaccgtccgagcttctgcccggaccgtccggcccatatgcagaccgtccggcttgctctgccggacaatctggggccgccctaggaccaccgtcgtccctgcttggtagaccggtgaccttggacgcggtcggaccgtccgagcttctgcctggaccgtccggcccttacgcggaccgtccggctttccctgccggacagtctgggcccgcaccaggactaccacatggcgtcccgataatggcaaacgcaaccggtcagttcggatttaccaccggacaagctggatacgcatacgcagaacctgttgttgcacaccatgcaccaaattattacacaccacagcagcagtatgtttcgccctctacatatttaaaccataacgcaccatacaatcacagaccgatcaacactatcgatcggtcacggcaagaaggtcggtatactaatgcccgaccaaatgatccccacagcccaggatccggtggtctgccaccgggtgcaatggagaaaattagggaagagatgactgaactatttcgagataagttcggagttagtgtagccagagtagggcaatcataccaaaagccgtataatcaccggtttgacactgtcccatatccacaaggggcaaggataccagaattttctaagttttctggtgagaatgggagaagcacacacgaacacataggccagttcctagcacacctaggcgaattggccgatggagaagcatttcgtgttcggttattttctttatcccttactggtactgcttttgcatggtacgccgccctgcctcctaattccattaattcctggaatgagttagaaagtaaatttcatgaacatttatttaccggggaatatgaattagggttagctgacttagcttcagttcgacaaggacgcgaagaatcggttaatgattatatccggaggttccgggacactagaaaccgatgctttcggatccatgtcgcagacaaagagctagcagggttagcttttaatgggttgctatcctacttaagagacaaattagatgggacccagttcttttcgatagcccagctacatcagcgggctttagcctgtgaaagccgatttaaagagacatcaaaatcggccgcccgtactatacatctaatagagcgtgatagttcagatgatgaatccgcatatgtatataccgctgagtttatttggccaacaaaggccaaatcttcagcatgttcttccttacnnnnnnnnnnnnnnnnnnnnnnnnnnnnnnnnnnnnnnnnnnnnnnnnnnnnnnnnnnnnnnnnnnnnnnnnnnnnnnnnnnnnnnnnnnnnnnnnnnnnnnnnnnnnnnnnnnnnnnnnnnnnnnnnnnnnnnnnnnnnnnnnnnnnnnnnnnnnnnnnnnnnnnnnnnnnnnnnnnnnnnnnnnnnnnnnnnnnnnnnnnnnnnnnnnnnnnnnnnnnnnnnnnnnnnnnnnnnnnnnnnnnnnnnnnnnnnnnnnnnnnnnnnnnnnnnnnnncctgttaatacaatagatatcgcatgcaaaaagatcttagttcgacccgaaatggccgataaaagcaaaagcaaagacatcatcattgacgatcctcgcacgtcaaatatatcgcaaaaggagattgctcgaaaggctccggacgataaggctaaaaagtccggaggcaccggggggcaggcacaattaatgagccaagcacgacagcctggcctgagcatcacaaacggtgtgacacctacgtgcggacagtccggtgctcagacagacggttcggctaactctgccggacaatccgcttatggccaaaggcgtcagcctccacacaaagccttaaaagggaaagagacgcaacgacaaagcacatatggtcggttgatcaaaactgactctacctttgatcagttactccccaagaatactagcaagaagaccgttctacgtgatcggtcaacgaagaaacatcggtcacctgctaaaacaaaacgggtaaacaaaacggctcgaaaggcgacacaacaagcatcgcctattcatcctatgagaccaaggtactttccacccgtttactcatcctcggtatattatcctgttcaaacatggaatggtacgatgatgaatccatggtatatgtatagtctgtcatgtggggccgcacctacacgcgggcccgcgacgccaggagggctgaggctagggcgtnnnnnnnnnnnnnnnnnnnnnnnnnnnnnnnnnnnnnnnnnnnnnggctgctacacgccttcgccgatgtcttcaccgagccgagcggactacctccagcacgcggccacgagcaccacatcgtcctcaagccaggctcctccccggtggcggtgcgaccgtacaggtacccggcggcgcacaaggacgaacttgagcggcagtgcgccgccatgatcgaccagggcatcgtccgccgcagtgactcggcgttctcttccccggtcatccttgtcaagaagctggacgggtcgtggcgcttctgcgtcgactaccgcgcgttgaacgcgctcactgtcaaagacgcgtatccgattccggtcgtcgacgagctcctcgacgagctccatggtgcacgcctcttcaccaagctnnnnnnnnnnnnnnnnnnnnnnnnnnnnnnnnnnnnnnnnnnnnnnnnnnnnnnnnnnnnnnnnnnnnnnnnnnnnnnnnnnnnnnnnnnnnnnnnnnnnnnnnnnnnnnnnnnnnnnnnnnnnnnnnnnnnnnnnnnnnnnnnnnnnnnnnnnnnnnnnnnnnnnnnnnnnnnnnnnnnnnnnnnnnnnnnnnnnnnnnnnnnnnnnnnnnnnnnnnnnnnnnnnnnnnnnnnnnnnnnnnnnnnnnnnnnnnnnnnnnnnnnnnnnnnnnnnnnnnnnnnnnnnnacgtcatttcagcggctggtgtcgctatggatcccgcgaaggtccaggccatccacgactggcgccaacctcgttcggcgcgcgccgtgcggggcttcctcggtctggcaggctactatcgcaagttcgtccacaactacggcgccattgcagcacccctcacagcactcctgaagaaagaggggttcgtgtggtccgacgaggcaagcgccgcttttcgtgccctcaaaagggcagtgacgacagcaccagtgttgacattaccggacttcaccaagcccttcatcgtggagtgcgacgcgtccacctatggcttcggggcggtgctcatacaggaggctcatccgctcgccttcttcagtcgaccggtggcgccccgccatcgctccctagcggcctatgagcgcgaactcatcgggctcgtgcttgccgtacggcattggaggccgtacctatgggggcgacgcttcgtcgtcaagacagaccactacagcctcaagtacctcctcgatcagcgcctggcgaccattccacaacatcattgggtgggtaagctcctcgggttcgacttctccgtcgagtacaagtcaggagcaacgnnnnnnnnnnnnnnnnnnnnnnnnnnnnnnnnnnnnnnnnnnnnnnnnnnnnnnnnnnnnnnnnnnnnnnnnnnnnnnnnnnnnnnnnnnnnnnnnnnnnnnnnnnnnnnnnnnnnnnnnnnnnnnnnnnnnnnnnnnnnnnnnnnnnnnnnnnnnnnnnnnnnnnnnnnnnnnnnnnnnnnnnnnnnnnnnnnnnnnnnnnnnnnnnnnnnnnnnnnnnnnnnnnnnnnnnnnnnnnnnnnnnnnnnnnnnnnnnnnnnnnnnnnnnnnnnnnnnnnnnnnnnnnnnnnnnnnnnnnnnnnnnnnnnnnnnnnnnnnnnnnnnnnnnnnnnnnnnnnnnnnnnnnnnnnnnnnnnnnnnnnnnnnnnnnnnnnnnnnnnnnnnnnnnnnnnnnnnnnnnnnnnnnnnnnnnnnnnnnnnnnnnnnnnnnnnnnnnnnnnnnnnnnnnnnnnnnnnnnnnnnnnnnnnnnnnnnnnnnnnnnnnnnnnnnnnnnnnnnnngctcatgggcactaagctgcacatgtcgtccgccttccacccacagtccgacggccagacggaagcggccaaccgcgtcatcattatgtacctccgctgtttcacaggcgaccgtcctcgacaatggcttcgctggctgccgtgggccgaatacgtgtacaacacggcataccagtcctcgctccgggagacgccattccgggtggtgtatggtcgtgacccgccctccatccgctcttatgagcctggtgaaacgagggtggatgcggtcgcacgcaacatggaggaacgcgaggcattcctggccgatgtgcgctatcgcctcgagcaggcccaagcggtgcagaaacgtcactacgacaagcaacaccggccagtgacatatgcagtcggcgactgggcactccttcgacttcgccagcgagctccgtcctcactgccacaacagacatcgggcaaactaaagccccgcttcctcggaccctaccgcgtcatcgagctcatcaacaatgtcgccgttcgcctggagctaccaccacaggccnnnnnnnnnnnnnnnnnnnnnnnnnnnnnnnnnnnnnnnnnnnnnnnnnnnnnnnnnnnnnnnnnnnnnnnnnnnnnnnnnnnnnnnnnnnnnnnnnnnnnnnnnnnnnnnnnnnnnnnnnnnnnnnnnnnnnnnnnnnnnnnnnnnnnnnnnnnnnnnnnnnnnnnnnnnnnnnnnnnnnnnnnnnnnnnnnnnnnnnnnnnnnnnnnnnnnnnnnnnnnnnnnnnnnnnnnnnnnnnnnnnnnnnnnnnnnnnnnnnnnnnnnnnnnnnnnnnnnnnnnnnnnnnnnnnnnnnnnnnnnnnnnnnnnnnnnnnnnnnnnnnnnnnnnnnnnnnnnnnnnnnnnnnnnnnnnnnnnnnnnnnnnnnnnnnnnnnnnnnnnnnnnnnnnnnnnnnnnnnnnnnnnnnnnnnnnnnnnnnnnnnnnnnnnnnnnnnnnnnnnnnnnnnnnnnnnnnnnnnnnnnnnnnnnnnnnnnnnnnnnnnnnnnnnnnnnnnnnnnngccggcgactttcgccggcccctgcgcacgcgcggaccgtccggcctgtaggtgcggaccgtctggccgtcaggcagggaacctttgcccctgctccaggtcgcggaccgtccggtccctggtcgcggaccgtccgcgcctgtgcagagagcaccgccgccggttcttgttgagtgtttggcgcccgaaaaaggtgtcaacacccagtcgtgcattgacggttgatatggcttgattatttactgaccgaaaaaatcactttactcaccgtgatttttatggttgtagaatttcttcttgggtatatcggcaatagatcagatccacgcaatagaaaacactagaacacaagtcaacacagagctaatcaaaattcctgtgctgcagacttatctgccaagcaaaatgcctgcggcattggtgccttaccggcaggacgagctcaagattctccgcggcgacgataatcctggaccatacaaggagcacgaccgcgtctaccgttacgactactacaacgacctcggtgagccagacaagggtgaagaccatgcccggcctgtcctcgggggcagccaagaacacccgtatccccgtcgctgcaggaccggccggcgtccaacagagacaggtaggttcaaggaagcaagctacattctggtccatacaacaagatgccagaaatttgtcctgaaacccttgttggctaacctttttacgcagaccccaactcggagagcaggctgtttctgctgaacctgaacatctacgtcccgcgcgacgagcggtttgggcatctcaagatgtcggacttcctcgggtactcactgaaggcgatcatcgaggctgtccttccgacgctggggacgttcgtcgacgatacgcccaaggagttcgattcgttcgaagacatccttgggctctacgagccgggtccagaggcgcccaacaacccactggtagcagaggtcaggaagagaatccccagcgagttcctcagaagcattctgcccaatggtagccatgaccaccccctgaagatgccccttccaaatatcatcagatcaggtaactggacttcatggaatgccttttttctacatgttaatagtcctaaaaaggttttaggtttgccatgactgaggctaaatcttggtactcaccagatgtgttgaaaaaggctccagagtttaagtttggctggaggaccgacgaagagtttgcgagggagacgcttgcaggcgtgaacccagtgctcatcaaacgtctgacggttagcatctatcttccatcatatggactggccaattcaatatacctgccccgcaactaagtaaaagggccttaaaaaattctttttttttcatggtctcaggagttcccagctaaaagtaccctggacccaagtcaatacggagaccatacgagcaagatcaccgaagctcacatccagcataacatggaaggcctgtcagtgcagaatgtatgcttggactgaacgcgcatactataacaaccgaaagattcaatacagataattgattaaaaccatcgactgattgccaaaacgaaccctgtgcaggcactgaagaagaacaggctcttcatcctagaccaccatgaccatttcatgccgtacctcaacaagatcaacgagttggaggggaacttcatctacgccagcaggaccctactgttcctgaaggacgatggcacgctgaagcccctggccgtcgagctgagcctgccccaccctgatggccagcagcacggcgcggtcagcaaggtgtacaccccagctcactccggcgctgagggccacgtctggcaacttgccaaggcttatgcctgcgtgaacgactccgcctggcatcagctgatcagccactggtacagagagctcttccttaatttgtttttctccttgataccaaaatgcaaaaatgttctttttcatgttcagagacaactaaaaacactaatcttgtgtgtgtttgcaggctgaacacgcacgcggtgatcgagccgttcgtcatcgcaacgaaccggcagctgagcgtggtgcatccagtgcacaagctgctgagcccacactaccgtgacacgctgaacatcaacgccctggcacgccagacgctcatcaacgccgacggcatcttcgagcgcaccgtgttccctgcaaagtacgcgctggggatgtcctccgacgtgtacaagagctggaatttcaacgagcaggctctcccagcagacctcgtcaagaggtacgtacatgtatagtactaactacattgagcagtaaacgcctatagcagtgacgagatggttctgacgggtttatttgctcctctggttgtgcgtttcagaggtgtggctgtgccggaccagtcgagcccctacggtgtccggttgctgatcaaggactacccttacgccgtggacgggctggtcatctggtgggcgatcgagcggtgggtcaaggagtacctggacgtctactaccccaacgacggcgagctccagcgcgacgtggagctgcaggcgtggtggaaggaggtgcgcgaggaggcgcacggcgacctcaaggaccgagactggtggcccaggatggacgccgtccagcggctggccagggcgtgcacgaccgtcatctgggtagcgtccgcgctgcacgcggccgtcaacttcgggcagtacccgtacgccgggtacctgccgaaccggccgaccgtgagccggcggccgatgccggagccgggcagcgacgactacaagaagctggaggcggggcagaaggaggcggacgcggtgttcatccgcaccatcaccagccagttccagaccatcctgggcatctcgctcatcgagatcctctccaagcactcctccgacgaggtgtacctcggccagcgcgacgagcctgagcgctggacgtcggacgccagggcgctggacgcgttcagaaggttcggaagccggctggtggagatcgagaagcggatcaggacgatgaacgacagcccgacgttgaagaaccggaaggggccggtggagatgccgtacatgctgctgtaccccaacacgtcggatgtcaccggcgagaagggcgaggggctcactgccatgggcattcccaacagcatctccatatga

SEQ ID NO: 16 - DNA, 5376 bp, Zea mays
atgctgagcgggatcatcgacgggctgacgggggcgaacaagcatgcgcggctcaagggcacggtggtgctcatgcgcaagaacgtgctggacctcaacgacttcggcgccaccgtcgtcgacagcatcagcgagttcctcggcaagggggtcacctgccagctcatcagctccactctcgtcgacgccaacaacggcaaccgcgggcgggtcggggcggaggcgaacctggagcagtggctgacgagcctgccgtcgctgacgaccggcgagtccaagttcggcgtcacgttcgactgggaggtggagaagctgggagtgccgggggccgtcgtcgtcaagaacaaccacgccgccgagttcttcctcaagacaatcaccctcgacgacgtgcccggccgcggcgccgtcaccttcgtcgccaactcctgggtctaccccgcgggcaagtaccgctacaaccgcgtcttcttctccaacgatacgtacctgccaagccagatgccggcggcgctgaagccgtaccgcgacgacgagctccgcaacctccgcggcgacgaccagcagggcccctaccaggagcacgaccgcgtgtaccgctacgacgtctacaacgacctcggcgagcccgacggcggcaacccgcgccccatcctcggcggctccgccgaccacccgtacccgcgccgctgccgcacgggccgcaagcccaccaaaaccgaccccaactcggagagccgactgtcgctggtggagcagatctacgtgccgcgggacgagcgcttcggccacctcaagatgtccgacttcctgggctactccatcaaggccatcacgcagggcatcatcccggcggtgcgcacgtacgtggacaccaccccgggcgagttcgactccttccaggacatcatcaacctgtacgagggcgggatcaagctgcccaagatccaggcgctcgaggacatgcgcaagctcttcccgctccagctcgtcaaggacctcctccccgccggcggggactacctgctcaagctccccatcccacagatcatccaaggcacgtcacgtataccgatcgatgtcaggggccggctgttgtctggtctgcatatatatatgtgctcctatgaggacaagaacgcgtggaggaccgacgaggagttcgcgcgggaggtgctcgccggcgtcaacccgatggtgatcacgcgcctcacggagttcccgcccaagagcacgctggaccccagcaagtacggcgaccacaccagcacgatcacggcggagcacatcgagaagaacctcgagggcctcacggtgcagcaggcgctggacggcaacaggctctacatcctggaccaccacgaccgcttcatgccgttcctcatcgacgtcaacaacctggagggcaacttcatctacgccaccaggacgctcttcttcctgcgcggcgacggcaggctcgcgcccctcgccatcgagctcagcgagccgtacatcgacggggacctcaccgtggccaagagcaaggtctacacgccggcgtccagcggcgtcgaggcctgggtgtggcagctcgccaaggcctatgtcgccgtcaacgactctggctggcaccaactcgtcagccactggctgaacacccacgcggtgatggagccgttcgtgatcgcgacgaaccggcagctgagcgtgacgcacccggtgcacaagctcctgagctcgcacttccgcgacaccatgaccatcaacgcgctggcgcggcagacgctcatcaacggcggcggcatcttcgagatgaccgtcttcccgggcaagtacgcgctgggcatgtcctccgtggtgtacaagagctggaacttcaccgagcagggcctccccgccgacctcgtcaagaggggcgtggcggtggcggacccgtccagcccgtacaaggtgcggctgctgatcgaggactacccgtacgcgagcgacgggctggccatctggcacgccatcgagcagtgggtgggcgagtacctggccatctactaccccgacgacggcgcgctgcggggcgacgaggagctgcaggcgtggtggaaggaggtgcgcgaggtcgggcacggcgaccacaaggacgcgccctggtggcccaagatgcaggccgtgtcggagctcgccagcgcctgcaccaccatcatctggatcgcgtcggcgctccacgccgccgtcaacttcggccagtacccgtacgcggggtacctcccgaacaggcccacggtgagccggcgccggatgccggagcccggcagcaaggagtacgaggagctggagcgcgacccggagcgcggcttcatccacaccatcacgagccagatccagaccatcatcggcatctcgctcatcgagatcctctccaagcactcctccgacgaggtgtacctcggccagcgcgacacccccgagtggacctccgacgcccgggcgctggcggcgttcaagaggttcagcgacgcgctggtcaagatcgagggcaaggtggtgggcgagaaccgcgacccgcagctgaggaacaggaacggccccgccgagttcccctacatgctgctctatcccaacacctctgaccacagcgaggcgagggagcgagcagcagggcaaggcatccacacccacacccaccggacactccctgagaagcgagaagcgagaagcgaagagcggccggccaccatgttctggcacggggtcgcggaccggctgacggggaagaacaaggaggcgtggaacgagggaaagatccgcggcacggtgaggctggtcaagaaggaggtgctggacgtcggcgacttcaacgcctcgctcctcgacggcgtacacaggatcctcggctgggacgacggcgtcgccttccagctcgtcagcgccaccgcggccgaccccagcaacgggagccgcggcaaggtcgggaaggcggcgcacctggaggaggcggtggtgtcgctcaagtcgacgacggacggggagaccgtgtaccgggtgagcttcgagtgggacgggtcgcagggcgtcccgggcgccgtcctggtcaggaacctgcagcacgccgagttcttcctcaagtcgctcaccctcgagggcgtccccggcaggggcaccgtcgtcttcgtcgccaactcgtggatctacccgcacaatctctactcccaggaacgcgtcttcttcgccaacgacacttatctgccaagcaaaatgcctgcggcattggtgccttaccggcaggacgagctcaagattctccgcggcgacgataatcctggaccatacaaggagcacgaccgcgtctaccgttacgactactacaacgacctcggtgagccagacaagggtgaagaccatgcccggcctgtcctcgggggcagccaagaacacccgtatccccgtcgctgcaggaccggccggcgtccaacagagacagaccccaactcggagagcaggctgtttctgctgaacctgaacatctacgtcccgcgcgacgagcggtttgggcatctcaagatgtcggacttcctcgggtactcactgaaggcgatcatcgaggctgtccttccgacgctggggacgttcgtcgacgatacgcccaaggagttcgattcgttcgaagacatccttgggctctacgagccgggtccagaggcgcccaacaacccactggtagcagaggtcaggaagagaatccccagcgagttcctcagaagcattctgcccaatggtagccatgaccaccccctgaagatgccccttccaaatatcatcagatcagatgtgttgaaaaaggctccagagtttaagtttggctggaggaccgacgaagagtttgcgagggagacgcttgcaggcgtgaacccagtgctcatcaaacgtctgacggagttcccagctaaaagtaccctggacccaagtcaatacggagaccatacgagcaagatcaccgaagctcacatccagcataacatggaaggcctgtcagtgcagaatgcactgaagaagaacaggctcttcatcctagaccaccatgaccatttcatgccgtacctcaacaagatcaacgagttggaggggaacttcatctacgccagcaggaccctactgttcctgaaggacgatggcacgctgaagcccctggccgtcgagctgagcctgccccaccctgatggccagcagcacggcgcggtcagcaaggtgtacaccccagctcactccggcgctgagggccacgtctggcaacttgccaaggcttatgcctgcgtgaacgactccgcctggcatcagctgatcagccactggctgaacacgcacgcggtgatcgagccgttcgtcatcgcaacgaaccggcagctgagcgtggtgcatccagtgcacaagctgctgagcccacactaccgtgacacgctgaacatcaacgccctggcacgccagacgctcatcaacgccgacggcatcttcgagcgcaccgtgttccctgcaaagtacgcgctggggatgtcctccgacgtgtacaagagctggaatttcaacgagcaggctctcccagcagacctcgtcaagagaggtgtggctgtgccggaccagtcgagcccctacggtgtccggttgctgatcaaggactacccttacgccgtggacgggctggtcatctggtgggcgatcgagcggtgggtcaaggagtacctggacgtctactaccccaacgacggcgagctccagcgcgacgtggagctgcaggcgtggtggaaggaggtgcgcgaggaggcgcacggcgacctcaaggaccgagactggtggcccaggatggacgccgtccagcggctggccagggcgtgcacgaccgtcatctgggtagcgtccgcgctgcacgcggccgtcaacttcgggcagtacccgtacgccgggtacctgccgaaccggccgaccgtgagccggcggccgatgccggagccgggcagcgacgactacaagaagctggaggcggggcagaaggaggcggacgcggtgttcatccgcaccatcaccagccagttccagaccatcctgggcatctcgctcatcgagatcctctccaagcactcctccgacgaggtgtacctcggccagcgcgacgagcctgagcgctggacgtcggacgccagggcgctggacgcgttcagaaggttcggaagccggctggtggagatcgagaagcggatcaggacgatgaacgacagcccgacgttgaagaaccggaaggggccggtggagatgccgtacatgctgctgtaccccaacacgtcggatgtcaccggcgagaagggcgaggggctcactgccatgggcattcccaacagcatctccatatga

SEQ ID NO: 17 - protein, 1791 aa, Zea mays
MLSGIIDGLTGANKHARLKGTVVLMRKNVLDLNDFGATVVDSISEFLGKGVTCQLISSTLVDANNGNRGRVGAEANLEQWLTSLPSLTTGESKFGVTFDWEVEKLGVPGAVVVKNNHAAEFFLKTITLDDVPGRGAVTFVANSWVYPAGKYRYNRVFFSNDTYLPSQMPAALKPYRDDELRNLRGDDQQGPYQEHDRVYRYDVYNDLGEPDGGNPRPILGGSADHPYPRRCRTGRKPTKTDPNSESRLSLVEQIYVPRDERFGHLKMSDFLGYSIKAITQGIIPAVRTYVDTTPGEFDSFQDIINLYEGGIKLPKIQALEDMRKLFPLQLVKDLLPAGGDYLLKLPIPQIIQGTSRIPIDVRGRLLSGLHIYMCSYEDKNAWRTDEEFAREVLAGVNPMVITRLTEFPPKSTLDPSKYGDHTSTITAEHIEKNLEGLTVQQALDGNRLYILDHHDRFMPFLIDVNNLEGNFIYATRTLFFLRGDGRLAPLAIELSEPYIDGDLTVAKSKVYTPASSGVEAWVWQLAKAYVAVNDSGWHQLVSHWLNTHAVMEPFVIATNRQLSVTHPVHKLLSSHFRDTMTINALARQTLINGGGIFEMTVFPGKYALGMSSVVYKSWNFTEQGLPADLVKRGVAVADPSSPYKVRLLIEDYPYASDGLAIWHAIEQWVGEYLAIYYPDDGALRGDEELQAWWKEVREVGHGDHKDAPWWPKMQAVSELASACTTIIWIASALHAAVNFGQYPYAGYLPNRPTVSRRRMPEPGSKEYEELERDPERGFIHTITSQIQTIIGISLIEILSKHSSDEVYLGQRDTPEWTSDARALAAFKRFSDALVKIEGKVVGENRDPQLRNRNGPAEFPYMLLYPNTSDHSEARERAAGQGIHTHTHRTLPEKREARSEERPATMFWHGVADRLTGKNKEAWNEGKIRGTVRLVKKEVLDVGDFNASLLDGVHRILGWDDGVAFQLVSATAADPSNGSRGKVGKAAHLEEAVVSLKSTTDGETVYRVSFEWDGSQGVPGAVLVRNLQHAEFFLKSLTLEGVPGRGTVVFVANSWIYPHNLYSQERVFFANDTYLPSKMPAALVPYRQDELKILRGDDNPGPYKEHDRVYRYDYYNDLGEPDKGEDHARPVLGGSQEHPYPRRCRTGRRPTETDPNSESRLFLLNLNIYVPRDERFGHLKMSDFLGYSLKAIIEAVLPTLGTFVDDTPKEFDSFEDILGLYEPGPEAPNNPLVAEVRKRIPSEFLRSILPNGSHDHPLKMPLPNIIRSDVLKKAPEFKFGWRTDEEFARETLAGVNPVLIKRLTEFPAKSTLDPSQYGDHTSKITEAHIQHNMEGLSVQNALKKNRLFILDHHDHFMPYLNKINELEGNFIYASRTLLFLKDDGTLKPLAVELSLPHPDGQQHGAVSKVYTPAHSGAEGHVWQLAKAYACVNDSAWHQLISHWLNTHAVIEPFVIATNRQLSVVHPVHKLLSPHYRDTLNINALARQTLINADGIFERTVFPAKYALGMSSDVYKSWNFNEQALPADLVKRGVAVPDQSSPYGVRLLIKDYPYAVDGLVIWWAIERWVKEYLDVYYPNDGELQRDVELQAWWKEVREEAHGDLKDRDWWPRMDAVQRLARACTTVIWVASALHAAVNFGQYPYAGYLPNRPTVSRRPMPEPGSDDYKKLEAGQKEADAVFIRTITSQFQTILGISLIEILSKHSSDEVYLGQRDEPERWTSDARALDAFRRFGSRLVEIEKRIRTMNDSPTLKNRKGPVEMPYMLLYPNTSDVTGEKGEGLTAMGIPNSISI

SEQ ID NO: 18 - DNA, 18 bp, Artificial Sequence
  Primer S3460 for Lox3 of Zea mays
cctcgtcgacgccaacaa

SEQ ID NO: 19 - DNA, 19 bp, Artificial Sequence
  Primer S3461 for Lox3 of Zey mays
acgtgacgccgaacttgga

SEQ ID NO: 20 - DNA, 25 bp, Artificial Sequence
  Primer S3428 for Elongation factor 1-alpha
ggtaaagagaagtcccacatcaaca

SEQ ID NO: 21 - DNA, 23 bp, Artificial Sequence
  Primer S3429 for Elongation factor 1-alpha
ctccttctcaaacctctcgatca

SEQ ID NO: 22 - DNA, 1913 bp, Zea mays
ttgtagttcatgcgcagtaagagttgtaacctcataatatgaccaaattcctgatctgctttatagagttgttgtgcctaattttgaattcgtcttactggctcaaaattatgtgcgcacacttattagtttgctctttattttctatgcctgctttatttttttatattacattgattgctctgtttaatatttgcttctttatttttacactgcttatgtgtatcaagcttttttcaagctcataactccggttacaacgttagatctagtttctgatcccatctgataaatttgtttctaatcgttgattcgtcttgttaacagttcaatctcacctccaaccatgggtaaagagaagtcccacatcaacattgtggttattggccacgttgactctggcaagtcgaccaccacaggacacctgatctacaagcttggaggcattgacaagcgtgtgatcgagaggtttgagaaggaggctgctgaaatgaacaagcggtccttcaagtacgcatgggtgctcgacaagctcaaggctgagcgtgagagaggtatcaccattgatatcgctctgtggaagtttgagaccaccaagtactactgcacggtcattgatgcccctggacaccgtgacttcatcaagaacatgatcactggtacctcccaggctgactgtgctgtccttatcattgactccaccactggtggttttgaggctggtatctccaaggatggccagacccgtgaacatgctctccttgcgttcacccttggagtgaagcagatgatttgctgctgcaacaagatggatgcaaccactccaaaatactccaaggcacgttatgatgagattgtgaaggaagtctcatcctacctcaagaaagttgggtacaaccctgataagattgccttcgttcccatttctggttttgagggcgacaacatgattgagaggtccaccaaccttgactggtacaaaggcccaaccctgcttgaggctcttgaccagatcaccgagcccaagaggccttcggacaagcccctgcgtctgcccctccaggatgtgtacaagattggtggtattggaactgtaccggttggtcgtgtggagactggtgtcatcaagcctggtatggtagtcacctttggtccaactggcctgactactgaggtgaagtctgttgagatgcaccatgaggcgcttcaggaggctcttccgggcgacaatgttggcttcaacgtgaagaacgttgctgtcaaggatctcaagcgtgggttcgtggcctccaactccaaggatgaccctgccaaggaggctgccagcttcacctcccaggtcatcatcatgaaccaccctgggcagattggcaacggctatgccccagtgctggactgccacacctcccacatcgccgtcaagtttgctgagctcattaccaagatcgacaggcgatctggcaaggagctcgagaaggagcccaagttcctgaagaacggtgatgctggtatggtgaagatgattcccaccaagcctatggtggtggagacattctccgcgtatcctcccctgggtaggtttgccgtccgcgacatgaggcagacggttgctgttggagtcatcaagagtgtggagaagaaggacccaaccggcgccaaggtgaccaaggcggccgccaagaagaaatgatgcgatcccgtgtctgcttttgcagtgcctggataacttgccactaaagttgtgtatgcggttgttgctgttattgcgtggactgtttgctgcggtgtctcctgtttgtttgggtagcgcagcgtcggcctcttcaggtgtctgttgtctgttgtctttactatcagtaatgctcctgagacttgtatttctccttttggcgccgctaaatggaattttcgaa

SEQ ID NO: 23 - protein, 447 aa, Zea mays
MGKEKSHINIVVIGHVDSGKSTTTGHLIYKLGGIDKRVIERFEKEAAEMNKRSFKYAWVLDKLKAERERGITIDIALWKFETTKYYCTVIDAPGHRDFIKNMITGTSQADCAVLIIDSTTGGFEAGISKDGQTREHALLAFTLGVKQMICCCNKMDATTPKYSKARYDEIVKEVSSYLKKVGYNPDKIAFVPISGFEGDNMIERSTNLDWYKGPTLLEALDQITEPKRPSDKPLRLPLQDVYKIGGIGTVPVGRVETGVIKPGMVVTFGPTGLTTEVKSVEMHHEALQEALPGDNVGFNVKNVAVKDLKRGFVASNSKDDPAKEAASFTSQVIIMNHPGQIGNGYAPVLDCHTSHIAVKFAELITKIDRRSGKELEKEPKFLKNGDAGMVKMIPTKPMVVETFSAYPPLGRFAVRDMRQTVAVGVIKSVEKKDPTGAKVTKAAAKKK

SEQ ID NO: 24 - protein, 494 aa, Zea mays
MDTSHHYHPWLNFSLAHHCDLEEEERGAAAELAAIAGAAPPPKLEDFLGGGVATGGPEAVAPAEMYDSDLKFIAAAGFLGGSAAAAATSPLSSLDQAGSKLALPAAAAAPAPEQRKAVDSFGQRTSIYRGVTRHRWTGRYEAHLWDNSCRREGQSRKGRQVYLGGYDKEEKAARAYDLAALKYWGSSTTTNFPVAEYEKEVEEMKNMTRQEFVASLRRKSSGFSRGASIYRGVTRHHQHGRWQARIGRVAGNKDLYLGTFSTEEEAAEAYDIAAIKFRGLNAVTNFEISRYNVETIMSSNLPVASMSSSSAAAAGGRSSKALESPPSGSLDGGGGMPVVEGSTAPPLFIPVKYDQQQQEYLSMLALQHHHQQQQAGNLLQGPLVGFGGLYSSGVNLDFANSHGTAAPSSMAHHCYANGTASASHEHQHQHQMQQGGENETQPQPQQSSSSCSSLPFATPVAFNGSYESSITAAGPFGYSYPNVAAFQTPIYGME

SEQ ID NO: 25 - DNA, 1485 bp, Zea mays
atggacacctcgcaccactatcatccatggctcaacttctccctcgcccaccactgtgacctcgaggaggaggagaggggcgcggccgccgagctggccgcgatagccggcgccgcgccgccgccgaagctggaggacttcctcggcggaggcgtcgccaccggtggtccggaggcggtggcgcccgcggagatgtacgactcggacctcaagttcatagccgccgccgggttccttggcggctcggcggcggcggcggcgacgtcgccgctgtcctccctcgaccaggccggttccaagctggccttgcctgcggcggcggctgctccggcgccggagcagaggaaggccgtcgactcctttgggcagcgcacgtccatctaccgcggcgtcacacggcaccggtggactggcaggtacgaggcacatctgtgggacaacagctgccgacgcgaagggcagagccgcaagggccgccaagtatatttgggtggctatgataaggaggagaaggctgccagggcgtatgatcttgcagctttgaagtactggggttctagcaccaccaccaactttccggttgctgagtatgagaaggaggtcgaggagatgaagaacatgacgcgacaagagtttgttgcttcccttcgaaggaagagcagtggattctctcggggtgcttccatctacagaggtgtaaccagacatcaccagcatggacggtggcaggcgaggatcggaagggtggccggtaacaaggacctctaccttgggacgttcagcaccgaggaggaagctgcagaggcctacgacatagcggccatcaagttcagaggcctgaacgccgtcacaaacttcgagatcagccggtacaacgtggagaccataatgagcagcaaccttccagtcgcgagcatgtcgtcgtcgtcggcggcggcggcgggtggccggagcagcaaggcgctggagtcccctccgtccggctcgcttgacggcggcggcggcatgccagtcgtcgaaggcagcacggcaccgccgctgttcattccggtgaagtacgaccagcagcagcaggagtacctgtcgatgctcgcgttgcagcaccaccaccagcagcaacaagcagggaacctgttgcaggggccgctagtagggttcggcggcctctactcctccggggtgaacctggatttcgccaactcccacggcacggcggctccgtcgtcgatggcccaccactgctacgccaatggcaccgcgtccgcctcgcatgagcaccagcaccagcaccagatgcagcagggcggcgagaacgagacgcagccgcagccgcagcagagctccagcagctgctcctccctgccattcgccaccccggtcgctttcaatgggtcctatgaaagctccatcacggcggcaggcccctttggatactcctacccaaatgtggcagcctttcagacgccgatctatggaatggaatga

SEQ ID NO: 26 - protein, 164 aa, Artificial Sequence
  Regeneration booster P8
MVSKGEEVIKEFSGSTRWNPTAEQVKVLREIYYRAGLRTPSADQIRQISSQLKRYGKVEGKNVFYWFQNHKARERQKKRLSTVGSAGSAAGSGEFRHVKTLPLFPLHNNEDSGSGLDLDLNLELRLSATAAATSGSQRASALDLDLELRLGFALGNESCGLHDN

SEQ ID NO: 27 - DNA, 498 bp, Artificial Sequence
  Regeneratio booster P8 CDS
atggtttcgaagggggaagaagtcattaaagagttttcagggtctacgcgctggaaccctaccgctgaacaagtcaaggttttgagggaaatatattaccgcgcgggtcttaggacgccatccgcggatcagatccgccaaatatcctcacagctgaaacggtatggaaaggtggaaggaaaaaacgtgttttattggttccagaaccataaagcgcgggaaagacaaaaaaagcggctcagcaccgttgggagcgctggctcagcagcgggttcaggtgagttcaggcacgttaaaacactgcccttgttccctttgcacaataatgaagactcagggagcggtttggacttggatctgaaccttgagttgcgcctgtcggcgactgctgctgccacttcgggctcacagcgggcgtctgccctcgatctggacttggagctcagactcggtttcgcgcttggtaatgagtcgtgtggactgcacgacaactagtga

SEQ ID NO: 28 - protein, 1252 aa, Artificial Sequence
  LbCpf1-RR
MAPKKKRKVSKLEKFTNCYSLSKTLRFKAIPVGKTQENIDNKRLLVEDEKRAEDYKGVKKLLDRYYLSFINDVLHSIKLKNLNNYISLFRKKTRTEKENKELENLEINLRKEIAKAFKGNEGYKSLFKKDIIETILPEFLDDKDEIALVNSFNGFTTAFTGFFDNRENMFSEEAKSTSIAFRCINENLTRYISNMDIFEKVDAIFDKHEVQEIKEKILNSDYDVEDFFEGEFFNFVLTQEGIDVYNAIIGGFVTESGEKIKGLNEYINLYNQKTKQKLPKFKPLYKQVLSDRESLSFYGEGYTSDEEVLEVFRNTLNKNSEIFSSIKKLEKLFKNFDEYSSAGIFVKNGPAISTISKDIFGEWNVIRDKWNAEYDDIHLKKKAVVTEKYEDDRRKSFKKIGSFSLEQLQEYADADLSVVEKLKEIIIQKVDEIYKVYGSSEKLFDADFVLEKSLKKNDAVVAIMKDLLDSVKSFENYIKAFFGEGKETNRDESFYGDFVLAYDILLKVDHIYDAIRNYVTQKPYSKDKFKLYFQNPQFMRGWDKDKETDYRATILRYGSKYYLAIMDKKYAKCLQKIDKDDVNGNYEKINYKLLPGPNKMLPRVFFSKKWMAYYNPSEDIQKIYKNGTFKKGDMFNLNDCHKLIDFFKDSISRYPKWSNAYDFNFSETEKYKDIAGFYREVEEQGYKVSFESASKKEVDKLVEEGKLYMFQIYNKDFSDKSHGTPNLHTMYFKLLFDENNHGQIRLSGGAELFMRRASLKKEELVVHPANSPIANKNPDNPKKTTTLSYDVYKDKRFSEDQYELHIPIAINKCPKNIFKINTEVRVLLKHDDNPYVIGIDRGERNLLYIVVVDGKGNIVEQYSLNEIINNFNGIRIKTDYHSLLDKKEKERFEARQNWTSIENIKELKAGYISQVVHKICELVEKYDAVIALEDLNSGFKNSRVKVEKQVYQKFEKMLIDKLNYMVDKKSNPCATGGALKGYQITNKFESFKSMSTQNGFIFYIPAWLTSKIDPSTGFVNLLKTKYTSIADSKKFISSFDRIMYVPEEDLFEFALDYKNFSRTDADYIKKWKLYSYGNRIRIFRNPKKNNVFDWEEVCLTSAYKELFNKYGINYQQGDIRALLCEQSDKAFYSSFMALMSLMLQMRNSITGRTDVDFLISPVKNSDGIFYDSRNYEAQENAILPKNADANGAYNIARKVLWAIGQFKKAEDEKLDKVKIAISNKEWLEYAQTSVKHKRPAATKKAGQAKKKK

SEQ ID NO: 29 - DNA, 3759 bp, Artificial Sequence
  LbCpf1-RR CDS
atggcgccgaagaagaagcgcaaggtgtccaagctcgagaagttcacgaactgctactccctctccaagaccctccgcttcaaggccatccccgtgggcaagacccaggagaacatcgacaacaagcgcctcctggtcgaggacgagaagagggcggaggactacaagggcgtgaagaagctcctggaccgctactacctctccttcatcaacgacgtcctgcacagcatcaagctcaagaacctgaacaactacatctccctgttccgcaagaagacgaggaccgagaaggagaacaaggagctcgagaacctggagatcaacctccgcaaggagatcgccaaggcgttcaagggcaacgagggctacaagagcctgttcaagaaggacatcatcgagacgatcctcccggagttcctggacgacaaggacgagatcgccctcgtgaactccttcaacggcttcaccacggcgttcaccggcttcttcgacaaccgcgagaacatgttcagcgaggaggccaagtccacgagcatcgcgttccgctgcatcaacgagaacctgaccaggtacatctccaacatggacatcttcgagaaggtcgacgccatcttcgacaagcacgaggtgcaggagatcaaggagaagatcctcaacagcgactacgacgtcgaggacttcttcgagggcgagttcttcaacttcgtcctgacgcaggagggcatcgacgtgtacaacgccatcatcggtggcttcgtgaccgagtccggcgagaagatcaagggcctcaacgagtacatcaacctgtacaaccagaagaccaagcagaagctcccgaagttcaagcccctctacaagcaggtcctgtccgaccgcgagtccctgagcttctacggcgagggctacacgagcgacgaggaggtcctcgaggtgttcaggaacaccctgaacaagaacagcgagatcttctccagcatcaagaagctcgagaagctgttcaagaacttcgacgagtactccagcgccggcatcttcgtcaagaacggcccggcgatctccacgatcagcaaggatatcttcggcgagtggaacgtgatcagggacaagtggaacgccgagtacgacgacatccacctcaagaagaaggcggtggtcaccgagaagtacgaggacgaccgcaggaagtccttcaagaagatcggctccttcagcctcgagcagctgcaggagtacgccgacgcggacctctccgtggtcgagaagctgaaggagatcatcatccagaaggtcgacgagatctacaaggtgtacggctccagcgagaagctgttcgacgccgacttcgtcctcgagaagtccctgaagaagaacgacgccgtggtcgcgatcatgaaggacctcctggactccgtgaagagcttcgagaactacatcaaggcgttcttcggcgagggcaaggagacgaaccgcgacgagtccttctacggcgacttcgtcctcgcctacgacatcctcctgaaggtggaccacatctacgacgcgatcaggaactacgtgacccagaagccgtacagcaaggacaagttcaagctgtacttccagaacccccagttcatgcgcggctgggacaaggacaaggagacggactaccgcgccaccatcctccgctacggcagcaagtactacctggccatcatggacaagaagtacgcgaagtgcctccagaagatcgacaaggacgacgtcaacggcaactacgagaagatcaactacaagctcctgccgggccccaacaagatgctgccgagggtgttcttctccaagaagtggatggcctactacaaccccagcgaggacatccagaagatctacaagaacggcacgttcaagaagggcgacatgttcaacctcaacgactgccacaagctgatcgacttcttcaaggactccatcagccgctacccgaagtggtccaacgcctacgacttcaacttcagcgagacagagaagtacaaggacatcgcgggcttctacagggaggtcgaggagcagggctacaaggtgtccttcgagtccgccagcaagaaggaggtcgacaagctcgtggaggagggcaagctgtacatgttccagatctacaacaaggacttctccgacaagagccacggcacgcccaacctccacaccatgtacttcaagctcctgttcgacgagaacaaccacggccagatccgcctctccggcggcgccgagctgttcatgaggagggcgagcctcaagaaggaggagctggtggtccaccccgctaacagcccaatcgcgaacaagaacccggacaaccccaagaagaccacgaccctctcctacgacgtgtacaaggacaagcgcttcagcgaggaccagtacgagctgcacatcccgatcgccatcaacaagtgccccaagaacatcttcaagatcaacaccgaggtcagggtgctcctgaagcacgacgacaacccctacgtgatcggcatcgaccgcggcgagaggaacctcctgtacatcgtggtcgtggacggcaagggcaacatcgtggagcagtactccctgaacgagatcatcaacaacttcaacggcatccgcatcaagacggactaccacagcctcctggacaagaaggagaaggagcgcttcgaggccaggcagaactggacctccatcgagaacatcaaggagctcaaggcgggctacatcagccaggtcgtgcacaagatctgcgagctggtcgagaagtacgacgccgtgatcgcgctcgaggacctgaactccggcttcaagaacagcagggtcaaggtggagaagcaggtctaccagaagttcgagaagatgctcatcgacaagctgaactacatggtggacaagaagtccaacccgtgcgctacgggcggcgcgctcaagggctaccagatcaccaacaagttcgagagcttcaagtccatgagcacccagaacggcttcatcttctacatcccggcctggctgacgtccaagatcgaccccagcaccggcttcgtcaacctcctgaagacgaagtacacctccatcgcggacagcaagaagttcatctccagcttcgaccgcatcatgtatgtgccggaggaggacctcttcgagttcgccctggactacaagaacttctccaggacggacgcggattacatcaagaagtggaagctctacagctacggcaaccgcatcaggatcttccgcaaccccaagaagaacaacgtcttcgactgggaggaggtgtgcctcacctccgcctacaaggagctgttcaacaagtacggcatcaactaccagcagggcgacatcagggcgctcctgtgcgagcagagcgacaaggccttctactccagcttcatggcgctcatgtccctcatgctgcagatgcgcaacagcatcacgggcaggaccgacgtcgacttcctgatctccccggtgaagaacagcgacggcatcttctacgacagccgcaactacgaggcccaggagaacgcgatcctgccaaagaacgcggacgccaacggcgcctacaacatcgcgaggaaggtgctgtgggccatcggccagttcaagaaggcggaggacgagaagctcgacaaggtcaagatcgccatctccaacaaggagtggctggagtacgcgcagacctcggtgaagcacaagaggcccgctgccaccaagaaggcgggccaggccaagaagaagaagtga

SEQ ID NO: 30 - protein, 238 aa, Artificial Sequence
  tdTomato
MVSKGEEVIKEFMRFKVRMEGSMNGHEFEIEGEGEGRPYEGTQTAKLKVTKGGPLPFAWDILSPQFMYGSKAYVKHPADIPDYKKLSFPEGFKWERVMNFEDGGLVTVTQDSSLQDGTLIYKVKMRGTNFPPDGPVMQKKTMGWEASTERLYPRDGVLKGEIHQALKLKDGGHYLVEFKTIYMAKKPVQLPGYYYVDTKLDITSHNEDYTIVEQYERSEGRHHLFLYGMDELYKSRGT

SEQ ID NO: 31 - DNA, 717 bp, Artificial Sequence
  tdTomato
atggtgagcaagggcgaggaggtcatcaaagagttcatgcgcttcaaggtgcgcatggagggctccatgaacggccacgagttcgagatcgagggcgagggcgagggccgcccctacgagggcacccagaccgccaagctgaaggtgaccaagggcggccccctgcccttcgcctgggacatcctgtccccccagttcatgtacggctccaaggcgtacgtgaagcaccccgccgacatccccgattacaagaagctgtccttccccgagggcttcaagtgggagcgcgtgatgaacttcgaggacggcggtctggtgaccgtgacccaggactcctccctgcaggacggcacgctgatctacaaggtgaagatgcgcggcaccaacttcccccccgacggccccgtaatgcagaagaagaccatgggctgggaggcctccaccgagcgcctgtacccccgcgacggcgtgctgaagggcgagatccaccaggccctgaagctgaaggacggcggccactacctggtggagttcaagaccatctacatggccaagaagcccgtgcaactgcccggctactactacgtggacaccaagctggacatcacctcccacaacgaggactacaccatcgtggaacagtacgagcgctccgagggccgccaccacctgttcctgtacggcatggacgagctgtacaagtctagaggtacctga

SEQ ID NO: 32 - DNA, 21 bp, Artificial Sequence
  Protospacer m7GEP336
gcacgttcttgcgcatgagca

SEQ ID NO: 33 - DNA, 21 bp, Artificial Sequence
  Protospacer m7GEP337
gcgccaccgtcgttgacagca

SEQ ID NO: 34 - DNA, 21 bp, Artificial Sequence
  Protospacer m7GEP338
ctgtgcagacaacggcaaccg

SEQ ID NO: 35 - DNA, 21 bp, Artificial Sequence
  Protospacer m7GEP339
agcttctccacctcccagtcg

SEQ ID NO: 36 - protein, 1791 aa, Artificial Sequence; identical to SEQ ID NO: 17
  Zm00008a004913

SEQ ID NO: 37 - protein, 1790 aa, Artificial Sequence
  WVP18-09358-016
MLSGIIDGLTGANKHARLKGTVVLMRKNVLDLNDFGATVVDSISEFLGKGVTCQLISSTLVDANNGNRGRVGAEANLEQWLTSLPSLTTGESKFGVTFDWEVEKLGVPGAVVVKNNHAAEFFLKTITLDDVPGRGAVTFVANSWVYPAGKYRYNRVFFSNDTYLPSQMPAALKPYRDDELRNLRGDDQQGPYQEHDRVYRYDVYNDLGEPDGGNPRPILGGSADHPYPRRCRTGRKPTKTDPNSESRLSLVEQIYVPRDERFGHLKMSDFLGYSIKAITQGIIPAVRTYVDTTPGEFDSFQDIINLYEGGIKLPKIQALEDMRKLFPLQLVKDLLPAGGDYLLKLPIPQIIQGTSRIPIDVRGRLLSGLHIYMCSYEDKNAWRTDEEFAREVLAGVNPMVITRLTEFPPKSTLDPSKYGDHTSTITAEHIEKNLEGLTVQQALDGNRLYILDHHDRFMPFLIDVNNLEGNFIYATRTLFFLRGDGRLAPLAIELSEPYIDGDLTVAKSKVYTPASSGVEAWVWQLAKAYVAVNDSGWHQLVSHWLNTHAVMEPFVIATNRQLSVTHPVHKLLSSHFRDTMTINALARQTLINGGGIFEMTVFPGKYALGMSSVVYKSWNFTEQGLPADLVKRGVAVADPSSPYKVRLLIEDYPYASDGLAIWHAIEQWVGEYLAIYYPDDGALRGDEELQAWKEVREVGHGDHKDAPWWPKMQAVSELASACTTIIWIASALHAAVNFGQYPYAGYLPNRPTVSRRRMPEPGSKEYEELERDPERGFIHTITSQIQTIIGISLIEILSKHSSDEVYLGQRDTPEWTSDARALAAFKRFSDALVKIEGKVVGENRDPQLRNRNGPAEFPYMLLYPNTSDHSEARERAAGQGIHTHTHRTLPEKREARSEERPATMFWHGVADRLTGKNKEAWNEGKIRGTVRLVKKEVLDVGDFNASLLDGVHRILGWDDGVAFQLVSATAADPSNGSRGKVGKAAHLEEAVVSLKSTTDGETVYRVSFEWDGSQGVPGAVLVRNLQHAEFFLKSLTLEGVPGRGTVVFVANSWIYPHNLYSQERVFFANDTYLPSKMPAALVPYRQDELKILRGDDNPGPYKEHDRVYRYDYYNDLGEPDKGEDHARPVLGGSQEHPYPRRCRTGRRPTETDPNSESRLFLLNLNIYVPRDERFGHLKMSDFLGYSLKAIIEAVLPTLGTFVDDTPKEFDSFEDILGLYEPGPEAPNNPLVAEVRKRIPSEFLRSILPNGSHDHPLKMPLPNIIRSDVLKKAPEFKFGWRTDEEFARETLAGVNPVLIKRLTEFPAKSTLDPSQYGDHTSKITEAHIQHNMEGLSVQNALKKNRLFILDHHDHFMPYLNKINELEGNFIYASRTLLFLKDDGTLKPLAVELSLPHPDGQQHGAVSKVYTPAHSGAEGHVWQLAKAYACVNDSAWHQLISHWLNTHAVIEPFVIATNRQLSVVHPVHKLLSPHYRDTLNINALARQTLINADGIFERTVFPAKYALGMSSDVYKSWNFNEQALPADLVKRGVAVPDQSSPYGVRLLIKDYPYAVDGLVIWWAIERWVKEYLDVYYPNDGELQRDVELQAWWKEVREEAHGDLKDRDWWPRMDAVQRLARACTTVIWVASALHAAVNFGQYPYAGYLPNRPTVSRRPMPEPGSDDYKKLEAGQKEADAVFIRTITSQFQTILGISLIEILSKHSSDEVYLGQRDEPERWTSDARALDAFRRFGSRLVEIEKRIRTMNDSPTLKNRKGPVEMPYMLLYPNTSDVTGEKGEGLTAMGIPNSISI

SEQ ID NO: 38 - protein, 1791 aa, Artificial Sequence
  WVP18-09344-014
MLSGIIDGLTGANKHARLKGTVVLMRKNVLDLNDFGATVVDSISEFLGKGVTCQLISSTLVDANNGNRGRVGAEANLEQWLTSLPSLTTGESKFGVTFDWEVEKLGVPGAVVVKNNHAAEFFLKTITLDDVPGRGAVTFVANSWVYPAGKYRYNRVFFSNDTYLPSQMPAALKPYRDDELRNLRGDDQQGPYQEHDRVYRYDVYNDLGEPDGGNPRPILGGSADHPYPRRCRTGRKPTKTDPNSESRLSLVEQIYVPRDERFGHLKMSDFLGYSIKAITQGIIPAVRTYVDTTPGEFDSFQDIINLYEGGIKLPKIQALEDMRKLFPLQLVKDLLPAGGDYLLKLPIPQIIQGTSRIPIDVRGRLLSGLHIYMCSYEDKNAWRTDEEFAREVLAGVNPMVITRLTEFPPKSTLDPSKYGDHTSTITAEHIEKNLEGLTVQQALDGNRLYILDHHDRFMPFLIDVNNLEGNFIYATRTLFFLRGDGRLAPLAIELSEPYIDGDLTVAKSKVYTPASSGVEAWVWQLAKAYVAVNDSGWHQLVSHWLNTHAVMEPFVIATNRQLSVTHPVHKLLSSHFRDTMTINALARQTLINGGGIFEMTVFPGKYALGMSSVVYKSWNFTEQGLSADLVKRGVAVADPSSPYKVRLLIEDYPYASDGLAIWHAIEQWVGEYLAIYYPDDGALRGDEELQAWWKEVREVGHGDHKDAPWWPKMQAVSELASACTTIIWIASALHAAVNFGQYPYAGYLPNRPTVSRRRMPEPGSKEYEELERDPERGFIHTITSQIQTIIGISLIEILSKHSSDEVYLGQRDTPEWTSDARALAAFKRFSDALVKIEGKVVGENRDPQLRNRNGPAEFPYMLLYPNTSDHSEARERAAGQGIHTHTHRTLPEKREARSEERPATMFWHGVADRLTGKNKEAWNEGKIRGTVRLVKKEVLDVGDFNASLLDGVHRILGWDDGVAFQLVSATAADPSNGSRGKVGKAAHLEEAVVSLKSTTDGETVYRVSFEWDGSQGVPGAVLVRNLQHAEFFLKSLTLEGVPGRGTVVFVANSWIYPHNLYSQERVFFANDTYLPSKMPAALVPYRQDELKILRGDDNPGPYKEHDRVYRYDYYNDLGEPDKGEDHARPVLGGSQEHPYPRRCRTGRRPTETDPNSESRLFLLNLNIYVPRDERFGHLKMSDFLGYSLKAIIEAVLPTLGTFVDDTPKEFDSFEDILGLYEPGPEAPNNPLVAEVRKRIPSEFLRSILPNGSHDHPLKMPLPNIIRSDVLKKAPEFKFGWRTDEEFARETLAGVNPVLIKRLTEFPAKSTLDPSQYGDHTSKITEAHIQHNMEGLSVQNALKKNRLFILDHHDHFMPYLNKINELEGNFIYASRTLLFLKDDGTLKPLAVELSLPHPDGQQHGAVSKVYTPAHSGAEGHVWQLAKAYACVNDSAWHQLISHWLNTHAVIEPFVIATNRQLSVVHPVHKLLSPHYRDTLNINALARQTLINADGIFERTVFPAKYALGMSSDVYKSWNFNEQALPADLVKRGVAVPDQSSPYGVRLLIKDYPYAVDGLVIWWAIERWVKEYLDVYYPNDGELQRDVELQAWWKEVREEAHGDLKDRDWWPRMDAVQRLARACTTVIWVASALHAAVNFGQYPYAGYLPNRPTVSRRPMPEPGSDDYKKLEAGQKEADAVFIRTITSQFQTILGISLIEILSKHSSDEVYLGQRDEPERWTSDARALDAFRRFGSRLVEIEKRIRTMNDSPTLKNRKGPVEMPYMLLYPNTSDVTGEKGEGLTAMGIPNSISI

SEQ ID NO: 39 - protein, 1790 aa, Artificial Sequence
  WVP18-09309-014_339-009
MLSGIIDGLTGANKHARLKGTVVLMRKNVLDLNDFGATVVDSISEFLGKGVTCQLISSTLVDANNGNRGRVGAEANLEQWLTSLPSLTTGESKFGVTFDWEVEKLGVPGAVVVKNNHAAEFFLKTITLDDVPGRGAVTFVANSWVYPAGKYRYNRVFFSNDTYLPSQMPAALKPYRDDELRNLRGDDQQGPYQEHDRVYRYDVYNDLGEPDGGNPRPILGGSADHPYPRRCRTGRKPTKTDPNSESRLSLVEQIYVPRDERFGHLKMSDFLGYSIKAITQGIIPAVRTYVDTTPGEFDSFQDIINLYEGGIKLPKIQALEDMRKLFPLQLVKDLLPAGGDYLLKLPIPQIIQGTSRIPIDVRGRLLSGLHIYMCSYEDKNAWRTDEEFAREVLAGVNPMVITRLTEFPPKSTLDPSKYGDHTSTITAEHIEKNLEGLTVQQALDGNRLYILDHHDRFMPFLIDVNNLEGNFIYATRTLFFLRGDGRLAPLAIELSEPYIDGDLTVAKSKVYTPASSGVEAWVWQLAKAYVAVNDSGWHQLVSHWLNTHAVMEPFVIATNRQLSVTHPVHKLLSSHFRDTMTINALARQTLINGGGIFEMTVFPGKYALGMSSVVYKSWNFTEQGLPADLVKRGVAVADPSSPYKVRLLIEDYPYASDGLAIWHAIEQVGEYLAIYYPDDGALRGDEELQAWWKEVREVGHGDHKDAPWWPKMQAVSELASACTTIIWIASALHAAVNFGQYPYAGYLPNRPTVSRRRMPEPGSKEYEELERDPERGFIHTITSQIQTIIGISLIEILSKHSSDEVYLGQRDTPEWTSDARALAAFKRFSDALVKIEGKVVGENRDPQLRNRNGPAEFPYMLLYPNTSDHSEARERAAGQGIHTHTHRTLPEKREARSEERPATMFWHGVADRLTGKNKEAWNEGKIRGTVRLVKKEVLDVGDFNASLLDGVHRILGWDDGVAFQLVSATAADPSNGSRGKVGKAAHLEEAVVSLKSTTDGETVYRVSFEWDGSQGVPGAVLVRNLQHAEFFLKSLTLEGVPGRGTVVFVANSWIYPHNLYSQERVFFANDTYLPSKMPAALVPYRQDELKILRGDDNPGPYKEHDRVYRYDYYNDLGEPDKGEDHARPVLGGSQEHPYPRRCRTGRRPTETDPNSESRLFLLNLNIYVPRDERFGHLKMSDFLGYSLKAIIEAVLPTLGTFVDDTPKEFDSFEDILGLYEPGPEAPNNPLVAEVRKRIPSEFLRSILPNGSHDHPLKMPLPNIIRSDVLKKAPEFKFGWRTDEEFARETLAGVNPVLIKRLTEFPAKSTLDPSQYGDHTSKITEAHIQHNMEGLSVQNALKKNRLFILDHHDHFMPYLNKINELEGNFIYASRTLLFLKDDGTLKPLAVELSLPHPDGQQHGAVSKVYTPAHSGAEGHVWQLAKAYACVNDSAWHQLISHWLNTHAVIEPFVIATNRQLSVVHPVHKLLSPHYRDTLNINALARQTLINADGIFERTVFPAKYALGMSSDVYKSWNFNEQALPADLVKRGVAVPDQSSPYGVRLLIKDYPYAVDGLVIWWAIERWVKEYLDVYYPNDGELQRDVELQAWWKEVREEAHGDLKDRDWWPRMDAVQRLARACTTVIWVASALHAAVNFGQYPYAGYLPNRPTVSRRPMPEPGSDDYKKLEAGQKEADAVFIRTITSQFQTILGISLIEILSKHSSDEVYLGQRDEPERWTSDARALDAFRRFGSRLVEIEKRIRTMNDSPTLKNRKGPVEMPYMLLYPNTSDVTGEKGEGLTAMGIPNSISI

SEQ ID NO: 40 - protein, 1791 aa, Artificial Sequence
  WVP18-09307-014
MLSGIIDGLTGANKHARLKGTVVLMRKNVLDLNDFGATVVDSISEFLGKGVTCQLISSTLVDANNGNRGRVGAEANLEQWLTSLPSLTTGESKFGVTFDWEVEKLGVPGAVVVKNNHAAEFFLKTITLDDVPGRGAVTFVANSWVYPAGKYRYNRVFFSNDTYLPSQMPAALKPYRDDELRNLRGDDQQGPYQEHDRVYRYDVYNDLGEPDGGNPRPILGGSADHPYPRRCRTGRKPTKTDPNSESRLSLVEQIYVPRDERFGHLKMSDFLGYSIKAITQGIIPAVRTYVDTTPGEFDSFQDIINLYEGGIKLPKIQALEDMRKLFPLQLVKDLLPAGGDYLLKLPIPQIIQGTSRIPIDVRGRLLSGLHIYMCSYEDKNAWRTDEEFAREVLAGVNPMVITRLTEFPPKSTLDPSKYGDHTSTITAEHIEKNLEGLTVQQALDGNRLYILDHHDRFMPFLIDVNNLEGNFIYATRTLFFLRGDGRLAPLAIELSEPYIDGDLTVAKSKVYTPASSGVEAWVWQLAKAYVAVNDSGWHQLVSHWLNTHAVMEPFVIATNRQLSVTHPVHKLLSSHFRDTMTINALARQTLINGGGIFEMTVFPGKYALGMSSVVYKSWNFTEQGLPADLVKRGVAVADPSSPYKVRLLIEDYPYASDGLAIWHAIEQWVGEYLAIYYPDDGALRGDEELQAWWKEVREVGHGDHKDAPWWPKMQAVSELASACTTIIWIASALHAAVNFGQYPYAGYLPNRPTVSRRRMPEPSSKEYEELERDPERGFIHTITSQIQTIIGISLIEILSKHSSDEVYLGQRDTPEWTSDARALAAFKRFSDALVKIEGKVVGENRDPQLRNRNGPAEFPYMLLYPNTSDHSEARERAAGQGIHTHTHRTLPEKREARSEERPATMFWHGVADRLTGKNKEAWNEGKIRGTVRLVKKEVLDVGDFNASLLDGVHRILGWDDGVAFQLVSATAADPSNGSRGKVGKAAHLEEAVVSLKSTTDGETVYRVSFEWDGSQGVPGAVLVRNLQHAEFFLKSLTLEGVPGRGTVVFVANSWIYPHNLYSQERVFFANDTYLPSKMPAALVPYRQDELKILRGDDNPGPYKEHDRVYRYDYYNDLGEPDKGEDHARPVLGGSQEHPYPRRCRTGRRPTETDPNSESRLFLLNLNIYVPRDERFGHLKMSDFLGYSLKAIIEAVLPTLGTFVDDTPKEFDSFEDILGLYEPGPEAPNNPLVAEVRKRIPSEFLRSILPNGSHDHPLKMPLPNIIRSDVLKKAPEFKFGWRTDEEFARETLAGVNPVLIKRLTEFPAKSTLDPSQYGDHTSKITEAHIQHNMEGLSVQNALKKNRLFILDHHDHFMPYLNKINELEGNFIYASRTLLFLKDDGTLKPLAVELSLPHPDGQQHGAVSKVYTPAHSGAEGHVWQLAKAYACVNDSAWHQLISHWLNTHAVIEPFVIATNRQLSVVHPVHKLLSPHYRDTLNINALARQTLINADGIFERTVFPAKYALGMSSDVYKSWNFNEQALPADLVKRGVAVPDQSSPYGVRLLIKDYPYAVDGLVIWWAIERWVKEYLDVYYPNDGELQRDVELQAWWKEVREEAHGDLKDRDWWPRMDAVQRLARACTTVIWVASALHAAVNFGQYPYAGYLPNRPTVSRRPMPEPGSDDYKKLEAGQKEADAVFIRTITSQFQTILGISLIEILSKHSSDEVYLGQRDEPERWTSDARALDAFRRFGSRLVEIEKRIRTMNDSPTLKNRKGPVEMPYMLLYPNTSDVTGEKGEGLTAMGIPNSISI

SEQ ID NO: 41 - DNA, 5376 bp, Artificial Sequence; identical to SEQ ID NO: 16
  Zm00008a004913

SEQ ID NO: 42 - DNA, 5376 bp, Artificial Sequence
  WVP18-09358-016
atgctgagcgggatcatcgacgggctgacgggggcgaacaagcatgcgcggctcaagggcacggtggtgctcatgcgcaagaacgtgctggacctcaacgacttcggcgccaccgtcgtcgacagcatcagcgagttcctcggcaagggggtcacctgccagctcatcagctccactctcgtcgacgccaacaacggcaaccgcgggcgggtcggggcggaggcgaacctggagcagtggctgacgagcctgccgtcgctgacgaccggcgagtccaagttcggcgtcacgttcgactgggaggtggagaagctgggagtgccgggggccgtcgtcgtcaagaacaaccacgccgccgagttcttcctcaagacaatcaccctcgacgacgtgcccggccgcggcgccgtcaccttcgtcgccaactcctgggtctaccccgcgggcaagtaccgctacaaccgcgtcttcttctccaacgatacgtacctgccaagccagatgccggcggcgctgaagccgtaccgcgacgacgagctccgcaacctccgcggcgacgaccagcagggcccctaccaggagcacgaccgcgtgtaccgctacgacgtctacaacgacctcggcgagcccgacggcggcaacccgcgccccatcctcggcggctccgccgaccacccgtacccgcgccgctgccgcacgggccgcaagcccaccaaaaccgaccccaactcggagagccgactgtcgctggtggagcagatctacgtgccgcgggacgagcgcttcggccacctcaagatgtccgacttcctgggctactccatcaaggccatcacgcagggcatcatcccggcggtgcgcacgtacgtggacaccaccccgggcgagttcgactccttccaggacatcatcaacctgtacgagggcgggatcaagctgcccaagatccaggcgctcgaggacatgcgcaagctcttcccgctccagctcgtcaaggacctcctccccgccggcggggactacctgctcaagctccccatcccacagatcatccaaggcacgtcacgtataccgatcgatgtcaggggccggctgttgtctggtctgcatatatatatgtgctcctatgaggacaagaacgcgtggaggaccgacgaggagttcgcgcgggaggtgctcgccggcgtcaacccgatggtgatcacgcgcctcacggagttcccgcccaagagcacgctggaccccagcaagtacggcgaccacaccagcacgatcacggcggagcacatcgagaagaacctcgagggcctcacggtgcagcaggcgctggacggcaacaggctctacatcctggaccaccacgaccgcttcatgccgttcctcatcgacgtcaacaacctggagggcaacttcatctacgccaccaggacgctcttcttcctgcgcggcgacggcaggctcgcgcccctcgccatcgagctcagcgagccgtacatcgacggggacctcaccgtggccaagagcaaggtctacacgccggcgtccagcggcgtcgaggcctgggtgtggcagctcgccaaggcctatgtcgccgtcaacgactctggctggcaccaactcgtcagccactggctgaacacccacgcggtgatggagccgttcgtgatcgcgacgaaccggcagctgagcgtgacgcacccggtgcacaagctcctgagctcgcacttccgcgacaccatgaccatcaacgcgctggcgcggcagacgctcatcaacggcggcggcatcttcgagatgaccgtcttcccgggcaagtacgcgctgggcatgtcctccgtggtgtacaagagctggaacttcaccgagcagggcctccccgccgacctcgtcaagaggggcgtggcggtggcggacccgtccagcccgtacaaggtgcggctgctgatcgaggactacccgtacgcgagcgacgggctggccatctggcacgccatcgagcagtgggtgggcgagtacctggccatctactaccccgacgacggcgcgctgcggggcgacgaggagctgcaggcgtggtgaaaggaggtgcgcgaggtcgggcacggcgaccacaaggacgcgccctggtggcccaagatgcaggccgtgtcggagctcgccagcgcctgcaccaccatcatctggatcgcgtcggcgctccacgccgccgtcaacttcggccagtacccgtacgcggggtacctcccgaacaggcccacggtgagccggcgccggatgccggagcccggcagcaaggagtacgaggagctggagcgcgacccggagcgcggcttcatccacaccatcacgagccagatccagaccatcatcggcatctcgctcatcgagatcctctccaagcactcctccgacgaggtgtacctcggccagcgcgacacccccgagtggacctccgacgcccgggcgctggcggcgttcaagaggttcagcgacgcgctggtcaagatcgagggcaaggtggtgggcgagaaccgcgacccgcagctgaggaacaggaacggccccgccgagttcccctacatgctgctctatcccaacacctctgaccacagcgaggcgagggagcgagcagcagggcaaggcatccacacccacacccaccggacactccctgagaagcgagaagcgagaagcgaagagcggccggccaccatgttctggcacggggtcgcggaccggctgacggggaagaacaaggaggcgtggaacgagggaaagatccgcggcacggtgaggctggtcaagaaggaggtgctggacgtcggcgacttcaacgcctcgctcctcgacggcgtacacaggatcctcggctgggacgacggcgtcgccttccagctcgtcagcgccaccgcggccgaccccagcaacgggagccgcggcaaggtcgggaaggcggcgcacctggaggaggcggtggtgtcgctcaagtcgacgacggacggggagaccgtgtaccgggtgagcttcgagtgggacgggtcgcagggcgtcccgggcgccgtcctggtcaggaacctgcagcacgccgagttcttcctcaagtcgctcaccctcgagggcgtccccggcaggggcaccgtcgtcttcgtcgccaactcgtggatctacccgcacaatctctactcccaggaacgcgtcttcttcgccaacgacacttatctgccaagcaaaatgcctgcggcattggtgccttaccggcaggacgagctcaagattctccgcggcgacgataatcctggaccatacaaggagcacgaccgcgtctaccgttacgactactacaacgacctcggtgagccagacaagggtgaagaccatgcccggcctgtcctcgggggcagccaagaacacccgtatccccgtcgctgcaggaccggccggcgtccaacagagacagaccccaactcggagagcaggctgtttctgctgaacctgaacatctacgtcccgcgcgacgagcggtttgggcatctcaagatgtcggacttcctcgggtactcactgaaggcgatcatcgaggctgtccttccgacgctggggacgttcgtcgacgatacgcccaaggagttcgattcgttcgaagacatccttgggctctacgagccgggtccagaggcgcccaacaacccactggtagcagaggtcaggaagagaatccccagcgagttcctcagaagcattctgcccaatggtagccatgaccaccccctgaagatgccccttccaaatatcatcagatcagatgtgttgaaaaaggctccagagtttaagtttggctggaggaccgacgaagagtttgcgagggagacgcttgcaggcgtgaacccagtgctcatcaaacgtctgacggagttcccagctaaaagtaccctggacccaagtcaatacggagaccatacgagcaagatcaccgaagctcacatccagcataacatggaaggcctgtcagtgcagaatgcactgaagaagaacaggctcttcatcctagaccaccatgaccatttcatgccgtacctcaacaagatcaacgagttggaggggaacttcatctacgccagcaggaccctactgttcctgaaggacgatggcacgctgaagcccctggccgtcgagctgagcctgccccaccctgatggccagcagcacggcgcggtcagcaaggtgtacaccccagctcactccggcgctgagggccacgtctggcaacttgccaaggcttatgcctgcgtgaacgactccgcctggcatcagctgatcagccactggctgaacacgcacgcggtgatcgagccgttcgtcatcgcaacgaaccggcagctgagcgtggtgcatccagtgcacaagctgctgagcccacactaccgtgacacgctgaacatcaacgccctggcacgccagacgctcatcaacgccgacggcatcttcgagcgcaccgtgttccctgcaaagtacgcgctggggatgtcctccgacgtgtacaagagctggaatttcaacgagcaggctctcccagcagacctcgtcaagagaggtgtggctgtgccggaccagtcgagcccctacggtgtccggttgctgatcaaggactacccttacgccgtggacgggctggtcatctggtgggcgatcgagcggtgggtcaaggagtacctggacgtctactaccccaacgacggcgagctccagcgcgacgtggagctgcaggcgtggtggaaggaggtgcgcgaggaggcgcacggcgacctcaaggaccgagactggtggcccaggatggacgccgtccagcggctggccagggcgtgcacgaccgtcatctgggtagcgtccgcgctgcacgcggccgtcaacttcgggcagtacccgtacgccgggtacctgccgaaccggccgaccgtgagccggcggccgatgccggagccgggcagcgacgactacaagaagctggaggcggggcagaaggaggcggacgcggtgttcatccgcaccatcaccagccagttccagaccatcctgggcatctcgctcatcgagatcctctccaagcactcctccgacgaggtgtacctcggccagcgcgacgagcctgagcgctggacgtcggacgccagggcgctggacgcgttcagaaggttcggaagccggctggtggagatcgagaagcggatcaggacgatgaacgacagcccgacgttgaagaaccggaaggggccggtggagatgccgtacatgctgctgtaccccaacacgtcggatgtcaccggcgagaagggcgaggggctcactgccatgggcattcccaacagcatctccatatga

SEQ ID NO: 43 - DNA, 5376 bp, Artificial Sequence
  WVP18-09344-014
atgctgagcgggatcatcgacgggctgacgggggcgaacaagcatgcgcggctcaagggcacggtggtgctcatgcgcaagaacgtgctggacctcaacgacttcggcgccaccgtcgtcgacagcatcagcgagttcctcggcaagggggtcacctgccagctcatcagctccactctcgtcgacgccaacaacggcaaccgcgggcgggtcggggcggaggcgaacctggagcagtggctgacgagcctgccgtcgctgacgaccggcgagtccaagttcggcgtcacgttcgactgggaggtggagaagctgggagtgccgggggccgtcgtcgtcaagaacaaccacgccgccgagttcttcctcaagacaatcaccctcgacgacgtgcccggccgcggcgccgtcaccttcgtcgccaactcctgggtctaccccgcgggcaagtaccgctacaaccgcgtcttcttctccaacgatacgtacctgccaagccagatgccggcggcgctgaagccgtaccgcgacgacgagctccgcaacctccgcggcgacgaccagcagggcccctaccaggagcacgaccgcgtgtaccgctacgacgtctacaacgacctcggcgagcccgacggcggcaacccgcgccccatcctcggcggctccgccgaccacccgtacccgcgccgctgccgcacgggccgcaagcccaccaaaaccgaccccaactcggagagccgactgtcgctggtggagcagatctacgtgccgcgggacgagcgcttcggccacctcaagatgtccgacttcctgggctactccatcaaggccatcacgcagggcatcatcccggcggtgcgcacgtacgtggacaccaccccgggcgagttcgactccttccaggacatcatcaacctgtacgagggcgggatcaagctgcccaagatccaggcgctcgaggacatgcgcaagctcttcccgctccagctcgtcaaggacctcctccccgccggcggggactacctgctcaagctccccatcccacagatcatccaaggcacgtcacgtataccgatcgatgtcaggggccggctgttgtctggtctgcatatatatatgtgctcctatgaggacaagaacgcgtggaggaccgacgaggagttcgcgcgggaggtgctcgccggcgtcaacccgatggtgatcacgcgcctcacggagttcccgcccaagagcacgctggaccccagcaagtacggcgaccacaccagcacgatcacggcggagcacatcgagaagaacctcgagggcctcacggtgcagcaggcgctggacggcaacaggctctacatcctggaccaccacgaccgcttcatgccgttcctcatcgacgtcaacaacctggagggcaacttcatctacgccaccaggacgctcttcttcctgcgcggcgacggcaggctcgcgcccctcgccatcgagctcagcgagccgtacatcgacggggacctcaccgtggccaagagcaaggtctacacgccggcgtccagcggcgtcgaggcctgggtgtggcagctcgccaaggcctatgtcgccgtcaacgactctggctggcaccaactcgtcagccactggctgaacacccacgcggtgatggagccgttcgtgatcgcgacgaaccggcagctgagcgtgacgcacccggtgcacaagctcctgagctcgcacttccgcgacaccatgaccatcaacgcgctggcgcggcagacgctcatcaacggcggcggcatcttcgagatgaccgtcttcccgggcaagtacgcgctgggcatgtcctccgtggtgtacaagagctggaacttcaccgagcagggcctctccgccgacctcgtcaagaggggcgtggcggtggcggacccgtccagcccgtacaaggtgcggctgctgatcgaggactacccgtacgcgagcgacgggctggccatctggcacgccatcgagcagtgggtgggcgagtacctggccatctactaccccgacgacggcgcgctgcggggcgacgaggagctgcaggcgtggtggaaggaggtgcgcgaggtcgggcacggcgaccacaaggacgcgccctggtggcccaagatgcaggccgtgtcggagctcgccagcgcctgcaccaccatcatctggatcgcgtcggcgctccacgccgccgtcaacttcggccagtacccgtacgcggggtacctcccgaacaggcccacggtgagccggcgccggatgccggagcccggcagcaaggagtacgaggagctggagcgcgacccggagcgcggcttcatccacaccatcacgagccagatccagaccatcatcggcatctcgctcatcgagatcctctccaagcactcctccgacgaggtgtacctcggccagcgcgacacccccgagtggacctccgacgcccgggcgctggcggcgttcaagaggttcagcgacgcgctggtcaagatcgagggcaaggtggtgggcgagaaccgcgacccgcagctgaggaacaggaacggccccgccgagttcccctacatgctgctctatcccaacacctctgaccacagcgaggcgagggagcgagcagcagggcaaggcatccacacccacacccaccggacactccctgagaagcgagaagcgagaagcgaagagcggccggccaccatgttctggcacggggtcgcggaccggctgacggggaagaacaaggaggcgtggaacgagggaaagatccgcggcacggtgaggctggtcaagaaggaggtgctggacgtcggcgacttcaacgcctcgctcctcgacggcgtacacaggatcctcggctgggacgacggcgtcgccttccagctcgtcagcgccaccgcggccgaccccagcaacgggagccgcggcaaggtcgggaaggcggcgcacctggaggaggcggtggtgtcgctcaagtcgacgacggacggggagaccgtgtaccgggtgagcttcgagtgggacgggtcgcagggcgtcccgggcgccgtcctggtcaggaacctgcagcacgccgagttcttcctcaagtcgctcaccctcgagggcgtccccggcaggggcaccgtcgtcttcgtcgccaactcgtggatctacccgcacaatctctactcccaggaacgcgtcttcttcgccaacgacacttatctgccaagcaaaatgcctgcggcattggtgccttaccggcaggacgagctcaagattctccgcggcgacgataatcctggaccatacaaggagcacgaccgcgtctaccgttacgactactacaacgacctcggtgagccagacaagggtgaagaccatgcccggcctgtcctcgggggcagccaagaacacccgtatccccgtcgctgcaggaccggccggcgtccaacagagacagaccccaactcggagagcaggctgtttctgctgaacctgaacatctacgtcccgcgcgacgagcggtttgggcatctcaagatgtcggacttcctcgggtactcactgaaggcgatcatcgaggctgtccttccgacgctggggacgttcgtcgacgatacgcccaaggagttcgattcgttcgaagacatccttgggctctacgagccgggtccagaggcgcccaacaacccactggtagcagaggtcaggaagagaatccccagcgagttcctcagaagcattctgcccaatggtagccatgaccaccccctgaagatgccccttccaaatatcatcagatcagatgtgttgaaaaaggctccagagtttaagtttggctggaggaccgacgaagagtttgcgagggagacgcttgcaggcgtgaacccagtgctcatcaaacgtctgacggagttcccagctaaaagtaccctggacccaagtcaatacggagaccatacgagcaagatcaccgaagctcacatccagcataacatggaaggcctgtcagtgcagaatgcactgaagaagaacaggctcttcatcctagaccaccatgaccatttcatgccgtacctcaacaagatcaacgagttggaggggaacttcatctacgccagcaggaccctactgttcctgaaggacgatggcacgctgaagcccctggccgtcgagctgagcctgccccaccctgatggccagcagcacggcgcggtcagcaaggtgtacaccccagctcactccggcgctgagggccacgtctggcaacttgccaaggcttatgcctgcgtgaacgactccgcctggcatcagctgatcagccactggctgaacacgcacgcggtgatcgagccgttcgtcatcgcaacgaaccggcagctgagcgtggtgcatccagtgcacaagctgctgagcccacactaccgtgacacgctgaacatcaacgccctggcacgccagacgctcatcaacgccgacggcatcttcgagcgcaccgtgttccctgcaaagtacgcgctggggatgtcctccgacgtgtacaagagctggaatttcaacgagcaggctctcccagcagacctcgtcaagagaggtgtggctgtgccggaccagtcgagcccctacggtgtccggttgctgatcaaggactacccttacgccgtggacgggctggtcatctggtgggcgatcgagcggtgggtcaaggagtacctggacgtctactaccccaacgacggcgagctccagcgcgacgtggagctgcaggcgtggtggaaggaggtgcgcgaggaggcgcacggcgacctcaaggaccgagactggtggcccaggatggacgccgtccagcggctggccagggcgtgcacgaccgtcatctgggtagcgtccgcgctgcacgcggccgtcaacttcgggcagtacccgtacgccgggtacctgccgaaccggccgaccgtgagccggcggccgatgccggagccgggcagcgacgactacaagaagctggaggcggggcagaaggaggcggacgcggtgttcatccgcaccatcaccagccagttccagaccatcctgggcatctcgctcatcgagatcctctccaagcactcctccgacgaggtgtacctcggccagcgcgacgagcctgagcgctggacgtcggacgccagggcgctggacgcgttcagaaggttcggaagccggctggtggagatcgagaagcggatcaggacgatgaacgacagcccgacgttgaagaaccggaaggggccggtggagatgccgtacatgctgctgtaccccaacacgtcggatgtcaccggcgagaagggcgaggggctcactgccatgggcattcccaacagcatctccatatga

SEQ ID NO: 44 - DNA, 5376 bp, Artificial Sequence
  WVP18-09309-014_339-009
atgctgagcgggatcatcgacgggctgacgggggcgaacaagcatgcgcggctcaagggcacggtggtgctcatgcgcaagaacgtgctggacctcaacgacttcggcgccaccgtcgtcgacagcatcagcgagttcctcggcaagggggtcacctgccagctcatcagctccactctcgtcgacgccaacaacggcaaccgcgggcgggtcggggcggaggcgaacctggagcagtggctgacgagcctgccgtcgctgacgaccggcgagtccaagttcggcgtcacgttcgactgggaggtggagaagctgggagtgccgggggccgtcgtcgtcaagaacaaccacgccgccgagttcttcctcaagacaatcaccctcgacgacgtgcccggccgcggcgccgtcaccttcgtcgccaactcctgggtctaccccgcgggcaagtaccgctacaaccgcgtcttcttctccaacgatacgtacctgccaagccagatgccggcggcgctgaagccgtaccgcgacgacgagctccgcaacctccgcggcgacgaccagcagggcccctaccaggagcacgaccgcgtgtaccgctacgacgtctacaacgacctcggcgagcccgacggcggcaacccgcgccccatcctcggcggctccgccgaccacccgtacccgcgccgctgccgcacgggccgcaagcccaccaaaaccgaccccaactcggagagccgactgtcgctggtggagcagatctacgtgccgcgggacgagcgcttcggccacctcaagatgtccgacttcctgggctactccatcaaggccatcacgcagggcatcatcccggcggtgcgcacgtacgtggacaccaccccgggcgagttcgactccttccaggacatcatcaacctgtacgagggcgggatcaagctgcccaagatccaggcgctcgaggacatgcgcaagctcttcccgctccagctcgtcaaggacctcctccccgccggcggggactacctgctcaagctccccatcccacagatcatccaaggcacgtcacgtataccgatcgatgtcaggggccggctgttgtctggtctgcatatatatatgtgctcctatgaggacaagaacgcgtggaggaccgacgaggagttcgcgcgggaggtgctcgccggcgtcaacccgatggtgatcacgcgcctcacggagttcccgcccaagagcacgctggaccccagcaagtacggcgaccacaccagcacgatcacggcggagcacatcgagaagaacctcgagggcctcacggtgcagcaggcgctggacggcaacaggctctacatcctggaccaccacgaccgcttcatgccgttcctcatcgacgtcaacaacctggagggcaacttcatctacgccaccaggacgctcttcttcctgcgcggcgacggcaggctcgcgcccctcgccatcgagctcagcgagccgtacatcgacggggacctcaccgtggccaagagcaaggtctacacgccggcgtccagcggcgtcgaggcctgggtgtggcagctcgccaaggcctatgtcgccgtcaacgactctggctggcaccaactcgtcagccactggctgaacacccacgcggtgatggagccgttcgtgatcgcgacgaaccggcagctgagcgtgacgcacccggtgcacaagctcctgagctcgcacttccgcgacaccatgaccatcaacgcgctggcgcggcagacgctcatcaacggcggcggcatcttcgagatgaccgtcttcccgggcaagtacgcgctgggcatgtcctccgtggtgtacaagagctggaacttcaccgagcagggcctccccgccgacctcgtcaagaggggcgtggcggtggcggacccgtccagcccgtacaaggtgcggctgctgatcgaggactacccgtacgcgagcgacgggctggccatctggcacgccatcgagcagtgagtgggcgagtacctggccatctactaccccgacgacggcgcgctgcggggcgacgaggagctgcaggcgtggtggaaggaggtgcgcgaggtcgggcacggcgaccacaaggacgcgccctggtggcccaagatgcaggccgtgtcggagctcgccagcgcctgcaccaccatcatctggatcgcgtcggcgctccacgccgccgtcaacttcggccagtacccgtacgcggggtacctcccgaacaggcccacggtgagccggcgccggatgccggagcccggcagcaaggagtacgaggagctggagcgcgacccggagcgcggcttcatccacaccatcacgagccagatccagaccatcatcggcatctcgctcatcgagatcctctccaagcactcctccgacgaggtgtacctcggccagcgcgacacccccgagtggacctccgacgcccgggcgctggcggcgttcaagaggttcagcgacgcgctggtcaagatcgagggcaaggtggtgggcgagaaccgcgacccgcagctgaggaacaggaacggccccgccgagttcccctacatgctgctctatcccaacacctctgaccacagcgaggcgagggagcgagcagcagggcaaggcatccacacccacacccaccggacactccctgagaagcgagaagcgagaagcgaagagcggccggccaccatgttctggcacggggtcgcggaccggctgacggggaagaacaaggaggcgtggaacgagggaaagatccgcggcacggtgaggctggtcaagaaggaggtgctggacgtcggcgacttcaacgcctcgctcctcgacggcgtacacaggatcctcggctgggacgacggcgtcgccttccagctcgtcagcgccaccgcggccgaccccagcaacgggagccgcggcaaggtcgggaaggcggcgcacctggaggaggcggtggtgtcgctcaagtcgacgacggacggggagaccgtgtaccgggtgagcttcgagtgggacgggtcgcagggcgtcccgggcgccgtcctggtcaggaacctgcagcacgccgagttcttcctcaagtcgctcaccctcgagggcgtccccggcaggggcaccgtcgtcttcgtcgccaactcgtggatctacccgcacaatctctactcccaggaacgcgtcttcttcgccaacgacacttatctgccaagcaaaatgcctgcggcattggtgccttaccggcaggacgagctcaagattctccgcggcgacgataatcctggaccatacaaggagcacgaccgcgtctaccgttacgactactacaacgacctcggtgagccagacaagggtgaagaccatgcccggcctgtcctcgggggcagccaagaacacccgtatccccgtcgctgcaggaccggccggcgtccaacagagacagaccccaactcggagagcaggctgtttctgctgaacctgaacatctacgtcccgcgcgacgagcggtttgggcatctcaagatgtcggacttcctcgggtactcactgaaggcgatcatcgaggctgtccttccgacgctggggacgttcgtcgacgatacgcccaaggagttcgattcgttcgaagacatccttgggctctacgagccgggtccagaggcgcccaacaacccactggtagcagaggtcaggaagagaatccccagcgagttcctcagaagcattctgcccaatggtagccatgaccaccccctgaagatgccccttccaaatatcatcagatcagatgtgttgaaaaaggctccagagtttaagtttggctggaggaccgacgaagagtttgcgagggagacgcttgcaggcgtgaacccagtgctcatcaaacgtctgacggagttcccagctaaaagtaccctggacccaagtcaatacggagaccatacgagcaagatcaccgaagctcacatccagcataacatggaaggcctgtcagtgcagaatgcactgaagaagaacaggctcttcatcctagaccaccatgaccatttcatgccgtacctcaacaagatcaacgagttggaggggaacttcatctacgccagcaggaccctactgttcctgaaggacgatggcacgctgaagcccctggccgtcgagctgagcctgccccaccctgatggccagcagcacggcgcggtcagcaaggtgtacaccccagctcactccggcgctgagggccacgtctggcaacttgccaaggcttatgcctgcgtgaacgactccgcctggcatcagctgatcagccactggctgaacacgcacgcggtgatcgagccgttcgtcatcgcaacgaaccggcagctgagcgtggtgcatccagtgcacaagctgctgagcccacactaccgtgacacgctgaacatcaacgccctggcacgccagacgctcatcaacgccgacggcatcttcgagcgcaccgtgttccctgcaaagtacgcgctggggatgtcctccgacgtgtacaagagctggaatttcaacgagcaggctctcccagcagacctcgtcaagagaggtgtggctgtgccggaccagtcgagcccctacggtgtccggttgctgatcaaggactacccttacgccgtggacgggctggtcatctggtgggcgatcgagcggtgggtcaaggagtacctggacgtctactaccccaacgacggcgagctccagcgcgacgtggagctgcaggcgtggtggaaggaggtgcgcgaggaggcgcacggcgacctcaaggaccgagactggtggcccaggatggacgccgtccagcggctggccagggcgtgcacgaccgtcatctgggtagcgtccgcgctgcacgcggccgtcaacttcgggcagtacccgtacgccgggtacctgccgaaccggccgaccgtgagccggcggccgatgccggagccgggcagcgacgactacaagaagctggaggcggggcagaaggaggcggacgcggtgttcatccgcaccatcaccagccagttccagaccatcctgggcatctcgctcatcgagatcctctccaagcactcctccgacgaggtgtacctcggccagcgcgacgagcctgagcgctggacgtcggacgccagggcgctggacgcgttcagaaggttcggaagccggctggtggagatcgagaagcggatcaggacgatgaacgacagcccgacgttgaagaaccggaaggggccggtggagatgccgtacatgctgctgtaccccaacacgtcggatgtcaccggcgagaagggcgaggggctcactgccatgggcattcccaacagcatctccatatga

SEQ ID NO: 45 - DNA, 5376 bp, Artificial Sequence
  WVP18-09307-014
atgctgagcgggatcatcgacgggctgacgggggcgaacaagcatgcgcggctcaagggcacggtggtgctcatgcgcaagaacgtgctggacctcaacgacttcggcgccaccgtcgtcgacagcatcagcgagttcctcggcaagggggtcacctgccagctcatcagctccactctcgtcgacgccaacaacggcaaccgcgggcgggtcggggcggaggcgaacctggagcagtggctgacgagcctgccgtcgctgacgaccggcgagtccaagttcggcgtcacgttcgactgggaggtggagaagctgggagtgccgggggccgtcgtcgtcaagaacaaccacgccgccgagttcttcctcaagacaatcaccctcgacgacgtgcccggccgcggcgccgtcaccttcgtcgccaactcctgggtctaccccgcgggcaagtaccgctacaaccgcgtcttcttctccaacgatacgtacctgccaagccagatgccggcggcgctgaagccgtaccgcgacgacgagctccgcaacctccgcggcgacgaccagcagggcccctaccaggagcacgaccgcgtgtaccgctacgacgtctacaacgacctcggcgagcccgacggcggcaacccgcgccccatcctcggcggctccgccgaccacccgtacccgcgccgctgccgcacgggccgcaagcccaccaaaaccgaccccaactcggagagccgactgtcgctggtggagcagatctacgtgccgcgggacgagcgcttcggccacctcaagatgtccgacttcctgggctactccatcaaggccatcacgcagggcatcatcccggcggtgcgcacgtacgtggacaccaccccgggcgagttcgactccttccaggacatcatcaacctgtacgagggcgggatcaagctgcccaagatccaggcgctcgaggacatgcgcaagctcttcccgctccagctcgtcaaggacctcctccccgccggcggggactacctgctcaagctccccatcccacagatcatccaaggcacgtcacgtataccgatcgatgtcaggggccggctgttgtctggtctgcatatatatatgtgctcctatgaggacaagaacgcgtggaggaccgacgaggagttcgcgcgggaggtgctcgccggcgtcaacccgatggtgatcacgcgcctcacggagttcccgcccaagagcacgctggaccccagcaagtacggcgaccacaccagcacgatcacggcggagcacatcgagaagaacctcgagggcctcacggtgcagcaggcgctggacggcaacaggctctacatcctggaccaccacgaccgcttcatgccgttcctcatcgacgtcaacaacctggagggcaacttcatctacgccaccaggacgctcttcttcctgcgcggcgacggcaggctcgcgcccctcgccatcgagctcagcgagccgtacatcgacggggacctcaccgtggccaagagcaaggtctacacgccggcgtccagcggcgtcgaggcctgggtgtggcagctcgccaaggcctatgtcgccgtcaacgactctggctggcaccaactcgtcagccactggctgaacacccacgcggtgatggagccgttcgtgatcgcgacgaaccggcagctgagcgtgacgcacccggtgcacaagctcctgagctcgcacttccgcgacaccatgaccatcaacgcgctggcgcggcagacgctcatcaacggcggcggcatcttcgagatgaccgtcttcccgggcaagtacgcgctgggcatgtcctccgtggtgtacaagagctggaacttcaccgagcagggcctccccgccgacctcgtcaagaggggcgtggcggtggcggacccgtccagcccgtacaaggtgcggctgctgatcgaggactacccgtacgcgagcgacgggctggccatctggcacgccatcgagcagtgggtgggcgagtacctggccatctactaccccgacgacggcgcgctgcggggcgacgaggagctgcaggcgtggtggaaggaggtgcgcgaggtcgggcacggcgaccacaaggacgcgccctggtggcccaagatgcaggccgtgtcggagctcgccagcgcctgcaccaccatcatctggatcgcgtcggcgctccacgccgccgtcaacttcggccagtacccgtacgcggggtacctcccgaacaggcccacggtgagccggcgccggatgccggagcccagcagcaaggagtacgaggagctggagcgcgacccggagcgcggcttcatccacaccatcacgagccagatccagaccatcatcggcatctcgctcatcgagatcctctccaagcactcctccgacgaggtgtacctcggccagcgcgacacccccgagtggacctccgacgcccgggcgctggcggcgttcaagaggttcagcgacgcgctggtcaagatcgagggcaaggtggtgggcgagaaccgcgacccgcagctgaggaacaggaacggccccgccgagttcccctacatgctgctctatcccaacacctctgaccacagcgaggcgagggagcgagcagcagggcaaggcatccacacccacacccaccggacactccctgagaagcgagaagcgagaagcgaagagcggccggccaccatgttctggcacggggtcgcggaccggctgacggggaagaacaaggaggcgtggaacgagggaaagatccgcggcacggtgaggctggtcaagaaggaggtgctggacgtcggcgacttcaacgcctcgctcctcgacggcgtacacaggatcctcggctgggacgacggcgtcgccttccagctcgtcagcgccaccgcggccgaccccagcaacgggagccgcggcaaggtcgggaaggcggcgcacctggaggaggcggtggtgtcgctcaagtcgacgacggacggggagaccgtgtaccgggtgagcttcgagtgggacgggtcgcagggcgtcccgggcgccgtcctggtcaggaacctgcagcacgccgagttcttcctcaagtcgctcaccctcgagggcgtccccggcaggggcaccgtcgtcttcgtcgccaactcgtggatctacccgcacaatctctactcccaggaacgcgtcttcttcgccaacgacacttatctgccaagcaaaatgcctgcggcattggtgccttaccggcaggacgagctcaagattctccgcggcgacgataatcctggaccatacaaggagcacgaccgcgtctaccgttacgactactacaacgacctcggtgagccagacaagggtgaagaccatgcccggcctgtcctcgggggcagccaagaacacccgtatccccgtcgctgcaggaccggccggcgtccaacagagacagaccccaactcggagagcaggctgtttctgctgaacctgaacatctacgtcccgcgcgacgagcggtttgggcatctcaagatgtcggacttcctcgggtactcactgaaggcgatcatcgaggctgtccttccgacgctggggacgttcgtcgacgatacgcccaaggagttcgattcgttcgaagacatccttgggctctacgagccgggtccagaggcgcccaacaacccactggtagcagaggtcaggaagagaatccccagcgagttcctcagaagcattctgcccaatggtagccatgaccaccccctgaagatgccccttccaaatatcatcagatcagatgtgttgaaaaaggctccagagtttaagtttggctggaggaccgacgaagagtttgcgagggagacgcttgcaggcgtgaacccagtgctcatcaaacgtctgacggagttcccagctaaaagtaccctggacccaagtcaatacggagaccatacgagcaagatcaccgaagctcacatccagcataacatggaaggcctgtcagtgcagaatgcactgaagaagaacaggctcttcatcctagaccaccatgaccatttcatgccgtacctcaacaagatcaacgagttggaggggaacttcatctacgccagcaggaccctactgttcctgaaggacgatggcacgctgaagcccctggccgtcgagctgagcctgccccaccctgatggccagcagcacggcgcggtcagcaaggtgtacaccccagctcactccggcgctgagggccacgtctggcaacttgccaaggcttatgcctgcgtgaacgactccgcctggcatcagctgatcagccactggctgaacacgcacgcggtgatcgagccgttcgtcatcgcaacgaaccggcagctgagcgtggtgcatccagtgcacaagctgctgagcccacactaccgtgacacgctgaacatcaacgccctggcacgccagacgctcatcaacgccgacggcatcttcgagcgcaccgtgttccctgcaaagtacgcgctggggatgtcctccgacgtgtacaagagctggaatttcaacgagcaggctctcccagcagacctcgtcaagagaggtgtggctgtgccggaccagtcgagcccctacggtgtccggttgctgatcaaggactacccttacgccgtggacgggctggtcatctggtgggcgatcgagcggtgggtcaaggagtacctggacgtctactaccccaacgacggcgagctccagcgcgacgtggagctgcaggcgtggtggaaggaggtgcgcgaggaggcgcacggcgacctcaaggaccgagactggtggcccaggatggacgccgtccagcggctggccagggcgtgcacgaccgtcatctgggtagcgtccgcgctgcacgcggccgtcaacttcgggcagtacccgtacgccgggtacctgccgaaccggccgaccgtgagccggcggccgatgccggagccgggcagcgacgactacaagaagctggaggcggggcagaaggaggcggacgcggtgttcatccgcaccatcaccagccagttccagaccatcctgggcatctcgctcatcgagatcctctccaagcactcctccgacgaggtgtacctcggccagcgcgacgagcctgagcgctggacgtcggacgccagggcgctggacgcgttcagaaggttcggaagccggctggtggagatcgagaagcggatcaggacgatgaacgacagcccgacgttgaagaaccggaaggggccggtggagatgccgtacatgctgctgtaccccaacacgtcggatgtcaccggcgagaagggcgaggggctcactgccatgggcattcccaacagcatctccatatga

SEQ ID NO: 46 - DNA, 24 bp, Artificial Sequence
  crRNA1
accgccgctttctcctcctcctcg

SEQ ID NO: 47 - DNA, 24 bp, Artificial Sequence
  crRNA2.1
aggagactcttgttaagcatttag

SEQ ID NO: 48 - DNA, 24 bp, Artificial Sequence
  crRNA2.2
aggagactctttttaagcatttgg

SEQ ID NO: 49 - DNA, 24 bp, Artificial Sequence
  GGAGTGTCGTATTTGAGGAGTCCT
ggagtgtcgtatttgaggagtcct

SEQ ID NO: 50 - DNA, 17090 bp, Artificial Sequence
  pZFNnptII-LbCpf1-tDT-lox3_TTTV
ggagacggtcacagcttgtctgtaagcggatgccgggagcagacaagcccgtcagggcgcgtcagcgggtgttggcgggtgtcggggcgcagccatgacccagtcacgtagcgatagcggagtgtatactggcttaactatgcggcatcagagcagattgtactgagagtgcaccatatgcggtgtgaaataccgcacagatgcgtaaggagaaaataccgcatcaggcgctcttccgcttcctcgctcactgactcgctgcgctcggtcgttcggctgcggcgagcggtatcagctcactcaaaggcggtaatcggttatccacagaatcaggggataacgcaggaaagaacatgtgagcaaaaggccagcaaaaggccaggaaccgtaaaaaggccgcgttgctggcgtttttccataggctccgcccccctgacgagcatcacaaaaatcgacgctcaagtcagaggtggcgaaacccgacaggactataaagataccaggcgtttccccctggaagctccctcgtgcgctctcctgttccgaccctgccgcttaccggatacctgtccgcctttctcccttcgggaagcgtggcgctttctcatagctcacgctgtaggtatctcagttcggtgtaggtcgttcgctccaagctgggctgtgtgcacgaaccccccgttcagcccgaccgctgcgccttatccggtaactatcgtcttgagtccaacccggtaagacacgacttatcgccactggcagcagccactggtaacaggattagcagagcgaggtatgtaggcggtgctacagagttcttgaagtggtggcctaactacggctacactagaagaacagtatttggtatctgcgctctgctgaagccagttaccttcggaaaaagagttggtagctcttgatccggcaaacaaaccaccgctggtagcggtggtttttttgtttgcaagcagcagattacgcgcagaaaaaaaggatctcaagaagatcctttgatcttttctacggggtctgacgctcagtggaacgaaaactcacgttaagggattttggtcatgagattatcaaaaaggatcttcacctagatccttttcggcgtccacatcaacggcgtcggcggcgactgcccaggcaagaccgagatgcaccgcgatatcttgctgcgttcggatattttcgtggagttcccgccacagacccggattgaaggcgagatccagcaactcgcgccagatcatcctgtgacggaactttggcgcgtgatgactggccaggacgtcggccgaaagagcgacaagcagatcacgcttttcgacagcgtcggatttgcgatcgaggatttttcggcgctgcgctacgtccgcgaccgcgttgagggatcaagccacagcagcccactcgaccttctagccgacccagacgagccaagggatctttttggaatgctgctccgtcgtcaggctttccgacgtttgggtggttgaacagaagtcattatcgcacggaatgccaagcactcccgaggggaaccctgtggttggcatgcacatacaaatggacgaacggataaaccttttcacgcccttttaaatatccgattattctaataaacgctcttttctcttaggtttacccgccaatatatcctgtcaaacactgatagtttaaaccgaaggcgggaaacgacaatctgatcgggtaccgggccccccctcgaggtcgacggtatcgataagcttgatcctagggagctcaagcctatactgtacttaacttgattgcataattacttgatcatagactcatagtaaacttgattacacagataagtgaagaaacaaaccaattcaagacataaccaaagagaggtgaaagactgttttatatgtctaacattgcaccttaatatcacactgttagttcctttcttacttaaattcaacccattaaagtaaaaacaacagataataataatttgagaatgaacaaaaggaccatatcatttattaactcttatccatccatttgcattttgatgtccgaaaacaaaaactgaaagaacacagtaaattacaagcagaacaaatgatagaagaaaacagcttttccaatgccataatactcaaacttagtaggattctggtgtgtgggcaatgaaactgatgcattgaacttgacgaacgttgtcgaaaccgatgatacggacgaaagctgggaggcctggagctcggcgcgcctcacttcttctttttggcctggccagctttcttagtagcagcaggcctcttgtgcttaacggaggtctgagcgtactcaagccactctttgttggagatggcgatcttcaccttgtcgagcttctcatcttccgctttcttaaactgcccgatagcccagagaacctttctcgcaatgttgtaagccccgtttgcatcagcattcttcggcaggatagcgttctcttgagcctcatagttacggctgtcgtagaagatcccgtcagagttcttgaccggagagataaggaagtccacatcggtccttccggtgatagagttcctcatctggagcatgagagacatgagggccatgaatgagctgtagaatgccttgtcgctctgctcgcacaaaagagccctgatatcaccctgctggtagttgatgccgtacttgttgaacagttctttgtaggcagaggtgaggcacacttcttcccagtcgaacacgttgtttttcttcggatttcggaagatcctgatacggttcccgtaggagtagagcttccacttcttaatgtagtcggcgtcggtcctgctgaagttcttatagtcgagagcgaactcgaaaagatcctcttccggcacgtacatgatcctgtcgaaagacgagatgaacttcttgctgtcggcgatcgaggtgtacttggtcttgagcaggttcacgaaaccagtagaaggatcgatcttgctggtgagccaagcagggatatagaagatgaagccgttctgggtgctcatgctcttgaaggactcgaacttgttcgtgatctggtatcccttaagagcaccaccggtagcgcaagggttgctctttttgtccaccatgtagttgagcttgtcgatgagcatcttctcgaacttttggtagacctgcttctcaaccttcactctactgttcttgaacccagagttgaggtcctcaagagcgatcacagcatcgtacttttccaccagctcgcagatcttatgcaccacctgagagatgtagccggccttcaactctttgatgttttcgatagaagtccagttctgcctggcctcgaaacgctctttttctttcttatcgaggagtgagtggtagtcggtcttgatcctgatgccgttgaaattgttgataatctcgttcaggctgtactgctcgacgatgtttccctttccgtccaccacaacgatgtagaggaggtttctctcaccacgatcgattccgatcacgtaagggttatcatcgtgcttgagcagcaccctcacctcggtattgatcttgaagatgttcttcgggcacttgttgatagcgatcgggatatgaagctcgtactggtcctcgctgaaccttttgtccttgtagacgtcgtaagacagcgtggtggtctttttcgggttgtcaggattcttgttagcgattggagagttggccgggtgaacaaccaactcttctttcttgagtgaggccctacgcatgaagagttcagcaccaccagaaagtctgatctgcccgtggttgttctcgtcgaaaagcagcttgaagtacatcgtatggaggttaggagttccgtggctcttgtcggagaagtccttgttatagatctggaacatgtagagcttgccctcttcgaccaacttgtcaacctctttcttggaggcgctctcgaagctaaccttgtaaccctgttcctcaacctcacggtagaacccggcgatatccttgtacttttctgtctcgctgaagttaaagtcgtaagcgttagaccacttcgggtaacgcgagatgctgtccttgaagaaatcgatgagcttgtggcagtcgttgaggttgaacatgtcgcctttcttgaaggtcccgttcttgtagattttctggatgtcctcagacgggttgtagtaggccatccatttcttgctgaagaacaccttaggaagcatcttgttcggtcccggaaggagcttgtagttgatcttctcatagttcccgttcacgtcatccttgtcgatcttttggaggcacttggcgtatttcttgtccatgatggccaggtagtacttagacccgtacctgaggatggtggccctgtaatctgtctctttgtctttgtcccatccgcccatgaactgcgggttctgaaagtacaacttgaacttgtccttgctgtaaggcttctgggtcacgtagtttctgatggcgtcgtagatatggtccaccttgaggaggatatcgtaagcgagcacgaaatccccgtagaaagactcgtccctattagtctctttgccctctccgaagaaggccttgatatagttctcgaaggacttcacgctgtcgagcaaatccttcatgatcgcgacgacagcgtcgttcttcttcagactcttctcgaggacgaaatcagcatcgaacaacttctcagaggacccgtacaccttgtagatctcgtcgaccttctggatgatgatctctttgagcttctcgaccacgctgagatcagcatcagcgtattcttgaagctgctcgaggctgaaagagccgatcttcttgaacgacttacgcctgtcatcctcgtacttctcagtgacgacagccttcttcttgaggtggatgtcatcgtactcagcattccacttgtccctgatcacgttccactcgccgaaaatatccttgctgatggtgctgatagcaggtccgttcttaacgaagatcccagcgctgctgtactcgtcgaagttcttgaaaagtttctccaacttcttgatggacgagaagatctcgctgttcttgttgagggtgttacggaaaacctcaagcacttcctcgtcagaggtgtaaccctcaccgtaaaatgagaggctctcacgatcagagagaacctgcttgtagagcggcttgaacttcgggagcttctgcttcgttttctggttgtacaggttgatgtactcgttgagtcccttaatcttctccccagactcggtcacgaatcctccgataatagcgttgtacacgtcgatgccctcttgggtgagaacgaagttgaagaactccccttcaaaaaagtcctcgacgtcgtagtcgctgttgaggatcttctctttgatttcttgcacctcgtgcttatcgaagatggcgtccaccttctcgaagatgtccatgttgctgatgtaacgcgtgaggttctcgttgatgcatctgaaagcgatagaggtgctcttggcctcttcgctgaacatgttttccctgttgtcgaagaatccggtgaaggcagtagtgaatccgttgaagctgttcacgagagcgatctcatccttatcgtccaggaactcaggcaggattgtctcgataatatccttcttgaagaggctcttgtatccctcgtttcccttgaaagccttggcgatctctttacggaggttgatctcgaggttctcaagctctttgttctctttctcggtcctggttttcttacggaagaggctgatgtagttgttgaggttcttgagcttgatgctgtggagcacatcgttgatgaagctgaggtagtacctgtcgaggagcttcttcacgcccttgtaatcttcagctctcttctcatcctcgacgaggagcctcttgttgtcgatattctcttgggtctttcccacagggatagccttgaacctgagggtcttagagaggctgtagcagttggtaaacttctcgagcttgctaaccttcctcttcttcttaggagccatggaggaagccattgtttggcgcgccgaattcgctgcacatacataacatatcaagatcagaacacacatatacacacacaaatacaatcaagtcaacaactccaaaaagtccagatctacatatatacatacgtaaataacaaaatcatgtaaataatcacaatcatgtaatccagatctatgcacatatatatatacacaattaataaaaaaaatgatataacagatctatatctatgtatgtaacaacacaatcagatgagagaagtgatgttttcagatctgtatacatacaaacacaaacagatgaacaattgatacgtagatccatatgtatacgtacaattagctacacgattaaatgaaaaaaatcaacgatttcggattggtacacacaaacgcaacaatatgaagaaattcatatctgattagatataaacataaccacgtgtagatacacagtcaaatcaacaaatttatagcttctaaacggatgagatgaacaagataaagatattcacataaggcatacataagataagcagattaacaaactagcaataatacatacctaattaaaacaaggaataacagagagagagagagagagagagatttaccttgaaaatgaagaggagaagagaggatttcttaaaattgggggtagagaaagaaagatgatgaattgtgagaaaggagagatagaagggggggttgtatatataggctgtagaagattatttttgtgtttgaggcggtgaaggaagaggggatctgactatgacacgtttgcggttacgtatttcgataggagtctttcaacgcttaacgccgttactctatatgaccgtttgggccgtaacggggccgtttgttaacgctgatgttgattcttttctttctttctttcttccttttttaaagaagcaattgtacaatcgttgctagctgtcaaacggataattcggatacggatatgcctatattcatatccgtaatttttgaattcgtaatcatgtcatagctgtttcctgtgtgaaattgttatccgctcacaattccacacaacatacgagccggaagcataaagtgtaaagcctggggtgcctaatgagtgagctaactcacattaattgcgttgcgctcactgcccgctttccagtcgggaaacctgtcgtgccagatcgaattcctgcagcccgggttcagaagaccagagggctattgagacttttcaacaaagggtaatatcgggaaacctcctcggattccattgcccagctatctgtcacttcatcgaaaggacagtagaaaaggaagatggcttctacaaatgccatcattgcgataaaggaaaggctatcgttcaagatgcctctaccgacagtggtcccaaagatggacccccacccacgaggaacatcgtggaaaaagaagacgttccaaccacgtcttcaaagcaagtggattgatgtgatacatggtggagcacgacactctcgtctactccaagaatatcaaagatacagtctcagaagaccagagggctattgagacttttcaacaaagggtaatatcgggaaacctcctcggattccattgcccagctatctgtcacttcatcgaaaggacagtagaaaaggaagatggcttctacaaatgccatcattgcgataaaggaaaggctatcgttcaagatgcctctaccgacagtggtcccaaagatggacccccacccacgaggaacatcgtggaaaaagaagacgttccaaccacgtcttcaaagcaagtggattgatgtgatatctccactgacgtaagggatgacgcacaatcccactatccttcgcaagacccttcctctatataaggaagttcatttcatttggagaggggttccatggtgagcaagggcgaggaggtcatcaaagagttcatgcgcttcaaggtgcgcatggagggctccatgaacggccacgagttcgagatcgagggcgagggcgagggccgcccctacgagggcacccagaccgccaagctgaaggtgaccaagggcggccccctgcccttcgcctgggacatcctgtccccccagttcatgtacggctccaaggcgtacgtgaagcaccccgccgacatccccgattacaagaagctgtccttccccgagggcttcaagtgggagcgcgtgatgaacttcgaggacggcggtctggtgaccgtgacccaggactcctccctgcaggacggcacgctgatctacaaggtgaagatgcgcggcaccaacttcccccccgacggccccgtaatgcagaagaagaccatgggctgggaggcctccaccgagcgcctgtacccccgcgacggcgtgctgaagggcgagatccaccaggccctgaagctgaaggacggcggccactacctggtggagttcaagaccatctacatggccaagaagcccgtgcaactgcccggctactactacgtggacaccaagctggacatcacctcccacaacgaggactacaccatcgtggaacagtacgagcgctccgagggccgccaccacctgttcctgtacggcatggacgagctgtacaagtctagaggtacctgataatttctactaagtgtagataccgccgctttctcctcctcctcgtaatttctactaagtgtagataggagactcttgttaagcatttagtaatttctactaagtgtagataggagactctttttaagcatttggtaatttctactaagtgtagatggagtgtcgtatttgaggagtccttaatttctactaagtgtagatcgaatttccccgatcgttcaaacatttggcaataaagtttcttaagattgaatcctgttgccggtcttgcgatgattatcatataatttctgttgaattacgttaagcatgtaataattaacatgtaatgcatgacgttatttatgagatgggtttttatgattagagtcccgcaattatacatttaatacgcgatagaaaacaaaatatagcgcgcaaactaggataaattatcgcgcgcggtgtcatctatgttactagatcgctcgagcggccgccatggccactagtgcggccgccatggcctctagagccgatcgtgaagtttctcatctaagcccccatttggacgtgaatgtagacacgtcgaaataaagatttccgaattagaataatttgtttattgctttcgcctataaatacgacggatcgtaatttgtcgttttatcaaaatgtactttcattttataataacgctgcggacatctacatttttgaattgaaaaaaaattggccataccccaccatcgacatgattggcacccaggtgttggaccgactcaaccagttctgggatatggccccacagtccggaatgacccccgccgatgacgcgggacaagccgttttacgtttggaactgacagaaccgcaacgttgaaggagccactcagccgcgggtttctggagtttaatgagctaagcacatacgtcagaaaccattattgcgcgttcaaaagtcgcctaaggtcactatcagctagcaaatatttcttgtcaaaaatgctccactgacgttccataaattcccctcggtatccaattagagtctcatattcactctcaatccatacaaaaacacatccaaaatcacagaaaatgggagcttggattgaacaagatggattgcacgcaggttctccggccgcttgggtggagaggctattcggctatgactgggcacaacagacaatcggctgctctgatgccgccgtgttccggctgtcagcgcaggggcgcccggttctttttgtcaagaccgacctgtccggtgccctgaatgaacttcaggacgaggcagcgcggctatcgtggctggccacgacgggcgttccttgcgcagctgtgctcgacgttgtcactgaagcgggaagggactggctgctattgggcgaagtgccggggcaggatctcctgtcatctcaccttgctcctgccgagaaagtatccatcatggctgatgcaatgcggcggctgcatacgcttgatccggctacctgcccattcgaccaccaagcgaaacatcgcatcgagcgagcacgtactcggatggaagccggtcttgtcgatcaggatgatctggacgaagagcatcaggggctcgcgccagccgaactgttcgccaggctcaaggcgcgcatgcccgacggcgaggatctcgtcgtgactcatggcgatgcctgcttgccgaatatcatggtggaaaatggccgcttttctggattcatcgactgtggccggctgggtgtggcggaccgctatcaggacatagcgttggctacccgtgatattgctgaagagcttggcggcgaatgggctgaccgcttcctcgtgctttacggtatcgccgctcccgattcgcagcgcatcgccttctatcgccttcttgacgagttcttctgacccgatgagctaagctagctatatcatcaatttatgtattacacataatatcgcactcagtctttcatctacggcaatgtaccagctgatataatcagttattgaaatatttctgaatttaaacttgcatcaataaatttatgtttttgcttggactataatacctgacttgttattttatcaataaatatttaaactatatttctttcaatccggaccataccccaccatcgacatgattggcacccaggtgttggaccgactcaaccagttctgggatatggccccacagataacatagagaaacccaacggataatataagcaaacacaaattacaatggttcactacccagcagaaaaattaccaacatttcaaatgttgtgccttctaaaagttaagactagaagaacatctatagagcagaattgaagcatagaaacgaatttccccgatcgttcaaacatttggcaataaagtttcttaagattgaatcctgttgccggtcttgcgatgattatcatataatttctgttgaattacgttaagcatgtaataattaacatgtaatgcatgacgttatttatgagatgggtttttatgattagagtcccgcaattatacatttaatacgcgatagaaaacaaaatatagcgcgcaaactaggataaattatcgcgcgcggtgtcatctatgttactagatcgctcgaactagagccgatcgtgaagtttctcatctaagcccccatttggacgtgaatgtagacacgtcgaaataaagatttccgaattagaataatttgtttattgctttcgcctataaatacgacggatcgtaatttgtcgttttatcaaaatgtactttcattttataataacgctgcggacatctacatttttgaattgaaaaaaaattggtaattactctttctttttctccatattgaccatcatactcattgctgatccatgtagatttcccggacatgaagccatttacaattgaatatatcctgccgccgctgccgctttgcacccggtggagcttgcatgttggtttctacgcagaactgagccggttaggcagataatttccattgagaactgagccatgtgcaccttccccccaacacggtgagcgacggggcaacggagtgatccacatgggacttttaaacatcatccgtcggatggcgttgcgagagaagcagtcgatccgtgagatcagccgacgcaccgggcaggcgcgcaacacgatcgcaaagtatttgaacgcaggtacaatcgagccgacgttcacgcggaacgaccaagcaagctatgttgcgattacttcgccaactattgcgataacaagaaaaagccagcctttcatgatatatctcccaatttgtgtagggcttattatgcacgcttaaaaataataaaagcagacttgacctgatagtttggctgtgagcaattatgtgcttagtgcatctaacgcttgagttaagccgcgccgcgaagcggcgtcggcttgaacgaattgttagacattatttgccgactaccttggtgatctcgcctttcacgtagtggacaaattcttccaactgatctgcgcgcgaggccaagcgatcttcttcttgtccaagataagcctgtctagcttcaagtatgacgggctgatactgggccggcaggcgctccattgcccagtcggcagcgacatccttcggcgcgattttgccggttactgcgctgtaccaaatgcgggacaacgtaagcactacatttcgctcatcgccagcccagtcgggcggcgagttccatagcgttaaggtttcatttagcgcctcaaatagatcctgttcaggaaccggatcaaagagttcctccgccgctggacctaccaaggcaacgctatgttctcttgcttttgtcagcaagatagccagatcaatgtcgatcgtggctggctcgaagatacctgcaagaatgtcattgcgctgccattctccaaattgcagttcgcgcttagctggataacgccacggaatgatgtcgtcgtgcacaacaatggtgacttctacagcgcggagaatctcgctctctccaggggaagccgaagtttccaaaaggtcgttgatcaaagctcgccgcgttgtttcatcaagccttacggtcaccgtaaccagcaaatcaatatcactgtgtggcttcaggccgccatccactgcggagccgtacaaatgtacggccagcaacgtcggttcgagatggcgctcgatgacgccaactacctctgatagttgagtcgatacttcggcgatcaccgcttccctcatgatgtttaactttgttttagggcgactgccctgctgcgtaacatcgttgctgctccataacatcaaacatcgacccacggcgtaacgcgcttgctgcttggatgcccgaggcatagactgtaccccaaaaaaacagtcataacaagccatgaaaaccgccactgcgccgttaccaccgctgcgttcggtcaaggttctggaccagttgcgtgagcgcatacgctacttgcattacagcttacgaaccgaacaggcttatgtccactgggttcgtgccttcatccgtttccacggtgtgcgtcacccggcaaccttgggcagcagcgaagtcgaggcatttctgtcctggctggcgaacgagcgcaaggtttcggtctccacgcatcgtcaggcatacccaccggtgccttgatgtgggcgccggcggtcgagtggcgacggcgcggcttgtccgcgccctggtagattgcctggccgtaggccagccatttttgagcggccagcggccgcgataggccgacgcgaagcggcggggcgtagggagcgcagcgaccgaagggtaggcgctttttgcagctcttcggctgtgcgctggccagacagttatgcacaggccaggcgggttttaagagttttaataagttttaaagagttttaggcggaaaaatcgccttttttctcttttatatcagtcacttacatgtgtgaccggttcccaatgtacggctttgggttcccaatgtacgggttccggttcccaatgtacggctttgggttcccaatgtacgtgctatccacaggaaagagaccttttcgacctttttcccctgctagggcaatttgccctagcatctgctccgtacattaggaaccggcggatgcttcgccctcgatcaggttgcggtagcgcatgactaggatcgggccagcctgccccgcctcctccttcaaatcgtactccggcaggtcatttgacccgatcagcttgcgcacggtgaaacagaacttcttgaactctccggcgctgccactgcgttcgtagatcgtcttgaacaaccatctggcttctgccttgcctgcggcgcggcgtgccaggcggtagagaaaacggccgatgccgggatcgatcaaaaagtaatcggggtgaaccgtcagcacgtccgggttcttgccttctgtgatctcgcggtacatccaatcagctagctcgatctcgatgtactccggccgcccggtttcgctctttacgatcttgtagcggctaatcaaggcttcaccctcggataccgtcaccaggcggccgttcttggccttcttcgtacgctgcatggcaacgtgcgtggtgtttaaccgaatgcaggtttctaccaggtcgtctttctgctttccgccatcggctcgccggcagaacttgagtacgtccgcaacgtgtggacggaacacgcggccgggcttgtctcccttcccttcccggtatcggttcatggattcggttagatgggaaaccgccatcagtaccaggtcgtaatcccacacactcgccatgccggccggccctgcggaaacctctacgtgcccgtctggaagctcgtagcggatcacctcgccagctcgtcggtcacgcttcgacagacggaaaacggccacgtccatgatgctgcgactatcgcgggtgcccacgtcatagagcatcggaacgaaaaaatctggttgctcgtcgcccttgggcggcttcctaatcgacggcgcaccggctgccggcggttgccgggattctttgcggattcgatcagcggccgcttgccacgattcaccggggcgtgcttctgcctcgatgcgttgccgctgggcggcctgcgccgccttcaacttctccaccaggtcatcacccagcgccgcgccgatttgtaccgggccggatggtttgcgaccgctcacgccgattcctcgggcttgggggttccagtgccattgcagggccggcagacaacccagccgcttacgcctggccaaccgcccgttcctccacacatggggcattccacggcgtcggtgcctggttgttcttgattttccatgccgcctcctttagccgctaaaattcatctactcatttattcatttgctcatttactctggtagctgcgcgatgtattcagatagcagctcggtaatggtcttgccttggcgtaccgcgtacatcttcagcttggtgtgatcctccgccggcaactgaaagttgacccgcttcatggctggcgtgtctgccaggctggccaacgttgcagccttgctgctgcgtgcgctcggacggccggcacttagcgtgtttgtgcttttgctcattttctctttacctcattaactcaaatgagttttgatttaatttcagcggccagcgcctggacctcgcgggcagcgtcgccctcgggttctgattcaagaacggttgtgccggcggcggcagtgcctgggtagctcacgcgctgcgtgatacgggactcaagaatgggcagctcgtacccggccagcgcctcggcaacctcaccgccgatgcgcgtgcctttgatcgcccgcgacacgacaaaggccgcttgtagccttccatccgtgacctcaatgcgctgcttaaccagctccaccaggtcggcggtggcccatatgtcgtaagggcttggctgcaccggaatcagcacgaagtcggctgccttgatcgcggacacagccaagtccgccgcctggggcgctccgtcgatcactacgaagtcgcgccggccgatggccttcacgtcgcggtcaatcgtcgggcggtcgatgccgacaacggttagcggttgatcttcccgcacggccgcccaatcgcgggcactgccctggggatcggaatcgactaacagaacatcggccccggcgagttgcagggcgcgggctagatgggttgcgatggtcgtcttgcctgacccgcctttctggttaagtacagcgataaccttcatgcgttccccttgcgtatttgtttatttactcatcgcatcatatacgcagcgaccgcatgacgcaagctgttttactcaaatacacatcacctttttagacggcggcgctcggtttcttcagcggccaagctcgccggccaggccgcgagcttggcatcagacaaaccggccaggatttcatgcagccgcacggttgagacgtgcgcgggcggctcgaacacgtacccggccgcgatcatctccgcctcgatctcttcggtaatgaaaaacggttcgtcctggccgtcctggtgcggtttcatgcttgttcctcttggcgttcattctcggcggccgccagggcgtcggcctcggtcaatgcgtcctcacggaaggcaccgcgccgcctggcctcggtgggcgtcacttcctcgctgcgctcaagtgcgcggtacagggtcgagcgatgcacgccaagcagtgcagccgcctctttcacggtgcggccttcctggtcgatcagctcgcgggcgtgcgcgatctgtgccggggtgagggtagggcgggggccaaacttcacgcctcgcgccttggcggcctcgcgcccgctccgggtgcggtcgatgattagggaacgctcgaactcggcaatgccggcgaacacggtcaacaccatgcggccggccggcgtggtggtgtcggcccacggctctgccaggctacgcaggcccgcgccggcctcctggatgcgctcggcaatgtccagtaggtcgcgggtgctgcgggccaggcggtctagcctggtcactgtcacaacgtcgccagggcgtaggtggtcaagcatcctggccagctccgggcggtcgcgcctggtgccggtgatcttctcggaaaacagcttggtgcagccggccgcgtgcagttcggcccgttggttggtcaagtcctggtcgtcggtgctgacgcgggcatagcccagcaggccagcggcggcgctcttgttcatggcgtaatgtctccggttctagtcgcaagtattctactttatgcgactaaaacacgcgacaagaaaacgccaggaaaagggcagggcggcagcctgtcgcgtaacttaggacttgtgcgacatgtcgttttcagaagacggctgcactgaacgtcagaagccgactgcactatagcagcggaggggttggatcgacctcgacgtacccctgcctcgcgcgtttcggtgatgacggtgaaaacctctgacacatgcagctccc

SEQ ID NO: 51 - DNA, 18 bp, Artificial Sequence
  cruaxxxxxxf02x
ggccagggcttccgtgat

SEQ ID NO: 52 - DNA, 21 bp, Artificial Sequence
  cruaxxxxxxr01x
ccgtcgttgtagaaccattgg

SEQ ID NO: 53 - DNA, 19 bp, Artificial Sequence
  nptIIxxxf01
gctgtgctcgacgttgtca

SEQ ID NO: 54 - DNA, 18 bp, Artificial Sequence
  nptIIxxxr01
cggcacttcgcccaatag

SEQ ID NO: 55 - DNA, 20 bp, Artificial Sequence
  tDTxxxf04
tcctcgttgtgggaggtgat

SEQ ID NO: 56 - DNA, 19 bp, Artificial Sequence
  tDTxxxr01
gtgcaactgcccggctact

SEQ ID NO: 57 - DNA, 29 bp, Artificial Sequence
  CruaxxxMGB
agtccttatgtgctccactttctggtgca

SEQ ID NO: 58 - DNA, 15 bp, Artificial Sequence
  nptIIxxxMGB
aagcgggaagggact

SEQ ID NO: 59 - DNA, 18 bp, Artificial Sequence
  tDTxxxMGB
agcttggtgtccacgtag

SEQ ID NO: 60 - DNA, 19 bp, Artificial Sequence
  LbCpf1- Fw
tgccggaagaggatctttt

SEQ ID NO: 61 - DNA, 23 bp, Artificial Sequence
  LbCpf1- Rv
agtcggcgtcggtcctgctgaag

SEQ ID NO: 62 - DNA, 18 bp, Artificial Sequence
  Probe for nuclease test
agttcgctctcgactata

SEQ ID NO: 63 - DNA, 24 bp, Artificial Sequence
  IR106_lox3_F1
cctctgacctccaaaagaccctta

SEQ ID NO: 64 - DNA, 22 bp, Artificial Sequence
  IR106_lox3_F2
ccattacttgtttggtcggcgt

SEQ ID NO: 65 - DNA, 21 bp, Artificial Sequence
  IR106_lox3_F3
gccatcacttgttttctcggc

SEQ ID NO: 66 - DNA, 20 bp, Artificial Sequence
  IR106_lox3_F4
ccgtcacttgttttctcggc

SEQ ID NO: 67 - DNA, 25 bp, Artificial Sequence
  IR106_lox3_R1
tcaaaggctaatataactgacacgt

SEQ ID NO: 68 - DNA, 23 bp, Artificial Sequence
  IR106_lox3_R2
ggcaaacgcgtttccttaattca

SEQ ID NO: 69 - DNA, 20 bp, Artificial Sequence
  IR106_lox3_R3
ataacgctgatgtgctaagc

SEQ ID NO: 70 - DNA, 24 bp, Artificial Sequence
  IR106_lox3_R4
gttaataacgctgatgtactaagc

SEQ ID NO: 71 - DNA, 22 bp, Artificial Sequence
  946R
gctctctcggcccccacttttt

SEQ ID NO: 72 - DNA, 20 bp, Artificial Sequence
  1145F
tgttctgcgcccaggctaca

SEQ ID NO: 73 - DNA, 20 bp, Artificial Sequence
  346F
tcgcgaacacaccggtcgta

SEQ ID NO: 74 - DNA, 20 bp, Artificial Sequence
  1948R
actcacatgcctcgccctca

SEQ ID NO: 75 - DNA, 5145 bp, Brassica napus
gtgaatccatatcggtcaaaaacagcggtacaaacacctctgaatataccattttcaataccactacttatgactatttttgtgtcaagtaattagctcttcaccggaacagaagtgtactataagctaggtaaatacaacgtattgttcattcagaataattgtgtgtactcttttatctcataacataagtattttctaatatttaaaagaaatacatttattcatgagaagtatatcatacgaattttctcaaaaaagtatatcataagaaagagacttaacatcacaaagactaattactttgaaaactagcatgttgacaaaaagaaagaagagtgaacataattaagaattcacattttgtaaaaggaaaaggaaaaaacatggctactgcgtagacggtagtccaatcaacaaaaaaacgtgtggacggcaatgagatccttctatctctatatatctctctcacttgccgattattagtaaccagaacgtacaccaactaataaactctcaacttcttcttgtttgccaacattatattacaaaacaactcaagattcattccatttaatactaactgattacatcatcgttatggccttagctaaagagttaatgggttatcctctgacctccaaaagacccttacttgtttggtcggcgtcgcatttcaagaagaggacacagccaacacaattctcgatcaagccttttgataggagaccaagaacgtccaaatccggggtcgttgcggccatcagtgaagatttggtcaaaacgctacgtttcaacacaaccaccggtgacagaaagagcgaggaggaggagaaagcggcggtgaaattcaaggtgagagctgtggttacggtgaggaacaagaacaaggaggattttaaggagactcttgttaagcatttagatgcttttggtgataagatcggtcgaaacgttgtcttggagcttgttagcaccgaacttgatccaagtaagtcgctttagtaaactcggttgaaaaacagaacatgataaaatatttttaaaaatggaaactttctatttgggcatttctaaaatcgtgtaatataaaatgggttatctcaaaatctctttatttgagatgggttttcgaatactaagataaatatcaaatcttttaactcgaacagaaacgaatatgccgaagaaaagcaatgcggcagttttaaaggactggtcaaagaagtcgaaaaccaaggcggagagggttcattacacggcggagttcacggtggacgcagcatttggctcaccgggagccatcaccgtcatgaataaacaccagaaagagttctttctggagagcatcaccatcgaaggtttcgcacttggccctgttcactttccatgcaactcttgggttcagtcccaaaaggatcacccagggaaacgaatctttttcactaataaggtaattaattttaaatatctgaatgatacagttatttacttaaatagttaaattactcatggtcccaagccattagctcacgtcattttcgatctcccgcaaaatcttattcaatattcatgtccggtgggtccatataataattatataccccttgtccaagttctaactatatgtaattaatgttgttacaaatgattaaacctaacgttatgtaaatttgtgtgcagccgcttttgccgagtgagacacctgatggattgaaaaaattgagggagagagagttgaagaatctaagaggagatgggagtggagcgaggaagttatcagacagaatctatgactttgatgtgtacaacgatcttggaaatcccgacaagtcatcagaactctctcggcccaagctcggcggcaaagagattccttaccctagacgatgtcgtaccggtcgccatccaactgataccggtacaattcataacaaaacattttatacatattttgagtacaatatgtaattaatgaatctctaatagtatgtgatttttatatgcattgttgacagataaagaagcggagagccgagtagagaagccattacctatgtacgtaccacgagatgagcaattcgaagagactaagcagaaaactttcgcagcagggaggctaaaagcggtcttacaccacctagttccctcgctgaaagccagcattttagctgaggactttgctgactttggcgagatagatggtctatataaagaaggattgctactcaagttagggtttcaagatgaaatctttgacaagttccctttgcccaaggccatcgttaatacactccaagaatcttctaaaggactcctcaaatacgacactcccaaaatactatcaagtaagcacacttaattaatatgatcctttgacatcaacttttgtttttcttatagaaaattgaacttctaccatttacaaccacatattattcaaagagtttttaatttattatatttgatctttgataactgagacccatcatgaatttttcatccccaccaaaagaaaacactttagttggaaagcaaacagaacccactaaaaagaatacagaaacgatcgacatatgattcacgttgttttcttaattcgttacaacgtgtcagttatattagcctttgaataaaaaagcccgtttgcctttatttaattcatcaccgtaacatggttagtagttagtacaagttattagttaattgattacaaaaaatttaaaataatgcagaggataaaaatgcatggctacgtgatgatgagtttgcacgtcaagccatagctggaatcaatccagtcaacattgagagggtaaggactttcccaccggtcagtaatcttgaccccgaaatctacggtccacaacactccgctctcacttccgaccacatcattggacatctcgacggactatccgtacaacaagtacgtataacaaatccacattgcttgatttagtatgtaactaaacgtaattatttattaactaagttttattttacatattattttccaggcgttggaagagaacagattgtatatgttgaattaccacgacatatttttaccgttcctagaccgaatcaatgcgctagacggacgcaaagcttatgctactcgaaccatattctttttgactcgtcttggtacacttaagcccgtagccattgagctaagtctccctccacatggccccaaccaccggtccaaacgcgtggttacacctcccgtcgatgcaacctctaattgggtgtggcagctcgctaaagcccacgttagctctaacgacgctggggtccaccagcttgtcaatcactggttagtacttaaaaacattcaagttattaaacatatacgtttcatgtagtgactctagagttattgatccttttgttggtgtgcaggttacgaacccatgcgtgcttggaaccgtttatattagctgcacatagacaactgagcgctatgcatccgatattcaagctattagacccgcacatgaggtacacgttggaaatcaatgcattggctagacaatcgttgatcagtgcagacggtgtgattgaagaaggcttcactgccggctcatacggcatggaaatgagcgccgccgcatacaagagcagctggcggttcgacatggaaggcctccctgccgatctcattcgcaggtactttagctagacaaaataatactcttagattatttcaaacacaacattaaacattttcattgtatattatatagtatttgattattttaaactgtgttttgttttttcagaggaatagcagttcctgacccgacacaaccacatggagttaaactcctaatcgaagactatccatacgccaacgacggtcttctactctggtcggctatccaaacctgggtccgaacctacgtggaacgctactacccaaacccgaacctaatcaaaacagactcggagctccaatcctggtactccgaatcaatcaacgtcggccacgccgatctccgcgacgccgagtggtggccagagctaaacaccgtcgacgatctcgtctccatcctcaccacactgatctggctcgcctcagctcagcacgcggctctcaacttcggacagtacccgtacggcggctacgtcccgaaccgtcctccgctgatgcggcggttgatccccgacgagtcggatccgttgtacgcgagtttcatctccgatccggagaagttttacttctcggcgatgccgagtttgttgcagacgtcgaagtttatggcggtggttgatactctgtcaacgcattcgccagatgaggagtatatcggggagagacagcagccgtcgatttggacgggagatggggagatcgttgatgcgttttatggattcgcggcggagatcggacggatagagaaggagattgagaaaaggaactctgatcctgaccgtagaaataggtgcggggctggtgttttgccgtatgagctgttggttccgagttccgagcctggtgttacgtgcagaggtgtacctaatagtgtgtcgatatagaaggaaattaaatatagggaaacatgtagaaattgctataaataatttttggaagaaattaaaatatattaaatttatagttacattacttcatcgtaaatttgtattttatagatgttttttttccgaagatagcttgaaatttatgtaactcgaatatttttaaaagtacttggacgatgcttcttggattctgacctaacttgagtcgcaggctatcttcgcacacgtataaacctagcaattttaagttgctgagaggaagatggatagatttgtacctttttaatatggcaagtcaaagagccatgacaaagtttattcgtgggattttattcacctaacctggatggttggatcataggagatcatttcattggtaggaacacaggaacttaagttggaatgaaggattcaaagaggcagagtcatcaacttagatttatcagaccagagccaacgacctgaccgatcgagttgcgcttagaagctgacgtagagaggaccgcaaagacaagataaataggagacatgcattcttttgaaaagctgtaataataagatcaacttaaaaaatctaactatttgcctataagacca

SEQ ID NO: 76 - DNA, 5366 bp, Brassica napus
gtacaaaaacttgaatataccactttcgttactacttattgttactatttgtgattaacaatgtgtacctgaacactacgtgattatcagtcaaacgatctgtcctgtaaataatactattactatacgctacgtaaatacagcgtattgttccctgtcacgctaatacatggtaatatcttttatctcatgtcgcataacatacgttttctaacatttaaaagagagacatttattatgatatcattaaaaatgtaaacatcgcaacaatatgagtagtcaattaatcactttgaaaactatattgttgacaaaaaaaatctagcttaagtgatatgttttgagagttcacattttcagaaaaataataaaactaaaacatgactttgcgtagacaatagtccaatgaaccaaaaaacgtgtggacggcaaagagttccttctctatatatacatctctttcacttgccgattattagtaagcagaacgtacaaacaactaataaactctcaacaatttcttcttcttcgccaacactatacaacaaaacagctcaagattcaatattcaattcaatactaattgattacaccatcgtgatggccttagttaaagagataatgggtcatcctctgatatcaggaaggccatcacttgttttctcggcttctcatttcaagaagaagacacagacaacgcaattctcgatcaagcctttcgatcggagaccaaaaacgtccaaatccggcgtcgtttcggccattagtgaagatttagtaaaaacgctgcgttttagcacaacaaccggagacagaaagagcgaggaggaggagaaagcggcggtgaaattcaaagtgagagctgtggttacagtgaggaacaagaacaaggaggattttaaggagactctttttaagcatttggatgcttttggtgacaagatcggtcggaacatcgtcttggagcttattagcaccgaacttgatccaagtaagtcactttcttctttgcttttatcacaaaacagagcactcaggaaaactttctaaaaatagaaacttttaaaaatcgtgtattaaaaatggatcatctcaaatatccaatctttgattcaaacagaaacgaatttgccgaagaaaagcaatgctgcggtgttaaaggattggtcagagaaatcgaaaaccaaggcggagagggttcattacacggcggagttcacggtggacgcagcgtttggcacgccgggagccatcaccatcatgaataaacaccagaaagagttttttctagagtgcataaccatcgaaggtttcgcacttggccctgttcactttccatgcaactcttgggttcagtcccaaaatgatcaccctgagaaacgaatcttcttcactaatcaggtaactgattaaaatatctgactgatacataattaattacggtcccagaccatttaagtcacgtcattttcgatctccaacgaattaatcacatatactaatcagtttcaaaatcttctccaatattcatgtctggtgggtccatataataatacttattagccagctttcaactatattcccataaataatatgttgtggttataaattattaaagatcaagttatgttaatttgtgtgcagccgtttttgccgagtgagacacctgaaggattaagaaaattaagggggaaagagttgaagaatctacgaggagatgggactggagtcaggaagttatcagacagaatctatgactttgatgtctacaacgatcttggaaatcccgacaagtcatctgaactctctcgtccgaaactcggtggcagagagaggccttaccctagacggtgtcgcactggtcgccagccaactgataccggtacaattcataacaacattcttaaaaacaatatctctaatagtatatgtgttttgggtgttatgaaatcaagcggatcatgaaattttgagacgataaacaagtcagtaattaacgattttttttaaaaaaaattaaaaaattggagagatacatttttataaattgactctaatttttttgaagttctacagccaatgtttcatttggtcatgtccaattgtccatgactggtactgtgaaaaaaatgtatctgatgttttatctgcattgttggcagataatgaagcggagagccgagtggaaaagccattacctatgtacgtgccacgagacgagcaatttgaagagactaagcaggacactttcgccgcagggaggttaaaagcggtgttacaccaccttgttccgtcgcttaaagctagtattttagctgatgacttttctgacttcggagagattgatgatctctacaaaaaaggcttgctactgaagttaggatttcaagatgagatattcaacaagttccctttgcctaagggcatcgttaataccctccaagaatcttcgaaaggactcctcaaatacgacactcccaaaatattatcgagtaagctcacttaattcataaaaaattttaacatcaaattttgattttaataaaaagggtgttttaatagaaaatgaactttgattttgtggcgattgttggtctttgataattgggaccattatgaagtgttatcgtcctaccaaaaagtaagaaataatcattttagttgaaaagcaggaataaaagagtgcataagcaaacatatgcatgtttcacgtgcttttcttgactcgttataacgctcgtgctagttatagtagtattagtttgtgaataaacaaaagcgcgtttgcctttcattaattcaaaatcataacatgcttagcacatcagcgttattaactaattgactttttttttaaaatgaatgcagaggataaaaacgcatggctacgagatgacgagttcgcacgtcaagccatagctggaatcaatccagtcaacattgagagagtcaagactttcccacccgtcagtaatcttgaccccgaaatctacggtccacaacactccgctctcacttccgaccacatcatcggacatcttgacggcttgtccgttcaacaagtacgttttatactataaacaaatccaaattactcgaataattactaaaagtgaaatttgatcaactaatttttgtttaattatttttcaggcgttggaagagaacagattgtatatgttggattaccatgacatattcttaccgttcctagaccaaatcaatgcgctcgatggacgcaaagcatatgctactcgaaccattttcttcttgactcgtcttggaacacttaagcccgtagccatcgagctaagcctcccttcccatggcccgaaccaccgatccaaacgagttgttacacctcctgtcgatgcaacctctaactgggtgtggcagctcgctaaagcacatgttagctccaacgatgctggagtccaccaacttgttaaccactggttagtactcaaaacgttaacttactaatcatttatgtaacaagttgttaataatgaatatagagttattgatatatttatcaatttttgttctaaaggttacgaacccatgcatgcttggaaccgtttataatagctgcacataggcaattaagcgctatgcatccgatattcaaactattggatccacacatgaggtatacgttggagatcaatgcactggctagacaatcattgatcagtgcagacggtgtgattgaaggaggcttcactgctggccaatacggtttggaaatgagctccgcagcctacaaaagtagttggcggttcgacatggaaggcctccctgccgatctcattcgcaggtattgtagctaaactttgttagacatatactattcttgattatgtcaaacacaattttatacgtatgatatctaatattgatcgttttattttgttttttagaggaatggcagttccagacccaacacaaccacatggacttaaactcctgatcgaagactatccatatgcgaacgacggtcttctaatatggtccgcaatccaaacatgggtccgaacttacgtggaacgttactatccaaactcgaactcaattcaaacagactcggaactccaatcgtggtactcggagtcaatcaacgtaggccatgcagatctccgcgaagccgagtggtggccaaagttagacaccgtggacgacctagtctccatcctcaccacactagtctggctcgcctccgctcaacacgccgctctcaacttcggacagtatccgtatggaggttacgtcccaaaccgacctccgctgatgcgacggttaatccctgacgagtcggatccggagtacgcaagttttatctcggatcctgagaaattttatttttcttcgatgccgagtttgttgcaaacgtcgaagtttatggcggtggttgatacgttgtcaacgcattctccggatgaggagtatatcggggagagacaacaaccgtccacttggaccggagatgcggagattgttgatgcgttttatggatttgcggcggagattggacggatagaaaaagagattgagaaaagaaacagtgatcctaaccgtagaaacaggtgtggagctggagttttgccttacgagttgttggttccgagttctgagccaggtgttacgtgcagaggtgtacctaatagtgtatcgatatagaatgagattaaatataggagaaaatgtagaaatctgttatatatgatttttgaaaatgaaataaaatatataaattggtacatttgaattttgcagatatgttctcgaagctagatttaaattcatattcataatattttgaaatatattcagacaatggatttgttcatctccggttaattatggcccaaaagaccataaaatttatgaaatttgaaaatttaaaataccatatgcttattgttgcgacgatggattatgatttgggctcattttatagataacttcaaagtgactccctttcgaattggatcatggagatctcgattgctcaacttaaatttttcaaaagaaaacttcaaagtggctctgtttcaactttaaattggacctaaaaccaaggcttcttgggttctgacctaacttgggtcacacactatctcctcagacgtataaaatatatatttgtaccttttcatcagggaaattaaggcagatcgagatatacactaaagagtcaagacaaggtttgttcttatggttttaacctaatctgacatacatacgaaccttaagttgggtagaaaaatcgaacgtacaaaaagctatttgtgtctggttgattctgatccaatgatgcagagtaatcaacttaattagatttatcagacaaaaagccaacaacc

SEQ ID NO: 77 - DNA, 5154 bp, Brassica napus
aaatttgaattaacatgttgtaaattggagaagtggtgaatccatatcggttaaaaacagcggtacaaaaggtatttacctattttgtgtcaagtaattagctcttcaccggaacagaagtgtactataagctaggtaaatacaacgtattgttcattcagaataatagtgtgtactctcttatctcataacgtaactattttctaacatttaaaagaaatacatttattcatgagaagtatatcataagaattttctcaaaagtgtatatcatagaaagagacttaacatcacaaagactaattactttgaaaactagcatgttgacaaaaagaaagaagagtgaacatgagaattcacattttgtaaaaggaaaaaataaaagcatggctattgcgtagacggtagttcaattaacaaaaaaacgtgtggacggcaatgagatccttctatctctatatatctctctcacttgccgattattagtaaccagaacgtacaccaactaataaactctcagcttcttcttgtttgccaacactaatctacaaaaaaactcaagattcattccatttaatactaactgattacatcatcgtgatggccttagctaaagagttaatgggttatccactgacctccaaaaggccattacttgtttggtcggcgtcgcatttcaagaagaggacacagccaacacaattatcgatcaagccttttgatcggagaccaagaacgtccaaatccggggtcgttgcggccatcagtgaagatttggtcaaaacgctacgtttcaacacaaccaccggtgacagaaagagcgaggaggaggagaaagcggcggtgaaattcaaggtgagagctgtggttacggtgaggaacaagaacaaggaggattttaaggagactcttgttaagcatttagatgcttttggtgataagatcggtcgaaacattgtcttggagcttgttagcaccgaacttgatccaagtaagtcgctttagtaactcggttgaaaaacagaacatgataaaatatttctaaaaatggaaactttatatttgggcatttctataatcgtgtaatataaaatgggttatctcaaaatctcttgatctgagatgggttttcgaatactaagataaatattaaatcttttaactcgaacagaaacgaatatgccgaagaaaagcaatgcggcagttttaaaggactggtcaaagaagtcgaaaaccaaggcggaaagggttcattacacggcggagttcacggtggacgcagcatttggctcaccgggagccatcaccgtcatgaataaacaccagaaagaattctttctagagagcatcaccatcgaaggtttcgcagttggtcctgttcactttccatgcaattcttgggttcagtcccaaaaggatcacccagagaaacgaatctttttcactaatcaggtaattaatttaaaatatctgagtgatacagttatttacttaaatagttcatttactcatggtcccaagccattaactcacgtcattttcgatttcccgcaaaatcttattcaatattcatgtccggtgggtccatataataattatataccccttgtccaagttctaactatatgtaattatgttgttacaaatgattaaaccttacgttatataaatttatgtgcagccgtttttgccgagtgggacacctgatggattgaaaaaattgagggagagagagttgaagaatctaagaggagatgggagtggagtgaggaagttatcagacagaatctatgactttgatgtgtacaacgatcttggaaatcccgacaagtcatcagaactctctcgccccaagcttggcggcaaagagattccttaccctagacgatgtcgtaccggtcgccatccaactgataccggtacaattcataaaaaaacattttatacatattttgagtacaatatgtaattaatgaatctctaatagtatgtgatttttatatgcattgttgacagataaagaagcggagagccgagtggagaagccattacctatgtacgtaccacgagatgagcaatttgaagagactaagcagaaaactttcgctgcagggaggttaaaagcggtcttacaccacctagttccgtctctcaaagccagcattttagctgaggactttgctgactttggcgagatagatggtctctataaagaaggattgctactcaagttagggtttcaagatgaaatttttaacaagttccctttgcccaaggccatcgttaatacactccaagaatcttctaaaggactcctcaaatacgacactcccaaaatattatcgagtaagcataattaacttataagatcctttaacatcaacttttgttttttttaatagaaaattgaacttctaccatttacagccacatattatttccaagagttttatctgattttattagctcctatatttgatctttgataactgagacccatcatgaaattttcatcccaccaaaaagaaaacaacatcactttagttgaaaagcaaaaaggacccactaaaagaatacagaaaccacatatgattcacgtggttttcttaattcgttacaacgtgtcaattatactattagcttttgaattaaggaaacgcgtttgcctttaacatggtttagtacatgcaagttattaattagttaattaatttcaaaaaattaaaattatgcagaggataaaaatgcatggctacgagatgacgagtttgcacgtcaagccatagctggaatcaatccagtcaacattgagagggtcaggactttcccacccgtcagtaatcttgaccccgaaatctacggtccacaacactccgctctcacttccgaccacatcattggacatctcgacggactatccgtacaacaagtacgtttatattacaacaaatccacattgcttgattaagtacgtaactaaatgtgaatactgattaactaaatgttattttacttgttgtttttttcaggcgttggaagagaacaggttgtataagttggattaccatgacatattcttaccgttcctagaccggatcaatgcactagacggacgcaaagcttatgctactcgaaccatattcttcttgactcgtctaggaacacttaaacccgtagccattgagctaagcctccctccccatggtcccaaccatcggtccaaacgcgtggttacacctcctgtcgacgcaacctctaattgggtgtggcagctcgctaaagcccacgttagctctaacgacgctggtgtccaccagcttgtcaatcactggttagtacttaaaaatattaaagttattaaacatctatgtttcaaatagtgactctagagttattgatcttttgttggtgtgcaggttacgaacccatgcgtgcttggaaccgtttatattagctgcacatagacaaatgagcgctatgcatccgatattcaagctattggatccgcacatgaggtacacgttggaaatcaatgcattggctagacaatcgttgatcagtgcagacggtgtgattgaagaaggcttcactgccggctcatacggcatggagatgagcgccgccgcatacaagagcagttggcggtttgacatggaaggcctccctgctgatctcattcggaggtaatttaattagacaaagatactagtctttattatttcaaacacaacattatacattttcattgaatattatatagtatttgattattttaaactgtgttttattcttttcagaggaatggcagttcctgactcgacacaaccacatggacttaaactcctaatcgaagactatccatacgctaacgacggtcttctactctggtcggctatccaaacctgggtccgaacctacgtggaacgctactatcccaacccgaacctaatcaaaacagactcggagctccagtcctggtactccgaatcaatcaacgtcggccacgctgatctccgcgacgccgagtggtggccaaagctaaacaccgtcgacgacctcgcctccatcctcaccacactaatctggctcgcctcagctcaacacgcggctctcaacttcggacagtacccgtacggcggctacgtccccaaccgtcctccgctgatgcggcggttgatccccgacgagtctgatccggagtacgcgagtttcatctccgatccggagaagttttacttctcggcgatgccgagtttgctgcagacgtcgaagtttatggcggtggttgatactctgtcaacgcattcgccggatgaggagtatatcggggagagacagcaaccgtcgatttggacgggagatgcggagatcgttgatgcgttttatggattcgcggcggagatcggacggatagagaaggagattgaggaaaggaactctgatcctgaccgtagaaataggtgcggggctggtgttttgccttatgagctgttggttccgagttccgagcctggtgttacttgcagaggtgtacctaatagtgtatcgatatagaaggaaatttaatatagggaaaatgtagaaattgctataaataatttttggaaaaaattaaaatatattaaattatagttacatcatcgtaaatttgtaatttatagatgttttttttacgaagatagcttcaaatttatgtaactcgaatatttttaaaagtacttggacgatgcttcttggattttgacctaacttgactcgcaggctatcttcgcacacgtataaacctagcaattttaagttgctgtgagaggaagatgtatagattcgtacctttttaatatggcaaatcaaggcactcaagagccatgacagtttattcgtgggattttattaacctatcatttcattggtaggaacacatgaaccttaagttggcacgaaagattcaacggcgcagagttatcaacttagttttatcagaccagagccaacgacctgaccgatcgagttgcgttcagaagctgacgtagagaggaccacacaaagagacgataaatagaagacatgcattcttttgaaaagctgtaataataagatcaacttagaaaatctaatcaatttgcctataagactaaattatatgagaatatatac

SEQ ID NO: 78 - DNA, 5330 bp, Brassica napus
cgtacaaaaactttaatataccactttcgttactactaattgttactattcgtggttaacaatgtgtacctgaacactacgtggttatcagtcaaacgatccgtcctgtaaataatactgccactatacgctacgtaaatacaacgtattgttccttgtcacgctgatacatggtaatatcttttatctcatgtcataacatacgttttctaacatttaaaagagagacatttattatgatatcattaaaaatgtaaacatcgcaacaatacgagtagtcaaactaatcactttgaaaactatattgttgacaaaaaaaaaatctagcttaagtgaatatgttttgagagttcacattttcagaaaaataataaaactaaaacatgactttgcgtagacaatagtccaatgaaccaaaaaacgtgtggacggcaaagagttccttctctatatatacatctctttcacttgccgattattagtaagcagaacgtacaaacaactaataaactctcaacaacttcttcttcttcgccaacactatacaacaaaacagctcaaggttcattcaattcgatactaattgattacaccatcgtgatggccttagttaaagagataatgggtcatcctctgatatcaggaaggccgtcacttgttttctcggcttctcatttcaagaagaagacacagacaacgcaattctcgatcaagccttttgatcggagaccaaacacgtccaaatccggcgtcgtttccgccattagtgaagatttagtaaaaacgctgcgttttagcacaacaaccggagacagaaagagcgaggaggaggagaaagcggcggtgaaattcaaagtgagagctgttgttacagtgaggaacaagaacaaggaggattttaaggagactctttttaagcatttggatgcttttggtgacaagatcggtcggaacatcgtcttggagcttattagcaccgaacttgatccaagtaagtcacttacttttttatttttttataactcggttacagaacagagcactcaggaaaactttctaaaaatagaaaaatttaaaaatcgtgtaattaaaaatggatcatctcaaatatccaatctttgctccaaacagaaacgaatttgccgaagaagagcaatgcagcggtgttaaaggattggtcagagaaatcgaaaaccaaggcggagagggttcattacacggcggagttcacagtcgacgcagcgtttggcacgccgggagccatcaccatcatgaataaacaccagaaagagttttttctagagtgcataaccatcgaaggtttcgcacttggccctgttcactttccatgcaactcttgggttcagtcccaaaatgatcaccctgagaaacgaatcttcttcactaatcaggtaattgattaaaatatctgactgatacataattaattacggtcccagacaatttaagtcacgtcattttcgatctccaacgaattaattacatatactaatcagtttcaaaatcttctacaatattcatgtctggtgggtccatataataatacttattagccagctttcaactatattcccataaataatatgtggttataaattattaaaaatcaagttatgttaatttgtgtgcagccgtttttgccgagtgagacacctgaaggattaagaaaactaagggggaaagagttgaagaatctaagaggagatgggactggagtcaggaagttatcagacagaatctatgactttgatgtctacaacgatcttggaaatcccgacaagtcatatgaactctctcgtccgaagctcggtggcagagagaggccttaccctagacggtgtcgcactggtcgccagccaactgataccggtacaattcataacaacattcttaaaaacaatatctctaatagtatatgtttttgggtgttatgaaatcaagcggatcctgaaattttgagacgataaacaagtcagtaaggatttttatttttttaaaattaaaaaatcggagagattcatttttataaattgactccaatttttttgaagttttagaaccaatgtttcatttggtttgcatgtccatgattggttttgtgaaaatatgtatctgatgttttatctgcatcgttggcagataatgaagcggagagccgagtggaaaagccattacctatgtacgtgccacgagacgagcaatttgaagagactaagcaggatactttcgccgcagggaggttaaaagcggtgttacaccaccttgttccgtcgcttaaagctagtattttagctgatgacttttctgactttggagagattgatgatctctacaaagaaggcttgctactcaagttagggtttcaagatgagatctttaacaagttccctttgcctaagggcatcgttaataccctccaagaatcttcgaaaggactcctcaaatacgacactccgaaaatattatcgagtaagctcacttaattcataaaattctttaacatcaaattttgattttaataaaaaggttgtttttaatagaaaatgaactttaatattttgtggcgattgttggtctttgataattgggaccattatgaagtgttatcgtcctaccaaaaagtaagaaataatcattttagttgaaaaggaggaataaaaaagagtacgtacataagcaaacatatgtttcacgtgcttttcttaactcgttataacgctcgtgctagtaatagtattagtttgtgaataaacaaaagcgcgtttgcctttcattaattcaaaatcataaaacatgcttagtacatcagcgttattaactaattgacttttttgtaaaatgaacgcagaggataaaaacgcatggctacgagatgacgagttcgcacgtcaagccatagctggaatcaatccagtcaacattgagagagtcaagactttcccacccgtcagtaatcttgaccccgaaatctacggtccacaacactccgctctcacttccgaccacatcatcggacatcttgacggcttgtccgttcaacaagtacgttttatactataaacaaatccaaattaagccctttctcaaaaaaaaaaaaaaaaaacaaatccaaattactcgaataattactaaatgtgaaatttgatcaactaattttttattcttcaggcgctggaagagaacagattgtttatgttggattaccacgacatattcttaccgttcctggaccggatcaatgcgctcgacggacgcaaagcatatgctactcgaaccatattcttcttgactcgtctcggaacacttaagcccgtagccatcgagctgagcctcccttcccatggcccgaaccaccgatccaaacgagttgttacacctcctgtcgatgcaacctctaactgggtgtggcagctcgctaaagcacatgttagctctaacgatgctggagtccaccaacttgtcaaccactggttagtactcaaaacacattgagttattaaacatttatttaacaagttgttaataataaatataggactgacatgtttttatccttcttttgatgttgtaaaggttacgaacacatgcatgcttggaaccgtttataatagctgcacataggcaattaagcgctatgcatccgatatttaaactattggatccacacatgaggtacacgttggagatcaatgcactggctagacaatcattgatcagtgcagacggtgtgattgaaggaggtttcactgctggccaatacggtttggaaatgagctccgcagcatacaaaagtagttggcggttcgatatggaaggcctccctgccgatctcattcgcaggtattgtataaacttttttagacatatactagtcttgattatgtcagacacaaatatacgtttttattgtatgatatctaatatcgatcgttttattttgtttttttttcagaggaatggcagttccagacccaacacaaccacatggacttaaactcctgatcgaagactatccatatgcgaacgacggtcttttaatatggtccgcaatccaaacatgggtccgaacttacgtggaacgttactatccaaactcgaactcaatccagacagactcggaactccaatcatggtactccgagtcaatcaacgtaggccatgcagatctacgcgaagccgagtggtggccaaagttagacaccgtggacgacctagtctccatcctcaccacactagtctggctcgcctccgctcaacacgccgctctcaacttcggacagtatccgtatggaggttacgtcccaaaccgacctccgctgatgcgacggttaatccctgacgagtcggatccggagtacgcaagttttatctcggatccagagaaattttatttttcgtccatgccgagtttgttgcaaacgtcgaagtttatggcggtggttgatactttgtcaacgcattcgcctgatgaggagtatataggggagagacaacaaccgtccacttggaccggagatgcggagattgttgatgcgttttatggatttgcggcggagattggacggattgaaaaagagattgagaaaagaaacagtgatcctagccgtagaaacaggtgtggagctggagttttgccttacgagttgttggttcctagttctgagccaggtgttacgtgcagaggtgtacctaatagtgtatcgatatagaatgagattaaatataggagaaaacgtagaaatctgttattatatgatttttgaaaatgaaataaaatatataattggtacatttgaattttgcagatatgttttcgaagctagatttaaattcatgttcataatattttgaaatatattcagacaatggatttgtgcatgtcaggttaattatagccaaagaagaccataaaatatatgaaaactgaaaattaaaaataccatatgcttatcgttgcgacgatggatcatgatttgggctcattttatagataacttcaaagtgactcctccctttcaaattggatcatggagatctcgattgctcaacttaaatttttcaaaaaaaactacttcaaagtggctctgtttcaactttaagttggacctgaaatttggcatggcttcttgggttctaacctaacttgggtcacaaactatctcctcatacgtataaaaaatatatttgtaccttttcatcagggaaattaaggcagatcgagatatacactaaagggccaagacaaggtttgttcttatggttttaacctaatctgatatcaggagaacatttcattggtatacatacga

SEQ ID NO: 79 - protein, 919 aa, Brassica napus
MALAKELMGYPLTSKRPLLVWSASHFKKRTQPTQFSIKPFDRRPRTSKSGVVAAISEDLVKTLRFNTTTGDRKSEEEEKAAVKFKVRAVVTVRNKNKEDFKETLVKHLDAFGDKIGRNVVLELVSTELDPKTNMPKKSNAAVLKDWSKKSKTKAERVHYTAEFTVDAAFGSPGAITVMNKHQKEFFLESITIEGFALGPVHFPCNSWVQSQKDHPGKRIFFTNKPLLPSETPDGLKKLRERELKNLRGDGSGARKLSDRIYDFDVYNDLGNPDKSSELSRPKLGGKEIPYPRRCRTGRHPTDTDKEAESRVEKPLPMYVPRDEQFEETKQKTFAAGRLKAVLHHLVPSLKASILAEDFADFGEIDGLYKEGLLLKLGFQDEIFDKFPLPKAIVNTLQESSKGLLKYDTPKILSKDKNAWLRDDEFARQAIAGINPVNIERVRTFPPVSNLDPEIYGPQHSALTSDHIIGHLDGLSVQQALEENRLYMLNYHDIFLPFLDRINALDGRKAYATRTIFFLTRLGTLKPVAIELSLPPHGPNHRSKRVVTPPVDATSNWVWQLAKAHVSSNDAGVHQLVNHWLRTHACLEPFILAAHRQLSAMHPIFKLLDPHMRYTLEINALARQSLISADGVIEEGFTAGSYGMEMSAAAYKSSWRFDMEGLPADLIRRGIAVPDPTQPHGVKLLIEDYPYANDGLLLWSAIQTWVRTYVERYYPNPNLIKTDSELQSWYSESINVGHADLRDAEWWPELNTVDDLVSILTTLIWLASAQHAALNFGQYPYGGYVPNRPPLMRRLIPDESDPLYASFISDPEKFYFSAMPSLLQTSKFMAVVDTLSTHSPDEEYIGERQQPSIWTGDGEIVDAFYGFAAEIGRIEKEIEKRNSDPDRRNRCGAGVLPYELLVPSSEPGVTCRGVPNSVSI

SEQ ID NO: 80 - protein, 919 aa, Brassica napus
MALVKEIMGHPLISGRPSLVFSASHFKKKTQTTQFSIKPFDRRPKTSKSGVVSAISEDLVKTLRFSTTTGDRKSEEEEKAAVKFKVRAVVTVRNKNKEDFKETLFKHLDAFGDKIGRNIVLELISTELDPKTNLPKKSNAAVLKDWSEKSKTKAERVHYTAEFTVDAAFGTPGAITIMNKHQKEFFLECITIEGFALGPVHFPCNSWVQSQNDHPEKRIFFTNQPFLPSETPEGLRKLRGKELKNLRGDGTGVRKLSDRIYDFDVYNDLGNPDKSSELSRPKLGGRERPYPRRCRTGRQPTDTDNEAESRVEKPLPMYVPRDEQFEETKQDTFAAGRLKAVLHHLVPSLKASILADDFSDFGEIDDLYKKGLLLKLGFQDEIFNKFPLPKGIVNTLQESSKGLLKYDTPKILSKDKNAWLRDDEFARQAIAGINPVNIERVKTFPPVSNLDPEIYGPQHSALTSDHIIGHLDGLSVQQALEENRLYMLDYHDIFLPFLDQINALDGRKAYATRTIFFLTRLGTLKPVAIELSLPSHGPNHRSKRVVTPPVDATSNWVWQLAKAHVSSNDAGVHQLVNHWLRTHACLEPFIIAAHRQLSAMHPIFKLLDPHMRYTLEINALARQSLISADGVIEGGFTAGQYGLEMSSAAYKSSWRFDMEGLPADLIRRGMAVPDPTQPHGLKLLIEDYPYANDGLLIWSAIQTWVRTYVERYYPNSNSIQTDSELQSWYSESINVGHADLREAEWWPKLDTVDDLVSILTTLVWLASAQHAALNFGQYPYGGYVPNRPPLMRRLIPDESDPEYASFISDPEKFYFSSMPSLLQTSKFMAVVDTLSTHSPDEEYIGERQQPSTWTGDAEIVDAFYGFAAEIGRIEKEIEKRNSDPNRRNRCGAGVLPYELLVPSSEPGVTCRGVPNSVSI

SEQ ID NO: 81 - protein, 919 aa, Brassica napus
MALAKELMGYPLTSKRPLLVWSASHFKKRTQPTQLSIKPFDRRPRTSKSGVVAAISEDLVKTLRFNTTTGDRKSEEEEKAAVKFKVRAVVTVRNKNKEDFKETLVKHLDAFGDKIGRNIVLELVSTELDPKTNMPKKSNAAVLKDWSKKSKTKAERVHYTAEFTVDAAFGSPGAITVMNKHQKEFFLESITIEGFAVGPVHFPCNSWVQSQKDHPEKRIFFTNQPFLPSGTPDGLKKLRERELKNLRGDGSGVRKLSDRIYDFDVYNDLGNPDKSSELSRPKLGGKEIPYPRRCRTGRHPTDTDKEAESRVEKPLPMYVPRDEQFEETKQKTFAAGRLKAVLHHLVPSLKASILAEDFADFGEIDGLYKEGLLLKLGFQDEIFNKFPLPKAIVNTLQESSKGLLKYDTPKILSKDKNAWLRDDEFARQAIAGINPVNIERVRTFPPVSNLDPEIYGPQHSALTSDHIIGHLDGLSVQQALEENRLYKLDYHDIFLPFLDRINALDGRKAYATRTIFFLTRLGTLKPVAIELSLPPHGPNHRSKRVVTPPVDATSNWVWQLAKAHVSSNDAGVHQLVNHWLRTHACLEPFILAAHRQMSAMHPIFKLLDPHMRYTLEINALARQSLISADGVIEEGFTAGSYGMEMSAAAYKSSWRFDMEGLPADLIRRGMAVPDSTQPHGLKLLIEDYPYANDGLLLWSAIQTWVRTYVERYYPNPNLIKTDSELQSWYSESINVGHADLRDAEWWPKLNTVDDLASILTTLIWLASAQHAALNFGQYPYGGYVPNRPPLMRRLIPDESDPEYASFISDPEKFYFSAMPSLLQTSKFMAVVDTLSTHSPDEEYIGERQQPSIWTGDAEIVDAFYGFAAEIGRIEKEIEERNSDPDRRNRCGAGVLPYELLVPSSEPGVTCRGVPNSVSI

SEQ ID NO: 82 - protein, 919 aa, Brassica napus
MALVKEIMGHPLISGRPSLVFSASHFKKKTQTTQFSIKPFDRRPNTSKSGVVSAISEDLVKTLRFSTTTGDRKSEEEEKAAVKFKVRAVVTVRNKNKEDFKETLFKHLDAFGDKIGRNIVLELISTELDPKTNLPKKSNAAVLKDWSEKSKTKAERVHYTAEFTVDAAFGTPGAITIMNKHQKEFFLECITIEGFALGPVHFPCNSWVQSQNDHPEKRIFFTNQPFLPSETPEGLRKLRGKELKNLRGDGTGVRKLSDRIYDFDVYNDLGNPDKSYELSRPKLGGRERPYPRRCRTGRQPTDTDNEAESRVEKPLPMYVPRDEQFEETKQDTFAAGRLKAVLHHLVPSLKASILADDFSDFGEIDDLYKEGLLLKLGFQDEIFNKFPLPKGIVNTLQESSKGLLKYDTPKILSKDKNAWLRDDEFARQAIAGINPVNIERVKTFPPVSNLDPEIYGPQHSALTSDHIIGHLDGLSVQQALEENRLFMLDYHDIFLPFLDRINALDGRKAYATRTIFFLTRLGTLKPVAIELSLPSHGPNHRSKRVVTPPVDATSNWVWQLAKAHVSSNDAGVHQLVNHWLRTHACLEPFIIAAHRQLSAMHPIFKLLDPHMRYTLEINALARQSLISADGVIEGGFTAGQYGLEMSSAAYKSSWRFDMEGLPADLIRRGMAVPDPTQPHGLKLLIEDYPYANDGLLIWSAIQTWVRTYVERYYPNSNSIQTDSELQSWYSESINVGHADLREAEWWPKLDTVDDLVSILTTLVWLASAQHAALNFGQYPYGGYVPNRPPLMRRLIPDESDPEYASFISDPEKFYFSSMPSLLQTSKFMAVVDTLSTHSPDEEYIGERQQPSTWTGDAEIVDAFYGFAAEIGRIEKEIEKRNSDPSRRNRCGAGVLPYELLVPSSEPGVTCRGVPNSVSI

SEQ ID NO: 83 - DNA, 2760 bp, Brassica napus
atggccttagctaaagagttaatgggttatcctctgacctccaaaagacccttacttgtttggtcggcgtcgcatttcaagaagaggacacagccaacacaattctcgatcaagccttttgataggagaccaagaacgtccaaatccggggtcgttgcggccatcagtgaagatttggtcaaaacgctacgtttcaacacaaccaccggtgacagaaagagcgaggaggaggagaaagcggcggtgaaattcaaggtgagagctgtggttacggtgaggaacaagaacaaggaggattttaaggagactcttgttaagcatttagatgcttttggtgataagatcggtcgaaacgttgtcttggagcttgttagcaccgaacttgatccaaaaacgaatatgccgaagaaaagcaatgcggcagttttaaaggactggtcaaagaagtcgaaaaccaaggcggagagggttcattacacggcggagttcacggtggacgcagcatttggctcaccgggagccatcaccgtcatgaataaacaccagaaagagttctttctggagagcatcaccatcgaaggtttcgcacttggccctgttcactttccatgcaactcttgggttcagtcccaaaaggatcacccagggaaacgaatctttttcactaataagccgcttttgccgagtgagacacctgatggattgaaaaaattgagggagagagagttgaagaatctaagaggagatgggagtggagcgaggaagttatcagacagaatctatgactttgatgtgtacaacgatcttggaaatcccgacaagtcatcagaactctctcggcccaagctcggcggcaaagagattccttaccctagacgatgtcgtaccggtcgccatccaactgataccgataaagaagcggagagccgagtagagaagccattacctatgtacgtaccacgagatgagcaattcgaagagactaagcagaaaactttcgcagcagggaggctaaaagcggtcttacaccacctagttccctcgctgaaagccagcattttagctgaggactttgctgactttggcgagatagatggtctatataaagaaggattgctactcaagttagggtttcaagatgaaatctttgacaagttccctttgcccaaggccatcgttaatacactccaagaatcttctaaaggactcctcaaatacgacactcccaaaatactatcaaaggataaaaatgcatggctacgtgatgatgagtttgcacgtcaagccatagctggaatcaatccagtcaacattgagagggtaaggactttcccaccggtcagtaatcttgaccccgaaatctacggtccacaacactccgctctcacttccgaccacatcattggacatctcgacggactatccgtacaacaagcgttggaagagaacagattgtatatgttgaattaccacgacatatttttaccgttcctagaccgaatcaatgcgctagacggacgcaaagcttatgctactcgaaccatattctttttgactcgtcttggtacacttaagcccgtagccattgagctaagtctccctccacatggccccaaccaccggtccaaacgcgtggttacacctcccgtcgatgcaacctctaattgggtgtggcagctcgctaaagcccacgttagctctaacgacgctggggtccaccagcttgtcaatcactggttacgaacccatgcgtgcttggaaccgtttatattagctgcacatagacaactgagcgctatgcatccgatattcaagctattagacccgcacatgaggtacacgttggaaatcaatgcattggctagacaatcgttgatcagtgcagacggtgtgattgaagaaggcttcactgccggctcatacggcatggaaatgagcgccgccgcatacaagagcagctggcggttcgacatggaaggcctccctgccgatctcattcgcagaggaatagcagttcctgacccgacacaaccacatggagttaaactcctaatcgaagactatccatacgccaacgacggtcttctactctggtcggctatccaaacctgggtccgaacctacgtggaacgctactacccaaacccgaacctaatcaaaacagactcggagctccaatcctggtactccgaatcaatcaacgtcggccacgccgatctccgcgacgccgagtggtggccagagctaaacaccgtcgacgatctcgtctccatcctcaccacactgatctggctcgcctcagctcagcacgcggctctcaacttcggacagtacccgtacggcggctacgtcccgaaccgtcctccgctgatgcggcggttgatccccgacgagtcggatccgttgtacgcgagtttcatctccgatccggagaagttttacttctcggcgatgccgagtttgttgcagacgtcgaagtttatggcggtggttgatactctgtcaacgcattcgccagatgaggagtatatcggggagagacagcagccgtcgatttggacgggagatggggagatcgttgatgcgttttatggattcgcggcggagatcggacggatagagaaggagattgagaaaaggaactctgatcctgaccgtagaaataggtgcggggctggtgttttgccgtatgagctgttggttccgagttccgagcctggtgttacgtgcagaggtgtacctaatagtgtgtcgatatag

SEQ ID NO: 84 - DNA, 2760 bp, Brassica napus
atggccttagttaaagagataatgggtcatcctctgatatcaggaaggccatcacttgttttctcggcttctcatttcaagaagaagacacagacaacgcaattctcgatcaagcctttcgatcggagaccaaaaacgtccaaatccggcgtcgtttcggccattagtgaagatttagtaaaaacgctgcgttttagcacaacaaccggagacagaaagagcgaggaggaggagaaagcggcggtgaaattcaaagtgagagctgtggttacagtgaggaacaagaacaaggaggattttaaggagactctttttaagcatttggatgcttttggtgacaagatcggtcggaacatcgtcttggagcttattagcaccgaacttgatccaaaaacgaatttgccgaagaaaagcaatgctgcggtgttaaaggattggtcagagaaatcgaaaaccaaggcggagagggttcattacacggcggagttcacggtggacgcagcgtttggcacgccgggagccatcaccatcatgaataaacaccagaaagagttttttctagagtgcataaccatcgaaggtttcgcacttggccctgttcactttccatgcaactcttgggttcagtcccaaaatgatcaccctgagaaacgaatcttcttcactaatcagccgtttttgccgagtgagacacctgaaggattaagaaaattaagggggaaagagttgaagaatctacgaggagatgggactggagtcaggaagttatcagacagaatctatgactttgatgtctacaacgatcttggaaatcccgacaagtcatctgaactctctcgtccgaaactcggtggcagagagaggccttaccctagacggtgtcgcactggtcgccagccaactgataccgataatgaagcggagagccgagtggaaaagccattacctatgtacgtgccacgagacgagcaatttgaagagactaagcaggacactttcgccgcagggaggttaaaagcggtgttacaccaccttgttccgtcgcttaaagctagtattttagctgatgacttttctgacttcggagagattgatgatctctacaaaaaaggcttgctactgaagttaggatttcaagatgagatattcaacaagttccctttgcctaagggcatcgttaataccctccaagaatcttcgaaaggactcctcaaatacgacactcccaaaatattatcgaaggataaaaacgcatggctacgagatgacgagttcgcacgtcaagccatagctggaatcaatccagtcaacattgagagagtcaagactttcccacccgtcagtaatcttgaccccgaaatctacggtccacaacactccgctctcacttccgaccacatcatcggacatcttgacggcttgtccgttcaacaagcgttggaagagaacagattgtatatgttggattaccatgacatattcttaccgttcctagaccaaatcaatgcgctcgatggacgcaaagcatatgctactcgaaccattttcttcttgactcgtcttggaacacttaagcccgtagccatcgagctaagcctcccttcccatggcccgaaccaccgatccaaacgagttgttacacctcctgtcgatgcaacctctaactgggtgtggcagctcgctaaagcacatgttagctccaacgatgctggagtccaccaacttgttaaccactggttacgaacccatgcatgcttggaaccgtttataatagctgcacataggcaattaagcgctatgcatccgatattcaaactattggatccacacatgaggtatacgttggagatcaatgcactggctagacaatcattgatcagtgcagacggtgtgattgaaggaggcttcactgctggccaatacggtttggaaatgagctccgcagcctacaaaagtagttggcggttcgacatggaaggcctccctgccgatctcattcgcagaggaatggcagttccagacccaacacaaccacatggacttaaactcctgatcgaagactatccatatgcgaacgacggtcttctaatatggtccgcaatccaaacatgggtccgaacttacgtggaacgttactatccaaactcgaactcaattcaaacagactcggaactccaatcgtggtactcggagtcaatcaacgtaggccatgcagatctccgcgaagccgagtggtggccaaagttagacaccgtggacgacctagtctccatcctcaccacactagtctggctcgcctccgctcaacacgccgctctcaacttcggacagtatccgtatggaggttacgtcccaaaccgacctccgctgatgcgacggttaatccctgacgagtcggatccggagtacgcaagttttatctcggatcctgagaaattttatttttcttcgatgccgagtttgttgcaaacgtcgaagtttatggcggtggttgatacgttgtcaacgcattctccggatgaggagtatatcggggagagacaacaaccgtccacttggaccggagatgcggagattgttgatgcgttttatggatttgcggcggagattggacggatagaaaaagagattgagaaaagaaacagtgatcctaaccgtagaaacaggtgtggagctggagttttgccttacgagttgttggttccgagttctgagccaggtgttacgtgcagaggtgtacctaatagtgtatcgatatag

SEQ ID NO: 85 - DNA, 2760 bp, Brassica napus
atggccttagctaaagagttaatgggttatccactgacctccaaaaggccattacttgtttggtcggcgtcgcatttcaagaagaggacacagccaacacaattatcgatcaagccttttgatcggagaccaagaacgtccaaatccggggtcgttgcggccatcagtgaagatttggtcaaaacgctacgtttcaacacaaccaccggtgacagaaagagcgaggaggaggagaaagcggcggtgaaattcaaggtgagagctgtggttacggtgaggaacaagaacaaggaggattttaaggagactcttgttaagcatttagatgcttttggtgataagatcggtcgaaacattgtcttggagcttgttagcaccgaacttgatccaaaaacgaatatgccgaagaaaagcaatgcggcagttttaaaggactggtcaaagaagtcgaaaaccaaggcggaaagggttcattacacggcggagttcacggtggacgcagcatttggctcaccgggagccatcaccgtcatgaataaacaccagaaagaattctttctagagagcatcaccatcgaaggtttcgcagttggtcctgttcactttccatgcaattcttgggttcagtcccaaaaggatcacccagagaaacgaatctttttcactaatcagccgtttttgccgagtgggacacctgatggattgaaaaaattgagggagagagagttgaagaatctaagaggagatgggagtggagtgaggaagttatcagacagaatctatgactttgatgtgtacaacgatcttggaaatcccgacaagtcatcagaactctctcgccccaagcttggcggcaaagagattccttaccctagacgatgtcgtaccggtcgccatccaactgataccgataaagaagcggagagccgagtggagaagccattacctatgtacgtaccacgagatgagcaatttgaagagactaagcagaaaactttcgctgcagggaggttaaaagcggtcttacaccacctagttccgtctctcaaagccagcattttagctgaggactttgctgactttggcgagatagatggtctctataaagaaggattgctactcaagttagggtttcaagatgaaatttttaacaagttccctttgcccaaggccatcgttaatacactccaagaatcttctaaaggactcctcaaatacgacactcccaaaatattatcgaaggataaaaatgcatggctacgagatgacgagtttgcacgtcaagccatagctggaatcaatccagtcaacattgagagggtcaggactttcccacccgtcagtaatcttgaccccgaaatctacggtccacaacactccgctctcacttccgaccacatcattggacatctcgacggactatccgtacaacaagcgttggaagagaacaggttgtataagttggattaccatgacatattcttaccgttcctagaccggatcaatgcactagacggacgcaaagcttatgctactcgaaccatattcttcttgactcgtctaggaacacttaaacccgtagccattgagctaagcctccctccccatggtcccaaccatcggtccaaacgcgtggttacacctcctgtcgacgcaacctctaattgggtgtggcagctcgctaaagcccacgttagctctaacgacgctggtgtccaccagcttgtcaatcactggttacgaacccatgcgtgcttggaaccgtttatattagctgcacatagacaaatgagcgctatgcatccgatattcaagctattggatccgcacatgaggtacacgttggaaatcaatgcattggctagacaatcgttgatcagtgcagacggtgtgattgaagaaggcttcactgccggctcatacggcatggagatgagcgccgccgcatacaagagcagttggcggtttgacatggaaggcctccctgctgatctcattcggagaggaatggcagttcctgactcgacacaaccacatggacttaaactcctaatcgaagactatccatacgctaacgacggtcttctactctggtcggctatccaaacctgggtccgaacctacgtggaacgctactatcccaacccgaacctaatcaaaacagactcggagctccagtcctggtactccgaatcaatcaacgtcggccacgctgatctccgcgacgccgagtggtggccaaagctaaacaccgtcgacgacctcgcctccatcctcaccacactaatctggctcgcctcagctcaacacgcggctctcaacttcggacagtacccgtacggcggctacgtccccaaccgtcctccgctgatgcggcggttgatccccgacgagtctgatccggagtacgcgagtttcatctccgatccggagaagttttacttctcggcgatgccgagtttgctgcagacgtcgaagtttatggcggtggttgatactctgtcaacgcattcgccggatgaggagtatatcggggagagacagcaaccgtcgatttggacgggagatgcggagatcgttgatgcgttttatggattcgcggcggagatcggacggatagagaaggagattgaggaaaggaactctgatcctgaccgtagaaataggtgcggggctggtgttttgccttatgagctgttggttccgagttccgagcctggtgttacttgcagaggtgtacctaatagtgtatcgatatag

SEQ ID NO: 86 - DNA, 2760 bp, Brassica napus
atggccttagttaaagagataatgggtcatcctctgatatcaggaaggccgtcacttgttttctcggcttctcatttcaagaagaagacacagacaacgcaattctcgatcaagccttttgatcggagaccaaacacgtccaaatccggcgtcgtttccgccattagtgaagatttagtaaaaacgctgcgttttagcacaacaaccggagacagaaagagcgaggaggaggagaaagcggcggtgaaattcaaagtgagagctgttgttacagtgaggaacaagaacaaggaggattttaaggagactctttttaagcatttggatgcttttggtgacaagatcggtcggaacatcgtcttggagcttattagcaccgaacttgatccaaaaacgaatttgccgaagaagagcaatgcagcggtgttaaaggattggtcagagaaatcgaaaaccaaggcggagagggttcattacacggcggagttcacagtcgacgcagcgtttggcacgccgggagccatcaccatcatgaataaacaccagaaagagttttttctagagtgcataaccatcgaaggtttcgcacttggccctgttcactttccatgcaactcttgggttcagtcccaaaatgatcaccctgagaaacgaatcttcttcactaatcagccgtttttgccgagtgagacacctgaaggattaagaaaactaagggggaaagagttgaagaatctaagaggagatgggactggagtcaggaagttatcagacagaatctatgactttgatgtctacaacgatcttggaaatcccgacaagtcatatgaactctctcgtccgaagctcggtggcagagagaggccttaccctagacggtgtcgcactggtcgccagccaactgataccgataatgaagcggagagccgagtggaaaagccattacctatgtacgtgccacgagacgagcaatttgaagagactaagcaggatactttcgccgcagggaggttaaaagcggtgttacaccaccttgttccgtcgcttaaagctagtattttagctgatgacttttctgactttggagagattgatgatctctacaaagaaggcttgctactcaagttagggtttcaagatgagatctttaacaagttccctttgcctaagggcatcgttaataccctccaagaatcttcgaaaggactcctcaaatacgacactccgaaaatattatcgaaggataaaaacgcatggctacgagatgacgagttcgcacgtcaagccatagctggaatcaatccagtcaacattgagagagtcaagactttcccacccgtcagtaatcttgaccccgaaatctacggtccacaacactccgctctcacttccgaccacatcatcggacatcttgacggcttgtccgttcaacaagcgctggaagagaacagattgtttatgttggattaccacgacatattcttaccgttcctggaccggatcaatgcgctcgacggacgcaaagcatatgctactcgaaccatattcttcttgactcgtctcggaacacttaagcccgtagccatcgagctgagcctcccttcccatggcccgaaccaccgatccaaacgagttgttacacctcctgtcgatgcaacctctaactgggtgtggcagctcgctaaagcacatgttagctctaacgatgctggagtccaccaacttgtcaaccactggttacgaacacatgcatgcttggaaccgtttataatagctgcacataggcaattaagcgctatgcatccgatatttaaactattggatccacacatgaggtacacgttggagatcaatgcactggctagacaatcattgatcagtgcagacggtgtgattgaaggaggtttcactgctggccaatacggtttggaaatgagctccgcagcatacaaaagtagttggcggttcgatatggaaggcctccctgccgatctcattcgcagaggaatggcagttccagacccaacacaaccacatggacttaaactcctgatcgaagactatccatatgcgaacgacggtcttttaatatggtccgcaatccaaacatgggtccgaacttacgtggaacgttactatccaaactcgaactcaatccagacagactcggaactccaatcatggtactccgagtcaatcaacgtaggccatgcagatctacgcgaagccgagtggtggccaaagttagacaccgtggacgacctagtctccatcctcaccacactagtctggctcgcctccgctcaacacgccgctctcaacttcggacagtatccgtatggaggttacgtcccaaaccgacctccgctgatgcgacggttaatccctgacgagtcggatccggagtacgcaagttttatctcggatccagagaaattttatttttcgtccatgccgagtttgttgcaaacgtcgaagtttatggcggtggttgatactttgtcaacgcattcgcctgatgaggagtatataggggagagacaacaaccgtccacttggaccggagatgcggagattgttgatgcgttttatggatttgcggcggagattggacggattgaaaaagagattgagaaaagaaacagtgatcctagccgtagaaacaggtgtggagctggagttttgccttacgagttgttggttcctagttctgagccaggtgttacgtgcagaggtgtacctaatagtgtatcgatatag

SEQ ID NO: 87 - DNA, 2094 bp, Zea mays
atgccggcggcgctgaagccgtaccgcgacgacgagctccgcaacctccgcggcgacgaccagcagggcccctaccaggagcacgaccgcgtgtaccgctacgacgtctacaacgacctcggcgagcccgacggcggcaacccgcgccccatcctcggcggctccgccgaccacccgtacccgcgccgctgccgcacgggccgcaagcccaccaaaaccgaccccaactcggagagccgactgtcgctggtggagcagatctacgtgccgcgggacgagcgcttcggccacctcaagatgtccgacttcctgggctactccatcaaggccatcacgcagggcatcatcccggcggtgcgcacgtacgtggacaccaccccgggcgagttcgactccttccaggacatcatcaacctgtacgagggcgggatcaagctgcccaagatccaggcgctcgaggacatgcgcaagctcttcccgctccagctcgtcaaggacctcctccccgccggcggggactacctgctcaagctccccatcccacagatcatccaagaggacaagaacgcgtggaggaccgacgaggagttcgcgcgggaggtgctcgccggcgtcaacccgatggtgatcacgcgcctcacggagttcccgcccaagagcacgctggaccccagcaagtacggcgaccacaccagcacgatcacggcggagcacatcgagaagaacctcgagggcctcacggtgcagcaggcgctggacggcaacaggctctacatcctggaccaccacgaccgcttcatgccgttcctcatcgacgtcaacaacctggagggcaacttcatctacgccaccaggacgctcttcttcctgcgcggcgacggcaggctcgcgcccctcgccatcgagctcagcgagccgtacatcgacggggacctcaccgtggccaagagcaaggtctacacgccggcgtccagcggcgtcgaggcctgggtgtggcagctcgccaaggcctatgtcgccgtcaacgactctggctggcaccaactcgtcagccactggctgaacacccacgcggtgatggagccgttcgtgatcgcgacgaaccggcagctgagcgtgacgcacccggtgcacaagctcctgagctcgcacttccgcgacaccatgaccatcaacgcgctggcgcggcagacgctcatcaacggcggcggcatcttcgagatgaccgtcttcccgggcaagtacgcgctgggcatgtcctccgtggtgtacaagagctggaacttcaccgagcagggcctccccgccgacctcgtcaagaggggcgtggcggtggcggacccgtccagcccgtacaaggtgcggctgctgatcgaggactacccgtacgcgagcgacgggctggccatctggcacgccatcgagcagtgggtgggcgagtacctggccatctactaccccgacgacggcgcgctgcggggcgacgaggagctgcaggcgtggtggaaggaggtgcgcgaggtcgggcacggcgaccacaaggacgcgccctggtggcccaagatgcaggccgtgtcggagctcgccagcgcctgcaccaccatcatctggatcgcgtcggcgctccacgccgccgtcaacttcggccagtacccgtacgcggggtacctcccgaacaggcccacggtgagccggcgccggatgccggagcccggcagcaaggagtacgaggagctggagcgcgacccggagcgcggcttcatccacaccatcacgagccagatccagaccatcatcggcatctcgctcatcgagatcctctccaagcactcctccgacgaggtgtacctcggccagcgcgacacccccgagtggacctccgacgcccgggcgctggcggcgttcaagaggttcagcgacgcgctggtcaagatcgagggcaaggtggtgggcgagaaccgcgacccgcagctgaggaacaggaacggccccgccgagttcccctacatgctgctctatcccaacacctctgaccacagtggcgccgccgcagggctcactgccaagggcatccccaacagcatctccatctga

SEQ ID NO: 88 - DNA, 2795 bp, Zea mays
catgccacgctgatctttctgtcttttggtgccgccccgattccgaacggcggcgcagacgtacctgccaagccagatgccggcggcgctgaagccgtaccgcgacgacgagctccgcaacctccgcggcgacgaccagcagggcccctaccaggagcacgaccgcgtgtaccgctacgacgtctacaacgacctcggcgagcccgacggcggcaacccgcgccccatcctcggcggctccgccgaccacccgtacccgcgccgctgccgcacgggccgcaagcccaccaaaaccggtgcgtgcgccgtgcgcggctcttctatcttctcggacgcaacatttgctgcagggcagagaggttgttgacgctgacctgtgaccgcatcgcagaccccaactcggagagccgactgtcgctggtggagcagatctacgtgccgcgggacgagcgcttcggccacctcaagatgtccgacttcctgggctactccatcaaggccatcacgcagggcatcatcccggcggtgcgcacgtacgtggacaccaccccgggcgagttcgactccttccaggacatcatcaacctgtacgagggcgggatcaagctgcccaagatccaggcgctcgaggacatgcgcaagctcttcccgctccagctcgtcaaggacctcctccccgccggcggggactacctgctcaagctccccatcccacagatcatccaaggcacgtcacgtataccgatcgatgtcaggggccggctgttgtctggtctgcatatatatatgtgctcctatggttaactgtgactgcgtacgtttcgcggaacagaggacaagaacgcgtggaggaccgacgaggagttcgcgcgggaggtgctcgccggcgtcaacccgatggtgatcacgcgcctcacggtgagtcactcactttgtgcaaaatgcgagacccgacccgagacggaatgtgcctgacgcgctcgatttacaggagttcccgcccaagagcacgctggaccccagcaagtacggcgaccacaccagcacgatcacggcggagcacatcgagaagaacctcgagggcctcacggtgcagcaggcgctggacggcaacaggctctacatcctggaccaccacgaccgcttcatgccgttcctcatcgacgtcaacaacctggagggcaacttcatctacgccaccaggacgctcttcttcctgcgcggcgacggcaggctcgcgcccctcgccatcgagctcagcgagccgtacatcgacggggacctcaccgtggccaagagcaaggtctacacgccggcgtccagcggcgtcgaggcctgggtgtggcagctcgccaaggcctatgtcgccgtcaacgactctggctggcaccaactcgtcagccactggtacgtacgaagaactacaactactcctatatatgtcctatatgacaatggcatcgcatcgtgtcatgtctatgacatcgccaaatgcatgcgttgatggtcatgatctattctctgcgtgcgtgcaggctgaacacccacgcggtgatggagccgttcgtgatcgcgacgaaccggcagctgagcgtgacgcacccggtgcacaagctcctgagctcgcacttccgcgacaccatgaccatcaacgcgctggcgcggcagacgctcatcaacggcggcggcatcttcgagatgaccgtcttcccgggcaagtacgcgctgggcatgtcctccgtggtgtacaagagctggaacttcaccgagcagggcctccccgccgacctcgtcaagaggggcgtggcggtggcggacccgtccagcccgtacaaggtgcggctgctgatcgaggactacccgtacgcgagcgacgggctggccatctggcacgccatcgagcagtgggtgggcgagtacctggccatctactaccccgacgacggcgcgctgcggggcgacgaggagctgcaggcgtggtggaaggaggtgcgcgaggtcgggcacggcgaccacaaggacgcgccctggtggcccaagatgcaggccgtgtcggagctcgccagcgcctgcaccaccatcatctggatcgcgtcggcgctccacgccgccgtcaacttcggccagtacccgtacgcggggtacctcccgaacaggcccacggtgagccggcgccggatgccggagcccggcagcaaggagtacgaggagctggagcgcgacccggagcgcggcttcatccacaccatcacgagccagatccagaccatcatcggcatctcgctcatcgagatcctctccaagcactcctccgacgaggtgtacctcggccagcgcgacacccccgagtggacctccgacgcccgggcgctggcggcgttcaagaggttcagcgacgcgctggtcaagatcgagggcaaggtggtgggcgagaaccgcgacccgcagctgaggaacaggaacggccccgccgagttcccctacatgctgctctatcccaacacctctgaccacagtggcgccgccgcagggctcactgccaagggcatccccaacagcatctccatctgagcgactggtaccactaccaccccaggagtgctacgtacgagctggtacatgaataagctaatataagcaatcgtgtaaacgggaagagagcggccggcacgagacggaccatgtattttgcgtaaacgtgtgggctggtgaatcgaattactaccacgtaataagtgaagtgcttgttgcaatcattggcctgccagcttcaagattcttgcagttactattct

SEQ ID NO: 89 - protein, 697 aa, Zea mays
MPAALKPYRDDELRNLRGDDQQGPYQEHDRVYRYDVYNDLGEPDGGNPRPILGGSADHPYPRRCRTGRKPTKTDPNSESRLSLVEQIYVPRDERFGHLKMSDFLGYSIKAITQGIIPAVRTYVDTTPGEFDSFQDIINLYEGGIKLPKIQALEDMRKLFPLQLVKDLLPAGGDYLLKLPIPQIIQEDKNAWRTDEEFAREVLAGVNPMVITRLTEFPPKSTLDPSKYGDHTSTITAEHIEKNLEGLTVQQALDGNRLYILDHHDRFMPFLIDVNNLEGNFIYATRTLFFLRGDGRLAPLAIELSEPYIDGDLTVAKSKVYTPASSGVEAWVWQLAKAYVAVNDSGWHQLVSHWLNTHAVMEPFVIATNRQLSVTHPVHKLLSSHFRDTMTINALARQTLINGGGIFEMTVFPGKYALGMSSVVYKSWNFTEQGLPADLVKRGVAVADPSSPYKVRLLIEDYPYASDGLAIWHAIEQWVGEYLAIYYPDDGALRGDEELQAWWKEVREVGHGDHKDAPWWPKMQAVSELASACTTIIWIASALHAAVNFGQYPYAGYLPNRPTVSRRRMPEPGSKEYEELERDPERGFIHTITSQIQTIIGISLIEILSKHSSDEVYLGQRDTPEWTSDARALAAFKRFSDALVKIEGKVVGENRDPQLRNRNGPAEFPYMLLYPNTSDHSGAAAGLTAKGIPNSISI